European Patent Specification EP 3 298 148 B1, published July 26, 2023. Title: Verfahren und Konstrukte zur gezielten Nukleinsäure Editierung in Pflanzen. Applicant: KWS SAAT SE. The sequence listing filed with the application follows.

SEQUENCE LISTING (61 sequences)

SEQ ID NO: 1 - DNA, 259 bp, Artificial sequence
  VP16 activator comprising sequence
ctaagctttcgacggcccccccgaccgacgtcagcctgggggacgagctccacttagacggcgaggacgtggcgatggcgcatgccgacgcgctagacgatttcgatctggacatgttgggggacggggattccccggggccgggatttaccccccacgactccgccccctacggcgctctggatacggccgacttcgagtttgagcagatgtttaccgatgcccttggaattgacgagtacggtgggtagagatcttc

SEQ ID NO: 2 - protein, 11 aa, Artificial sequence
  VP16 activator
DALDDFDLDML

SEQ ID NO: 3 - protein, 50 aa, Artificial sequence
  VP64 activator with glycine serine spacers
DALDDFDLDMLGSDALDDFDLDMLGSDALDDFDLDMLGSDALDDFDLDML

SEQ ID NO: 4 - DNA, 615 bp, Arabidopsis thaliana EAR 1 repressor
atggagagatcaaacagcatagagttgaggaacagcttctatggccgtgcaagaacttcaccatggagctatggagattatgataattgccaacaggatcatgattatcttctagggttttcatggccaccaagatcctacacttgcagcttctgcaaaagggaattcagatcggctcaagcacttggtggccacatgaatgttcacagaagagacagagcaagactcagattacaacagtctccatcatcatcttcaacaccttctcctccttaccctaaccctaattactcttactcaaccatggcaaactctcctcctcctcatcattctcctctaaccctatttccaaccctttctcctccatcctcaccaagatatagggcaggtttgatccgttccttgagccccaagtcaaaacatacaccagaaaacgcttgtaagactaagaaatcatctcttttagtggaggctggagaggctacaaggttcaccagtaaagatgcttgcaagatcctgaggaatgatgaaatcatcagcttggagcttgagattggtttgattaacgaatcagagcaagatctggatctagaactccgtttgggtttcgcttaa

SEQ ID NO: 5 - DNA, 972 bp, Petroselinum crispum Parsley_Ubi4
aaaaattacggatatgaatataggcatatccgtatccgaattatccgtttgacagctagcaacgattgtacaattgcttctttaaaaaaggaagaaagaaagaaagaaaagaatcaacatcagcgttaacaaacggccccgttacggcccaaacggtcatatagagtaacggcgttaagcgttgaaagactcctatcgaaatacgtaaccgcaaacgtgtcatagtcagatcccctcttccttcaccgcctcaaacacaaaaataatcttctacagcctatatatacaacccccccttctatctctcctttctcacaattcatcatctttctttctctacccccaattttaagaaatcctctcttctcctcttcattttcaaggtaaatctctctctctctctctctctctgttattccttgttttaattaggtatgtattattgctagtttgttaatctgcttatcttatgtatgccttatgtgaatatctttatcttgttcatctcatccgtttagaagctataaatttgttgatttgactgtgtatctacacgtggttatgtttatatctaatcagatatgaatttcttcatattgttgcgtttgtgtgtaccaatccgaaatcgttgatttttttcatttaatcgtgtagctaattgtacgtatacatatggatctacgtatcaattgttcatctgtttgtgtttgtatgtatacagatctgaaaacatcacttctctcatctgattgtgttgttacatacatagatatagatctgttatatcattttttttattaattgtgtatatatatatgtgcatagatctggattacatgattgtgattatttacatgattttgttatttacgtatgtatatatgtagatctggactttttggagttgttgacttgattgtatttgtgtgtgtatatgtgtgttctgatcttgatatgttatgtatgtgcagc

SEQ ID NO: 6 - DNA, 384 bp, Arabidopsis thaliana Arabidopsis_U6
ctttttttcttcttcttcgttcatacagtttttttttgtttatcagcttacattttcttgaaccgtagctttcgttttcttctttttaactttccattcggagtttttgtatcttgtttcatagtttgtcccaggattagaatgattaggcatcgaaccttcaagaatttgattgaataaaacatcttcattcttaagatatgaagataatcttcaaaaggcccctgggaatctgaaagaagagaagcaggcccatttatatgggaaagaacaatagtatttcttatataggcccatttaagttgaaaacaatcttcaaaagtcccacatcgcttagataagaaaacgaagctgagtttatatacagctagagtcgaagtagtg

SEQ ID NO: 7 - DNA, 1502 bp, Zea spp. Maize_Ubi_Intron
tgcagcgtgacccggtcgtgcccctctctagagataatgagcattgcatgtctaagttataaaaaattaccacatattttttttgtcacacttgtttgaagtgcagtttatctatctttatacatatatttaaactttactctacgaataatataatctatagtactacaataatatcagtgttttagagaatcatataaatgaacagttagacatggtctaaaggacaattgagtattttgacaacaggactctacagttttatctttttagtgtgcatgtgttctcctttttttttgcaaatagcttcacctatataatacttcatccattttattagtacatccatttagggtttagggttaatggtttttatagactaatttttttagtacatctattttattctattttagcctctaaattaagaaaactaaaactctattttagtttttttatttaataatttagatataaaatagaataaaataaagtgactaaaaattaaacaaataccctttaagaaattaaaaaaactaaggaaacatttttcttgtttcgagtagataatgccagcctgttaaacgccgtcgatcgacgagtctaacggacaccaaccagcgaaccagcagcgtcgcgtcgggccaagcgaagcagacggcacggcatctctgtcgctgcctctggacccctctcgagagttccgctccaccgttggacttgctccgctgtcggcatccagaaattgcgtggcggagcggcagacgtgagccggcacggcaggcggcctcctcctcctctcacggcaccggcagctacgggggattcctttcccaccgctccttcgctttcccttcctcgcccgccgtaataaatagacaccccctccacaccctctttccccaacctcgtgttgttcggagcgcacacacacacaaccagatctcccccaaatccacccgtcggcacctccgcttcaaggtacgccgctcgtcctccccccccccccctctctaccttctctagatcggcgttccggtccatggttagggcccggtagttctacttctgttcatgtttgtgttagatccgtgtttgtgttagatccgtgctgctagcgttcgtacacggatgcgacctgtacgtcagacacgttctgattgctaacttgccagtgtttctctttggggaatcctgggatggctctagccgttccgcagacgggatcgatctaggataggtatacatgttgatgtgggttttactgatgcatatacatgatggcatatgcagcatctattcatatgctctaaccttgagtacctatctattataataaacaagtatgttttataattattttgatcttgatatacttggatgatggcatatgcagcagctatatgtggatttttttagccctgccttcatacgctatttatttgcttggtactgtttcttttgtcgatgctcaccctgttgtttggtgttacttctgcagg

SEQ ID NO: 8 - DNA, 360 bp, Triticum spp. U6
gaccaagcccgttattctgacagttctggtgctcaacacatttatatttatcaaggagcacattgttactcactgctaggagggaatcgaactaggaatattgatcagaggaactacgagagagctgaagataactgccctctagctctcactgatctgggcgcatagtgagatgcagcccacgtgagttcagcaacggtctagcgctgggcttttaggcccgcatgatcgggctttgtcgggtggtcgacgtgttcacgattggggagagcaacgcagcagttcctcttagtttagtcccacctcgcctgtccagcagagttctgaccggtttataaactcgcttgctgcatcagactt

SEQ ID NO: 9 - DNA, 377 bp, Oryza spp. U3
aaggaatctttaaacatacgaacagatcacttaaagttcttctgaagcaacttaaagttatcaggcatgcatggatcttggaggaatcagatgtgcagtcagggaccatagcacaagacaggcgtcttctactggtgctaccagcaaatgctggaagccgggaacactgggtacgttggaaaccacgtgatgtggagtaagataaactgtaggagaaaagcatttcgtagtgggccatgaagcctttcaggacatgtattgcagtatgggccggcccattacgcaattggacgacaacaaagactagtattagtaccacctcggctatccacatagatcaaagctggtttaaaagagttgtgcagatgatccgtggc

SEQ ID NO: 10 - DNA, 763 bp, Zea spp. U3
gaattccatctaagtatcttggtaaagcatggattaatttggatgcccacttcaggtctatgcagctccggtgccttgtgattgtgagttgtgaccgatgctcatgctattctgcatttctgcgatgtatgtagctagtagatcttcaaaactaacaccgcatgccatcatcatccactgcttgattttagtctcaccgctggccaaaaatgtgatgatgccagaaacctcaactaccttgaatcaacacgggcccaacagtgtgatgacgacagaaacaaaaaaaaatgagccaatagttcagaaggaggcactatgcagaaactacatttctgaaggtgactaaaaggtgagcgtagagtgtaattactagtagtttagccaccattacccaaatgctttcgagcttgtattaagatttcctaagctgagcatcatcactgatctgcaggccaccctcgcttcgctgccaagatcaacagcaaccatgtggcggcaacatccagcattgcacatgggctaaagattgagctttgtgcctcgtctagggatcagctgaggttatcagtctttcctttttttcatccaggtgaggcatcaagctactactgcctcgattggctggacccgaagcccacatgtaggataccagaatgggccgacccaggacgcagtatgttggccagtcccaccggttagtgccatctcggttgctcacatgcgtagaagccagcttaaaaatttagctttggtgactcacagc

SEQ ID NO: 11 - DNA, 1880 bp, Brachypodium spp. EF1
cttcaccgccattgcaaaaattgtcaataaatatttagagtgggtggcatcagaaaaacatctctagtggactctcttcctatcatagctactcgggctgtagatagaacgagggcacaagagttgggtggcgtaggtttactcgtgacctcaactcttttggctgtgtcttacgtctaagatgggtttggcatgtgagaaacataggtctaagcaattcatgttagggctgttgcattgttgttgcatcaaccaaatgtccagatagcagttcatgctacatctagttgaaaaccctcatcattaggcggaacatgtgttcttttttagcatagtcaaagtcagattgcggcactcgctcatccacggaaagaattttccctgtgcaggcatctcgatcaaaagacgcaaattaatttttgaatagcgatataacaatatctaattaacgtttcttgttttctgcgaaatgtctttcatcataaaatgagtcatctcgatgagcccaagtgacatagcccaacaccccaccccaccaataaaagtgaagaaaacatgttgggaaaactataccaagtaaaatacgagttgttctaaagaaaaagtaaagtacgagttagatcgcaccctgtcctggagtgtggcttgatgatccaactcctagcattgtatccctgtttttggatgatgtaactattatttacaatgaataaagaggtgttttactagtaaaaaaatcttgaggggaggagaaaataatggaggtcttttttcaaaccgatggactattatttttagtgaaagagaataatattattggaaaaattattctatccacttattttatattggcagaatacaaagaatggtggggtccacgcggaacttgcggcccccgaaacctatcgagggcgcggtacccaagcaaggaacggaggaaacttgcggggcccgaaacctagtgataaaaggcatatcatccacacgatgaagatctgacggaccatatctcccaccacggaaagccatcagacgaggatcagacggccaggaaggaaccctagcgcccgccggtgccaatataaagcgccactctctctcgtcttaagccccagcctctccattcccctctccctctcgccgccgccgtctccttctcctactcccttcgaggtgtgttgttcatccgtcccgaatccatccatcccctcttcagatgtgttgttcatggctctaatagctctagatctgcttgtttgtgttgtttagctctagatctactcgcgcgcgcttctctctcgatctcctgtagaacaattttggttggttttttgtgcatatccatggtaattttgtctgcaatatggaggaggctttctaagctcctacgtagcatcgatctttagaattccctcggtttctgtttatttcttcgcgagggctctctgttatctgtaggagtagctgtaagcgcggttcgttacggattaatcgtcatgcttagttgaacctatcggtcgaaggatttgtgtgggttgtcgtgtagaattgacaccatctacttactgtactgatatgccgatctgtaggatactcttcattacttttgtttactgctagttgtggtgtagatttagcattctcaaacccatgctgtagcgtttctaatattgttacatagatctaccggtgcctgttaattgtattcgatcgggcgtttctacatctgtccgcccacctagttttatatgtggtaatcaaaattgcgttgacttcgtgatgctgtctgtgtactgtttttaatcgctcttacttagatgatcaacatggtgatggttacgatttactgttttctaatccctgttacttcgatgctgcag

SEQ ID NO: 12 - DNA, 2690 bp, Maize Streak Virus (MSV) South African Strain
atggatccacagaacgccctgtattatcagccgcgggtacccactgcagctccgacatccggaggagtgccgtggagtcgcgtaggcgaggtagctattttgagctttgttgcattgatttgcttttacctgctttacctttgggtgctgagagaccttatcttagttctgaaggctcgacaaggcagatccacggaggagctgatatttggtggacaagctgtggataggagcaaccctatccctaatctaccagcaccaccaagtcagggcaatcccgggccatttgttccaggcacgggataagcaatcagccatgtccacgtccaagaggaagcggggagatgatgcgaattggagtaagcgggtgcctaagaagaagccttcttcagctgggctgaagagggctggaagcaaggccgataggccatccctccaaatccagacactccagcatgctgggaccaccatgataactgtcccatccggaggagtatgtgacctcatcaacacctatgcccgaggatctgacgagggcaaccgccacaccagcgagactctgacgtacaagatcgccgtcgactaccacttcgttgccgacgcggctgcctgccgctactccaacaccggaaccggtgtaatgtggctggtgtatgacaccactcccggcggacaagctccgaccccgcaaactatatttgcctaccctgacacgctaaaagcgtggccggccacatggaaagtgagccgggagctgtgtcatcgcttcgtggtgaaacggcgatggttgttcaacatggagaccgacggtcggattggttcggatatccctccctcgaatacaagttggaagccttgcaagcgcaacatctacttccacaagttcacgagtgggttgggagtgagaacgcagtggaagaatgtaacggacggaggagttggtgccatccagagaggagctttgtacatggtcattgcccccggcaatggccttacatttactgcccatgggcagacccgcctgtactttaagagtgttggcaaccagtaatgaataaaaacgcccgttttattatatctgatgaatgctgaaagcttacattaatatgtcgtgcgatggcacgaaaaaacacacgcaatcaatacaggggggtagtcggcgggcggctaagggtggtgctcggcgggcaaaacatcgaaaaatcaagatctatatgaattacacttcctccgtaggaggaagcacagggggagaataccacttctcccccggcgacataatgtaaatgatgcagtttgcctcgaaatactccagctgccctggagtcatttccttcatccaatcttcatccgagttggcgaggattattgtaggcttagacttcttctgcacctttttcttcttaccatacttggggtttacaatgaaatccctctgacagccaactaactgtttccaacaaggacagaatttaaacggaatatcatctacgatgttgtagattgcgtcttcgttgtatgaagaccaatcaacattattttgccagtaattatgaacccctaggcttctggcccaagtagattttccggttcttgttgggccgacgatgtagaggctctgctttcttgatctttcatctgatgactggatacagaatccatccattggaggtcagagattgcatcctcgagggtataacaggtaggttgaaggagcatgtaagcttcgggactaacctggaagatgttaggctggagccaatcattgattgactcattacaaagtaaatcaggtgaggagggtggatgaggattggtgaactcttcctgaatctcaggaaaaagcttatttgcagagtattcaaaatactgcaattttgtggaccaatcaaagggaagctctttctggatcatggagaggtactctgctttggaagtagcgtgtgaaataatgtctcgcattatttcatctttagaaggctttttttcctttacctctgaatcagattttcctaggaagggggacttcctaggaatgaaagtacctctctcaaacacagccagaggttccttgagaatgtaatccctcactctgttaactgacttggcactctgaatatttgggtgaaacccatttatatcaaagaaccttgagtcagatatccttaccggcttctctgtctgaagcaatgcatgtaaatgcaaacttccatctttatgtgcctctcgggcacatagaatatacttgggaatccaacgaacgacgagctcccagatcatctgacaggcgatttcaggattttctggacactttggataggttaggaacgtgttagcgttcctgtgtgagaactgacggttggatgaggaggaggccatagcagacgacggaggctgaggctgagggatggcagactgggagctccaaactctatagtatacccgtgcgccttcgaaatccgccgctcccttgtcttatagtggttgtaaatgggccggaccggtccggcccagcaggaaaagaaggcgcgcactaatattaccgcgccttcttttcctgcgagggcccggtagggaccgagcgctttgatttaaagcctggttctgctttgtatgatttatctaaagcagcccaatctaaagaaaccggtcccgggcactataaattgcctaacaagtgcgattcattc

SEQ ID NO: 13 - DNA, 6337 bp, Maize rayado fino virus (MYDV)
gtcctctgcccccttcttgcgcccgatcgccgcaagtcgcattctgcaccagctctcgctcgtccagaaacagatcaatctttcggcctcttttcttgcactcttcttcgttgcacctctctagatgtctagtttcctgcgtggtggccatctcctcagcggagtcgagtccctcacaccaaccactcaccgcgacaccatcactgcacccatcgttgagtcccttgccaccccccttcgccgatccctcgaacgctacccttggtccatcccaaaggagttccattcgttcctccatacctgtggcgtcgacatctccggcttcggccatgccgctcatccccaccctgtccacaagaccatcgagacccacctccttctcgatgtctggcccaattacgcccggggcttgtctgatgtcatgttcatcaagcccgagaagttcgccaagctccagtcccgacagcccaatttcgcccacctcatcaactaccggctcgtgcctaaagacaccacccggtacccttccacttccacgaatctcccggactgcgagaccgtcttcatgcatgatgcgctcatgtactacaccccagggcagatcgctgacctcttcttcctttgcccccagctccagaagatctacgcctcgctggtcgtccctgcagagtcgagtttcacgcatctctcgctccatccggaactttaccgcttccgtttccagggttctgaccttgtctacgagccggagggcaaccctgccgccaactacacgcagccgcgttcggccctcgactggctccagaccaccggcttcaccgtcggtcacgaattcttctccgtcacacttctcgactctttcggcccggtccattccctcctcatccagcgtggccgcccccctgtctttcaggccgaagacgtcgcttccttccgcgtcccggacgccgtcgccctccctgctcctgcctccctccaccaggacctgcgtcaccgactggtcccccgcaaggtgtacgacgcactcttcaactacgtccgagccgtccgcacccttcgggtcacagaccccgctggtttcgtccggacccaggtcggtaagcctgagtacagttgggtcacctcttccgcctgggacaatctccagcacttcgcgctccagactgccgccgttcgtcccaacacctcgcatcccctctttcagtcgcccttcgcccgtttgtcccattggctccgcacccacacttgggcgctctggtgcatggcttccccctcggcctctgtctccgcttgggccgctgccagcgctcttggccggctcctcccgcttcacaccgaccgtctcaggttgttcggcttcgacatcgttgggcggagattctggcctcgtctcccattccatggccccgagccaaggttcctttgggagacccatccagcctgccgcccgccagtgctcttcgccgactcggcctttgagtgccaaatccttgctggtttggcaaaccggtgttctccctcccccttctggtcgcgcttgttccccacggcctctccgccgcactgggtcgcctattcagccttggccctagctgcagtgccacttgctgcgttagcgttgcgctggttttacggcccggattctccccaggctcttcatgatcagtaccacgccaccttccatcccgacccgtggactcttgacctcccccgccggcttcgccgcttcgagcgcgagcccttcatgcggacgggttccgcaccttcgcctcagtcgctccctccttctggaggctctcttcttcctgtcgagcctcctcttgcttcgagcgagcccgagcctgcccttgagccgccatcccccgcggccccggtcccgactccttctccagctccagttccagagcctcctccttctcccgagtcagtcgcccctccagtcgccgtcgcctcgcccgccgtgcaacctgttcgggctccgtccccctctccagcgcttttgggcgccgagcttcgtttcggggatcttcctcctgtctctgcttgggacagtgaccccgagatttcgaagcttggtgagtccacccaaggcaccgtttttgctgtcacccccggccctcgcgctcctgagccagacactgcccgcttagacgctgatccttcggctagcggccccgttatggagttccgcgagcttcagaagggcgcttacatcgagccgactggcgctttcctcacccgggctcgcaactcggtgtcctccagcatcccttatcctgcgagggcggcttgtcttctcgtggccgtcagtcaagcaacagggctccccacccgcactctctgggctgccctctgtgctaatcttccggattccgttcttgacgacggctcgctcgccaccttgggcctcaccaccgaccacttcgccgtcctcgcccgcatcttctccttgaggtgccgcttcgtgagtgagcatggcgatgttgagctcgggctccacgacgccacctctcgctttacgatccgccacacccccggccacttcgagctcgtggccgacaacttctcccttcccgctctcgtcggcgcctcttctgttccaggctccgacctagccgaagcgtgcaagcgtttcgtggctccggaccgcaccgttcttccattccgggacgtccacatccatcgcaccgacgtccgccgtgccaaaaacctcatttccaacatgaagaacggcttcgacggtgtcatggcgcaggccaatcctctggatccgaagagtgcccgagagcggttcctcatgctcgactcctgcctcgacattgccgcgcctcgccgggtccgtcttatccacatagcgggcttcgctggttgcgggaaatcctggccgatctcccatctgctccgtacccccgccttccgtgttttcaagctcgccgttccaaccaccgagcttcgcgacgagtggaaggccctcatggatcctcgcgaccaggacaagtggcgcttcggcacctgggagtcctctctcctcaagactgcccgcgtccttgtcattgatgaggtgtacaagatgcctcgcgggtaccttgatctggccatccatgcggacgccgccattcagttcgtgattttgctcggcgatccaattcaaggcgagtaccattccacacatcccagctcctccaatgcccgcctttctcccgagcatcggtatctccgcccgtatgtggacttctactgcttctggagtcgtcgcatccctcggaacgtggcccgcgccctcgatgtgcccacgacctcgaccgagatgggttttgctcgctactcgcagcagttcccattctccgggaagatcctcatctcggcgcgcgactccgccaagagcttggctgactgtggttatcatgctgtcaccatagctagcagccaagggtccactattgccggcccagcttatgtccacctcgacaatcattcgaggcgcctctcacatcaacattcgcttgtcgccatcactcgatccaagtccggcatagtattcactggcgacaaggctgcagcggatggcacctcctctgctaatctccttttctccgctgtgctcctcgaccgacgcctctcggtgcgctctctcttcagcgcgctcctgccttgctgtccgtttgtcacggagcctccaacgtctcgagccgttctccttcgcggagccggctacggcgtcgctcggccccttcgcgctcgtgacgcccctcctctcggccccgatttcgtcggagatgttattctggactcctccgccccgattcttggcgacggatcggccaacgctccccaggtcagcactcactttcttccagagacgcgtcggcctttgcacttcgacatcccttccgcccgccatcaagtggccgatcatcctctcgcgcccgatcactccgcctgcgctatcgagcccgtgtaccctggcgagagcttcgaatctctggcctctcttttcctcccccctacggatgccgagagcaaggagacttacttccgaggggagatgtcgaatcaattccctcatctcgacaagccgttcgagttaggtgcgcagacgtcgagcctcctcgcgccactccacaactccaaacatgatcccacgcttctcccggcttccatcggtaagagactgcgcttccgtcactcagaggctccctacgtcatcgctcctcgcgacgagatcttggggtcactcctctatgaggcctggtgtcgagcctatcgccgttctcctcgggacgtcgagccgttcgacccagacctctacgctgagtgcattaacctcaacgagttcgcgcagctctcctccaagacccaggcgactatcatggccaacgccaaccgcagcgacccagactggcgctggtccgccgttcgcattttcgccaagacgcagcataaggtcaacgagggctcgcttttcggctcctggaaagcttgccagaccctcgcgcttatgcacgacgccgtcgttttgctccttggccccgtcaagaagtatcaacgcttcttcgaccagcgcgatcggccttccactctttacgtccatgcgggccacacccccttcgagatggctgactggtgccgcgcccatttgacccccgcggtcaagctggccaatgactacaccgcctttgaccagtcacagcacggcgaggctgttgtcttcgagcgctacaagatgaatcgtctctcaattcctgccgagctcgtggacttgcacgtctatctgaagaccaatgtctccacccagtttggcccgttgacgtgcatgcgcctcactggtgagcccggcacctacgacgacaacaccgactacaacatcgccgtgctccatctcgagtacgctgtcggctctactccgctcatggtctctggtgatgactcgctgctcgactccgagcctcctgtccgtgaccagtggtccgccatcgctcccatgctcgctctcaccttcaagaaggagcgcggccgttatgccactttttgcggctattacgtcggcttcaccggcgcggtccgatcgcctccggccctttttgcgaagcttatgattgcggttgacgacggatccatctccgacaagctcatcgcctatctcacggagttcaccgttggtcattcttccggcgatgctttctggaccatcctcccagtcgaagctgttccttaccagagcgcctgctttgacttcttctgccgtcgagctccggcgcaagccaaagtgatgttgcggcttggcgaggccccagagtctcttctttccctggcgttcgagggtctgaagtgggcttcccactcggtgtacgcccttatgaattccagtcaccgacgccagttgcttcatagctcccgccgccctcgctctctccccgaggaccccgaagtgtcgcagcttcagggtgaattgcttcatcagttccaatcgcttcacctcccgcttcgtggtggcctcatgccaaatccgctcgctgcgcccttcaggctccttcagcaaagcagctcccttggtcccacttacgcagtcgcccccatcgctcgcgctccccaggtccctctgccctctatggccgacaatgccacccaagtcgggcctgttcctcctcgcgacgaccgcgttgatcgccagcctcctcttcctgatcctcctcgtgtgctcgagacgaccccgtcgcacttcctcgacctccctttccaatggaaggtcacggacttcacaggatacgccgcctaccacggaaccgacgacctgtccgcctccgcggtactgaccacgctctgtgctccgtaccgccacgccgagctcctctatgtcgagatctccgtcgctccgtgtcccccgtcgttctccaagcccatcatgttcaccgtcgtctggacaccggccaccctgtcccccgctgacggcaaggagaccgactactacgggggccgtcagatcactgtgggcgggcctgtcctgttgtccagcaccaccgccgtacccgcagacctggcccgcatgaaccccttcatcaagtccagcgtctcctacaatgacacgccccgctggaccatgtctgtcccccccgtcaccggtggggacaccaagatcccgctcgccactgccttcgttcgcgggatcgtccgcgtgtcagccccctctgggactgccaccccctctgcctgatccatcaaggcagcaataatgcgagaaggaaaactcgcccagccttgagctggtaagctgttaaacctccgcccatccatgtttgcaaaatctaaggtagcaggtcggccataagacctgtgggcc

SEQ ID NO: 14 - DNA, 5612 bp, Maize yellow dwarf virus (MYDV)
acaaaagggttctagagggaccctttatagcactcttctttcaccagaagtttcatgcgctgtgagattcactttgacgggacactcacgtttgctgaaatcccccgtgatctcacaatccgccttttagagtttcaaacagctctaagaaccatcgcttgttgtgttctcaaccaacgatacgatgctgaaactctggtgcgctctgcttttactattctgcctctcatgctccgtgaactcccattcacttgggagttccctagtgcggtacacgccgcctttgcgaagcatgcgttacgtaccgccggcagaatacctcctcccatggaactcatcttccatggtgacacgccaaaacacatgtatagagatttcctataccgcgttgtcacgagagatattgcagctagcctacagagatctcacgagaatttcatctgtggctataaacgcttccaactccggctggaaagtgtttgcagaagagttgagctccttggtgacacatttgcaccaaaacatatcgaggagctttcatggtcttcgcggactcgcggtggacggggtgcaggcgctcgcaggaggcttcctgctcgctgtaatctacacctggagctacttgatatcgctgctcttttgggttgttacaaccctggtatgcagatatacgttccagatgtcatcgatcgcctgtctctacgtctgtacaatgctcttggtccggctggcttcaaagatttttggagggtggccggttatgatcatctcgctgattgggactctgacatcgaagctctttcgggctctgtcattcaaaaagagctcaatctcctttgagatccctaccccagggtacaagacagtagagatacctcagaaaccacccaaagattgcgtcttgctggttcaacacaacgacgctctcaattcccctggaggatacgcatcatgtgttcgactcctcaacggaagcaatgctttgctcactgcaaaacatgtttccacccaggaaggtgatttgctcatcgcttcatccagaactggaaacaggatcaagttgtcattgttcaacacaatcctaaccacaaagaattccgacgtgggtctttatcaaggacctccaggttgggaatcaattcttggatgtaaagctgcagacatcgtaccagtggatgggctctcatgttgtgaggcctccatttataggcatgatggcaactggatgcgttccaacgcatccttggtcggaacagaaggcacttttgtctctgttttgagcaacaccattgagggttttagtggaactccctattttaacggaaaatccattttgggagttcatgtgggaggcaatgaaaccagaactaacaatctgatggcccccatacccagcatcccaggcctaacaaaacacaaatatgtgtttgaatcgccacaactcagaggccgcctgtttacagacgaggaagttgagaaactcgaattcgagattgatgaagctttccagaaagctcataatctcatacatttcaaatctaaaacaggaagaaactgggctgatgatgaggatgacatccactttgaagctccaaagtttcagggaaacgacgcacgcggtcccgtccgcgaaaacaaaacggtctctcccacccctacacactcgcccgtcgttacttcaggcaacgacactctcaacaaggtggtggaagcgttggtctcgaagatcgacgtctcagtaatcgagcggatggttgttcaaaagatctcggaatcagctttgaaacgcccaacgaacaacaatcggaaacacaggcgaaagcccaaaacttctcagcctactttgcctccctctacagatgggaggtacgtggcgcccgctcgcagatccccggcttcgaagcctgcggatccctccccaaatactacttcacaaaacaaaaagaagaatcagagtgggggaggttacttgcagagggaaacccggcgctggcaagtaaagtcagcggcttcgggtggccccaattcggacccgaggccgaattgaagagcctgcgccttcaggcgcagagatggctctcacgcgcggagtttgctaaaatcccgtcatctgaggacagggagcgcgtgatccggaagactgtggaggcatacaaaacttgccaaactcaatgccccaagacttctcaaagcaacctgcttgtgtgggaagactttctcgaagatttcaaacaagcagtgttctccctcgagcccgatgccggtgttggtgttcctttcgtgggatacgaccggcgtacgcaccgtggatggatcgaagatccaacacttctgccagttcttgcccgcatgaccttcgaccgattacataagatgtcgacggttaagtttgagcaacttacagcagaacaattggtgcaacagggcttgtgtgacccgatcagactatttgtcaagggggaacctcacaagcagtcaaagctcgatgaaggccgctaccgcctcattatgagtgtttcgttgctggatcaactggtagcccgggttctgtttcaaaatcagaacaagagggaaattgcactatggcgagccataccctcaaaacccggttttgggttgtctacagacgcccaatcgcgagaatttgtgcagaatctcgcgaaacagtgtggggtcaacacgactgaacttttggcaaattggccaacctacactgttccgactgactgctctggtttcgactggagtgttgcggattggatgctccaggatgatatggaggtccgcaaccgactcactcgcaacaacacagatctcaccaagcgcttgcgcgcttgctggttgaaatgtatatccaattctgtgttgtgcttgagtgatggcactctgctagcccagcgcatagcgggaatccagaaatctggttcttacaacaccagttcgagtaactctcgaatccgagtgatggccgcatatcattgcggtgctacctgggcgatggctatgggtgatgatgcactcgagtcagtcgacacgaacctagacgtgtataaaacactaggattcaaagtcgaggtctccaaacaactggagttttgttctcatatcttcgagaaggaagaccttgctcgcccggttaaccaaaacaagatgatctacaaactcttacatggttacaacccggcgaacggctcttcggaggtgatacagcgttatcttgacgcatgtatgagcgtactcaacgagttgcgccacgaccccgaaaccgttgagcttctgtaccagtggctggtcgctccagtccagaaacaaaaagtttaaaacagaagctctcaagtcagccaggcaaattcgagttgcaagcactggatgacctagtctcgatacataaaccaccacggattacaagttcttagccgggatcactctcggcctttgcatcacattcccatttataatccttggtgtgtacaaagtctaccgtacggtctccaacgatacaagcaaactcgctaatgaatttgggaggccgtagaaatggacgacgtggaacacggttacgcagacgcgtacgcattgctcgcaccacccaaccaatggttgtggtcgcgcaaacccagcgtagacgccgcatccgaagacgaggacgaccaagtggagacacttcaggaggacctcgagggcgaggaggctcgcgggagactttcgtattttcgaaggattctatcgcgggcagtgcctccggaaagctcaccttcggggcgtctctttctgagtgcgcagcattctctggtggaattctcaaggcctaccatgagtataagatcacaaaagtcatactggagttcatctccgaggccccttacaccgcagccggttccatcgcttatgagcttgatccccacaacaagctcagcaccctcgcatcaacaatcaacaaattctcgatcgtcaagggtggcaagcgtgcctatacgtccaaacaaatcggaggtggagtatggcgagattcgtccgaagaccaatttgcaatactctacaagggcagtggaaactcctcagttgccggctcgttccgcatcacgatggaggttcatacccaaaatccgaaataggtagacggagcttcccctgcaccagacccaacaccgacaccaacccccactccaacacctactccaactccaacgcccactcctgtgactcaggaagccttctacggctattctggtgtcccagaatgtaagatccagtccagaaagaactcggaattcatcgatatctattcgttgaatttcgttaaattgttctactggagagatgaggcgtggagctcggagaccctttcggcgggatacatacaaaatgattcgctccgcgcaaccccctaccttttggttccgaccaagaagggaaaatactctgtttatatagagtgtgagggttttcaagcggttaaagctaagggtggtaacaacgacggcaagatgagtggttttgtcacgtatgataaagatcaaagcggttggcaagtgtactcatgggctggttgctctctctcgcagatcaaagttaaagacactggtgtcgtggctcatcccgacatgaaggtgaatggttgctctttcaccaaaggccaacttattgagagagattttatttgttcgttccatctcgaagctacggaagatggatattgggctttgcaagcccccccagtagagaagtctgatgaccacaattttattgtgtcatacggttcttacaccgaaaagattcttgaatggggttcagtatccatatcaatagatgagataaatcgaacagaagctcgcaagattccgaaaagggataaggatctatcacaaagtggacgtttggccgacatgaccaacgtccccacagtgggggtggttgtagcagcgaccacgaaaccggacctgccggtagaacagccaaaccagttggctgtggtggagcaacccactgaagagcaacaaaagaaaagggcgactatcgaccaatggctcgatgccgttgaagctcttgctcccccagaacctgaagggttggtgacacaggtgagactaccaacagcagctgaacgaggtttgacctcgcaaaagctacctttgcaccaacgtggaaccttcaaagacctcgccaaccgagacgctgatacatacagtgtcgcatctcgtggattgactgggggcttgagaggaactcccgcaacacctcaggttgaaacgattgaggagaaccccgtccaagtggacgatgattccaaatctctcgtttcaagctcgtcaaggcttacaggcggtcttcgtcttagaacttcatatcgcatgaccactcaagaggccaagcaatatgatgagatcagacgaagctttggtaaagcacgcgcaaaagcctattatgacgatttgtgtaaggcgaactggtattagcccacacaccctggtcagggtcacagaccactcgccggagtataaacgagataggatggcaacctagccactccccttcctcccgatgggaaatagggtgagttccaagcccaaggaatgagatttcagtgcaatttttccactgaaatctatggt

SEQ ID NO: 15 - DNA, 9515 bp, Maize dwarf mosaic virus (MDMV)
aaaaacaacaagactcaacacaacacaaccaaacacgaccaaacacaaccaaattacacgttattggagcacattcagtttgcaggcaacggttcgtttgcaaggtgcatcgaaaagcctctctgaacacacgatcgcaatggcaggaacttggacccacgttactcacaagtggcagccaaaccttgacaaccctcgtgacgtcaggagaatcatggagctgttcgctgcaaagggccaggtctatgacgagaagcgagctctggagcacaacagtaaattacttcgtagagctcaggtggtggatgtcgaaccaatgatcacggttcaaccaaagaagtgtgcacagatatggaaagaggtggtggatcataatccaacacaccatttcgtgtacgcacgtttctctgaggttaagaagcaacagcctaccaaaccagttgcaacctcagttaataaactagtgagaaagactctagaaatacgagagaattttccagtgaatgttgagtttattggaaagaaacgcaagaacactacgagagtctcactgaggaaagtttttaacaaaactttcttacactgtggcacgcgacatgagaacaaccaattcaagcgagttgacacaaacatcactcgagattggattccagtgctatcaagcgtagcaaaatgttatgcgacactgtcgtctaacatgatgcacaacatacacaaagggcacagtggtctaacgttcattcaaaatggtgaacttttcatagtccgaggaagacttagaggtgaactatgcaatagcttggactgtacaaaggaagttcaggagatagaacactacgcagacccacaggcagctgatttttggaagggatacactaatgcatatgttgagaatagaaatatttcaacgacgcatacagagcatacgcctacaatgaacttagaaaagtgtggcaagcgtatggcgttattggaagttcttttccattcaacgttcaaaatcacatgcaagcattgtaacactgatgatcttgaattatcagatgatgaattcggagaaaaactttacaagaacattcagcgcatcgaagagcaacagagtgaatatctagccgaggaccaaaaactcaaacgggtgttatcattcatcaaggctagatgcacaccaaagtttgatcacttacctatgaattggcaagtcgcagacatcattggacattattcagataatcaagcaaaacaaattttagatgtcaatgaagcactgattaaagtgaacacactcacaccttcagatgcattaaaggcaagtgcagctcttctcgagttatcgagatggtataagaataggaaagaatcaacaaaagaggacaacttatccactttccgcaataagatatctccaaagagcacgattaacttagcattaatgtgcgacaatcaactcgattcaaatggtaactttgtttggggaaagagggaatatcatgcaaaaagattcttctcaaactactttgaagctgtggatccagctgattcatatgaaaaacacgtaacacgctttaatccaaacggacaaagaaaattatctatcggaaaattggttattcctttggacttccaacgtatccgtgattcatttgctggcatacctgtaacaaaacaaccgctttcaaatgcttgtctgagcagaatagacaaaacctacgtctacccttgttgctgtgtaactacagagtttggacaacctgcatactcagaaataatacctccgacaaaggggcatttaaccattggtaattctgtggatccgaagattgtcgatctgccaaacacagaccctccaacgatgtatatttcgaaggacggatattgctatataaacattttcttggcagccatgataaatgttaatgaggattcagctaaggattacacaaaattcatcagagatgaactcatagagagacttggtaaatggcccaaacttaaaaatgtagctactgcatgttatgcactttctgtaatgttcccagagatcaagaacgctgagttacctcaaatcttggttgatcatgaaaataagacaatgcacgttgtggattcatatggatcactaagcgttggctatcacatcttgaaagcgaataccgtgggacaactcatcaaaatgcagtacgagtcgatggaaagcgagatgagagaatatgcagttggtggtacaataacacacaaatcattttccaccttaattagccatctaatcaagaatatgtttaagccacgtgaaatgcggaaaataattgaagaagaacctttcttaattatgctatctgttgtatctcctactgttcttatatctctatataataattgtcacattgagaatgcaatggcgtattggataacgaagaatcaaggagtagcagcaatgttcgcacaattggaagcccttgcaaaagaaacatcaaaggcagagcttttaatccagcagatgacaatattagagaaagcttctaatcagctaaaattggccgtgatgggtctaaatcatgttgacccagctaagcgattgctttggtcacatttagaagtcatgtcgtcgagggcagccacaaataaagatcttctagaccaaggctacgctctatatagcgataggttgtatgccatcatcgaaaaaacctatgtagatcagttgaatcaagcgtggacagaattatcattgtttggaaaattctccgaaacatggcgtgtgtacaaggacaagaaatactacaagccatctttaatcctgcaaagaagcgtagatttaggcgctgtctacaatatatcagttacgcatcaaatatcaagtttagtgcagaaaagtcgcagtcgagtcagctctactttaaccaaactccaccaaggttcatgtgataaactatatagtttgcgtactaaagctataaatacaatttattggtttgttcctgatattttccgacttattcacattttcatagtactaagtttattatcaacagtagctaatactattatagtaacaatgcaagattacaagaaattacaaaaacaagttcgtgaggaagaatatgaaaaggaaataagcgaagtacgcgctatacacgcgaagttgcttaaaatacatgataacgaactcacttgcgaacagttcctgcagtacattaacgaaaatcatccaagattaattgaagcagctgttgaactatcaggagtgggtgtgatacatgagggcaagtccaaccttgaaatcaatctagagcaagcgatggctattggaacactaatcacaatgatatttgaccctacaaagagcgatgctgtatacaaagtattaaacaaaatgagaacaattttgagtacagttgaacaagatgcacctttcccacgcattgatttcacgaatatctttcggtcgcaggtaacccaccaaagtttagatttggacgaccctctcactatcaatactgataagaagcttacggtggatttcgacacaacccaagatcttccagcagatacttttagtaatgatgtgacatttgatcaatggtggtcgaatcaactcgaaaacaatagaactgttccgcactacagacttggtggtgagttcattgaattcacacgagaaaaagcagcatctgttagcatcagtatagcacattcgcaaattgagaaagaatatttactcggaggagcagtcggttcgggaaaatcaacaggtttaccataccatttgagccagcgaggaaaagttcttttattagagccgacacgaccactcgcagaaaacgtctgtagacaactacaaggggcaccgttcaatgtaagtcctacgctacagatgagaggtttgagctcctttggatcaacgcccattacaataatgacatcaggctttgcacttcatatgtacgcaaacaatccagacaaattgtcaaattatgactttgtcattttcgatgaatgtcatattatggaagccccagcaatggccttttactgtttgctaaaggagtacgcatttgatgggaaaataattaaggtctcagccacaccaccaggaagggaatgtgaattctctacgcaacacccagtcgatattcacgtttgcgagaatttaactcaaaaccaattcgtgcttgaacttgggactggatcaaaagctgatgccactaaatacggtaacaacattctggtttacgtggctagctacaacgatgttgattcattggcaagagcattaattgagcgacattattcagtgatcaaagttgatggcagaacgatgaagcagaacacaagtggaatccatccaaacggacatgatggaaagaaatgtttcatagttgccaccaatattatcgaaaacggagtaacattggacgtcgacgtcgttgttgactttggccttaaggttacggctgaattggacgttgataatagagcagtaatgtatcgtaaagtgagcatatcttatggtgagagaatccaacgacttggaagagttggaagaacaaaaccagggactgtcattagaattggaacaaccatgaagggacttcaagagataccagctatgatagcaactgaagcagctttcctttgtttcgcatatggcctcaaggttataacacataacgtttcaactacacacctatcgaaatgcacggttaagcaagcgagaactatgatgccatttgagctttcaccattcattatgtctgaattagtcaaatttgatggctcaatgcatcctcaaatacatgagattctcaagaaatacaagcttagagaatccgtgatcatgttgcgaccaaatgcaattcctcatacaaatgttcacaactggttaacagttaaagactacaacaaaattggctgtgatcttgagctagacgattatgtaaaggttccatacttcataagaggcattcctgagaaagtgtattcagatatctataagattgtactcgaatatggttcgaccagttgttatggaagactatcaagtgcatgtgcaggaaaagtagcttacacattacgcacggacccctttgctttaccacgaacaatcgctattgtgaatcagctcatagctgaggaacacgcaaaacgtgatcattataactcaatcacatcaaacccatcatcttcacatgctttttcccttacaggaatttgcaatatgttagcctcaaggtacatgaaggaccattcaagggaaaacattgagaaattgacacgtgttaaagaccaattgattgagtttagggggactggaggtgagttcaaaaatccagaagatttgcttgaatttggtgggctagttacagtcattcaccaaggcttagattccaccgcccggggtctacagctcaaaggaaggtggaacggagacttgattcagcgcgatttgatgatatcagctggcgttttcacaggcggtctactgatgctttggttcctcttccggaaatggtcatcaacagatgtcaaacatgaagctaagacaaaacgcagcaggcaaaaactcaaatttaggcaagcgcgcgacagcaaatatgcttatgacgttactggatctaaggatgcaattgaagaaaattttggatcagcttatgttaagaaagataagaaaaagggaacaaaagttggattgggagttaagcaacataagttctacatgctgtataattttgatccacaagattacaatctaattcgatttgtggacccacttacaggtgcaactcttgatgagcaaattcacgcagatatcaatatggtacgagaacatttcacagcaattcgagaagctgccataaataatgaccaacttgagtatcaacacatttattcaaatccaggaattaaagcatattttatacgaaatggatctcaaaatgctctcaaagtcgacatgactccacacgaaccactaagggttgttactggtaacaatatagcgggattccctgaatacgaaggcacgctacgacaaaccggaagagcacaagtgataccttcagaacaagtaccagcaccaaacgaggtggaagtggagcacgaagcaaaatctatgttaacgggattggtggattacacacctatagctaatcagattggcataattgaaaatcattcagatgatgttaggctttgcatgtatgctataggatatggatcatacttaatcactcctgcacacctcttcaaagcaagcaatggagagttaacatttcgatcttcgcgaggggtttacaagatgagaaactcagtggaagtaaagctacaccacgtaaaggggcgcgatttggttataattcaactccccaaagattttcctccattcccacagaaactcaagtttcaagcacctaatcgcgaaaacaaagtgtgcttggttggcgtcaatttccagcagaatcattcttcatgtgtagtttctgagagtagcactattgcgccaaaaggaaataatacattttggagtcattggatctcaacaacaggtggccaatgtggtttaccattagttgatatgaaaaccagaagcatagttggggtacatagccttgcatccgtaaatgcgaacgtaaatttcttcgtagcaatgccggaagacttcaacacataccttagtgaacttgtctcgaagaatgaatgggaaaaaggatggcaatataatccaaatttaatatcctggagtggactaaatctcgtatcctctgcacctaaaggcgcttttaaaacagcaaaacttgttgaggatttatcatttgatgttacagaacaagggatccaacatgaaacatggctaacgaagcacatacagcaaaatttgcaagttgtagccaaatgtcctggacaattggttacaaaacatgttgttaaaggtccgtgcccgcactttgcactatacttatccacgcacgaggaagctgagaagttctttagaccgcttatgggcaaatatgataagagtagactcaataaagcagctttcgttaaagatcttacaaaatatgcaaaaccaacttatattggcgaagtaaacactgcactatttgaaagagctgttgagcatgtcatacaactcctacgcaatgttgggattccaacatgtgagtacatcacagatgaagatgaaattttcaaatctttaaacatgaatgctgcggttggagcattatacacaggaaagaagagagaatatttttctgaatacacacaagaggatagagcagagataataaagcaatcgtgcgaaagagtttacgaaggcaagcttggaatttggaatgggtctctcaaggctgaaataagacctatagagaaaacggaagcaaataagacaaggacattcacagccgcaccattggaaacattgctagcgggtaaggtgtgtgtcgatgatttcaataatcaattttatgcacaccacttaaatggaccgtggacagttggaataactaaattctacggtggttggaatagattacttgagaagctaccagatggctggatctactgtgatgcagatggttcgcaactcgacagttcgctcactccttatctgataaatgcagtgctcaacattcgattacaatttatggagccgtggaacattggtgaacaaatgcttaaaaatttatacacggaaattgtttttacaccaattgcaacacctgatgggtcagtcatcaaaaagtttaaaggcaacaatagtggacagccatcaacagttgttggcaacacactaatggtgatcatagcctttaactatacgttgttatcgtgtggagttgacttggagaaggctgatgatgtgtgtcgaatgtatgcgaatggagacgatttattacttgcagtgaacccaacacatgttgacattctaaacgaatttggaaaacacttcgcagcgttagggttaaatttcgattttgaatcacgaacgagagataaatcagaactttggttcatgtcaacgcgaggtatcaagtacgaagaaatgtatatcccaaaattggaaaaagaacgaattgtagctattcttgaatgggatcgatcattaatccctcaataccgtcttgaagctgtctgtgcagcaatggttgaggcatggggatataaagatttgctccatgagatacgtaagttctatgcgtggctgctcgaaatgcaaccttttgctaacttagcaaaggaaggctcagcaccgtacatagccgagacagccctgagaaacttgtatactggtgctaaggtttcagaagatgaattgaatgtctatgcacgacaattcttcgatgatctttcagattatttggccgatgaagttatagatgtcaaacatcaagctggtgagaatgtcgatgctgggcagaagactgaagcacagaaggaagcagagaggaaggcagctgaagagaataaagcaaaggaagctgaggctaaacaaaaggaaaccaaggagaaaacgactgagaaagctggtgatggcgagtccacgggaaaagacaaagacgtggacgccggaacttcaggctcagtatcggtacctaagctaaaagctatgtccaaaaagatgcgtttgccacaagcgaagggaaagaatattctccatcttgacttcctattgaaatacaagccacaacaacaagacttatcgaacacccgagcaaccagggctgaattcgatagatggtatgaagcagtgcagaaagaatacgaacttgatgatacacaaatgacggttgtcatgagtggattaatggtttggtgcattgagaatggttgctcaccaaacatcaatggagtctggacaatgatggatggagacgaacagagaacatttcctttaaaacaggttattggaaatgcatctccaactttcagacaaattatgcatcattttagtgatgcagctgaagcatacattgagtatagaaattcaacagaaagatatatggcgagatatggacttcagcgaaacttaaccgactttagccttgcacgctatgcatttgatttttacgagatatcatctcgaactccagcacgtgcaaaggaagcccacatgcagatgaaggccgcagcagtccgtggttcaaacacacggatgtttggtcttgatgggaatgtcggagaaacccaagaaaatacagaacgccacacagctggcgacgttagtcgcaacatccactcccttttgggagttcagcaggggcattgatacggggttcaacttttacgcagtaatttagtaatatataagtaagctattgtggtgaggttgtacctcgttagttttatatatatattatgctacgtacctactatgtctgcaagtgagtgaggttgcacctcgacacttatagtgggcactattactagcttcgaatcacgagacggacggtccattgagtggttctaccacgaggatgcagcgagtttcgtggtgagagacaaaaaaaaaaaaaaaa

SEQ ID NO: 16 - DNA, 3249 bp, Neisseria meningitidis NmCas9
atggctgccttcaaacctaattcaatcaactacatcctcggcctcgatatcggcatcgcatccgtcggctgggcgatggtagaaattgacgaagaagaaaaccccatccgcctgattgatttgggcgtgcgcgtatttgagcgtgccgaagtaccgaaaacaggcgactcccttgccatggcaaggcgtttggcgcgcagtgttcgccgcctgacccgccgtcgcgcccaccgcctgcttcggacccgccgcctattgaaacgcgaaggcgtattacaagccgccaattttgacgaaaacggcttgattaaatccttaccgaatacaccatggcaacttcgcgcagccgcattagaccgcaaactgacgcctttagagtggtcggcagtcttgttgcatttaatcaaacatcgcggctatttatcgcaacggaaaaacgagggcgaaactgccgataaggagcttggcgctttgcttaaaggcgtagccggcaatgcccatgccttacagacaggcgatttccgcacaccggccgaattggctttaaataaatttgagaaagaaagcggccatatccgcaatcagcgcagcgattattcgcatacgttcagccgcaaagatttacaggcggagctgattttgctgtttgaaaaacaaaaagaatttggcaatccgcatgtttcaggcggccttaaagaaggtattgaaaccctactgatgacgcaacgccctgccctgtccggcgatgccgttcaaaaaatgttggggcattgcaccttcgaaccggcagagccgaaagccgctaaaaacacctacacagccgaacgtttcatctggctgaccaagctgaacaacctgcgtattttagagcaaggcagcgagcggccattgaccgataccgaacgcgccacgcttatggacgagccatacagaaaatccaaactgacttacgcacaagcccgtaagctgctgggtttagaagataccgcctttttcaaaggcttgcgctatggtaaagacaatgccgaagcctcaacattgatggaaatgaaggcctaccatgccatcagccgtgcactggaaaaagaaggattgaaagacaaaaaatccccattaaacctttctcccgaattacaagacgaaatcggcacggcattctccctgttcaaaaccgatgaagacattacaggccgtctgaaagaccgtatacagcccgaaatcttagaagcgctgttgaaacacatcagcttcgataagttcgtccaaatttccttgaaagcattgcgccgaattgtgcctctaatggaacaaggcaaacgttacgatgaagcctgcgccgaaatctacggagaccattacggcaagaagaatacggaagaaaagatttatctgccgccgattcccgccgacgaaatccgcaaccccgtcgtcttgcgcgccttatctcaagcacgtaaggtcattaacggcgtggtacgccgttacggctccccagctcgtatccatattgaaactgcaagggaagtaggtaaatcgtttaaagaccgcaaagaaattgagaaacgccaagaagaaaaccgcaaagaccgggaaaaagccgccgccaaattccgagagtatttccccaattttgtcggagaacccaaatccaaagatattctgaaactgcgcctgtacgagcaacaacacggcaaatgcctgtattcgggcaaagaaatcaacttaggccgtctgaacgaaaaaggctatgtcgaaatcgaccatgccctgccgttctcgcgcacatgggacgacagtttcaacaataaagtactggtattgggcagcgaaaaccaaaacaaaggcaatcaaaccccttacgaatacttcaacggcaaagacaacagccgcgaatggcaggaatttaaagcgcgtgtcgaaaccagccgtttcccgcgcagtaaaaaacaacggattctgctgcaaaaattcgatgaagacggctttaaagaacgcaatctgaacgacacgcgctacgtcaaccgtttcctgtgtcaatttgttgccgaccgtatgcggctgacaggtaaaggcaagaaacgtgtctttgcatccaacggacaaattaccaatctgttgcgcggcttttggggattgcgcaaagtgcgtgcggaaaacgaccgccatcacgccttggacgccgtcgtcgttgcctgctcgaccgttgccatgcagcagaaaattacccgttttgtacgctataaagagatgaacgcgtttgacggtaaaaccatagacaaagaaacaggagaagtgctgcatcaaaaaacacacttcccacaaccttgggaatttttcgcacaagaagtcatgattcgcgtcttcggcaaaccggacggcaaacccgaattcgaagaagccgataccctagaaaaactgcgcacgttgcttgccgaaaaattatcatctcgccccgaagccgtacacgaatacgttacgccactgtttgtttcacgcgcgcccaatcggaagatgagcgggcaagggcatatggagaccgtcaaatccgccaaacgactggacgaaggcgtcagcgtgttgcgcgtaccgctgacacagttaaaactgaaagacttggaaaaaatggtcaatcgggagcgcgaacctaagctatacgaagcactgaaagcacggctggaagcacataaagacgatcctgccaaagcctttgccgagccgttttacaaatacgataaagcaggcaaccgcacccaacaggtaaaagccgtacgcgtagagcaagtacagaaaaccggcgtatgggtgcgcaaccataacggtattgccgacaacgcaaccatggtgcgcgtagatgtgtttgagaaaggcgacaagtattatctggtaccgatttacagttggcaggtagcgaaagggattttgccggatagggctgttgtacaaggaaaagatgaagaagattggcaacttattgatgatagtttcaactttaaattctcattacaccctaatgatttagtcgaggttataacaaaaaaagctagaatgtttggttactttgccagctgccatcgaggcacaggtaatatcaatatacgcattcatgatcttgatcataaaattggcaaaaatggaatactggaaggtatcggcgtcaaaaccgccctttcattccaaaaataccaaattgacgaactgggcaaagaaatcagaccatgccgtctgaaaaaacgcccgcctgtccgttaa

SEQ ID NO: 17 - DNA, 3114 bp, Parvibaculum lavamentivorans
atggagaggattttcggctttgacatcggcacaacaagtatcggattcagcgtgattgattacagtagcacccagtccgcaggcaacatccagaggctgggcgtgcgcattttccctgaggcaagggacccagatgggacccccctgaaccagcagcggagacagaaacgcatgatgaggcgccagctgcgacggagaaggattcgccgaaaggcactgaatgagacactgcacgaagccggctttctgccagcttacgggtctgcagattggcccgtggtcatggccgacgagccttatgaactgcggagaaggggactggaggaaggcctgagtgcttacgagttcggacgggcaatctatcatctggcccagcaccggcattttaaaggcagagaactggaggaatccgatacacccgaccctgatgtggacgatgagaaggaagccgctaacgagagagcagccactctgaaggccctgaaaaatgaacagaccacactgggagcatggctggcccgccgacccccttctgaccgcaagcgaggaatccacgcccataggaacgtggtcgctgaggagttcgagcgcctgtgggaagtgcagtccaagtttcaccccgctctgaaatctgaggaaatgcgggcaagaatcagtgatacaattttcgcccagaggcctgtgttttggcgcaagaacactctgggagagtgcagattcatgcctggcgaaccactgtgtcccaaggggtcctggctgtctcagcagcggagaatgctggagaaactgaacaatctggctatcgcaggcgggaatgctaggccactggatgcagaggaacgcgacgccattctgagtaagctgcagcagcaggccagcatgtcctggccaggcgtgcggtcagctctgaaggcactgtacaaacagagaggcgagcccggggctgaaaagagcctgaaattcaacctggagctgggaggcgaatccaagctgctgggaaatgccctggaggctaaactggcagatatgtttggccctgactggccagctcacccccgaaagcaggagatccggcacgcagtgcatgaacggctgtgggctgcagattacggcgagacacccgacaagaaaagagtcatcattctgtccgagaaggatcgaaaagctcatcgggaagccgctgcaaactctttcgtggcagactttggaattactggcgagcaggcagctcagctgcaggccctgaagctgccaaccggctgggaaccttatagcatcccagcactgaacctgttcctggccgagctggaaaagggggagaggtttggagccctggtgaatggacctgattgggaaggctggaggcgcacaaacttcccccaccgcaatcagcctactggggagatcctggacaagctgccaagtcccgcctcaaaagaggaaagggaacgcattagccagctgcgcaacccaaccgtggtccgaacacagaatgagctgagaaaggtggtcaacaatctgatcgggctgtatggaaaacccgatcgaatccggattgaagtgggccgggacgtcgggaagtccaaaagagaaagggaggaaatccagtctggcattcgacggaacgagaagcagagaaagaaagccactgaagatctgatcaaaaacggaattgctaatcctagccgggacgatgtggagaagtggatcctgtggaaagagggccaggaaagatgcccatacaccggcgaccagattggcttcaatgccctgtttagagaaggcagatatgaggtggaacacatctggcctcgctctcgaagttttgataacagcccaaggaataagacactgtgtcgcaaagacgtgaacatcgagaagggaaataggatgcctttcgaggcatttggccatgacgaagatcggtggagcgccatccagattagactgcagggcatggtgtcagccaaagggggaactgggatgagccccggaaaggtcaaacgcttcctggctaagaccatgcctgaggattttgcagcccggcagctgaacgacacaagatacgctgcaaagcagatcctggcccagctgaaaaggctgtggccagacatgggacctgaggctccagtgaaggtcgaagcagtgactggacaggtcaccgcccagctgcgcaaactgtggactctgaacaatattctggctgacgatggggagaaaaccagagcagatcacaggcaccatgccatcgacgctctgacagtggcctgcactcatcctggaatgaccaacaagctgagcaggtattggcagctgcgcgacgatccacgagcagagaagccagctctgactccaccctgggataccatccgcgccgacgctgagaaagccgtgtctgaaattgtggtcagtcaccgggtgagaaagaaagtcagcggcccactgcataaggagactacctacggcgatacagggactgacattaagaccaaatccggcacatatagacagttcgtgaccaggaagaaaatcgagtcactgagcaagggggagctggatgaaattcgcgacccccgaatcaaagaaattgtggcagctcacgtcgcaggacgaggaggcgaccccaagaaggccttccctccatacccctgtgtgtctcccggaggccctgagatccggaaggtcagactgaccagtaaacagcagctgaacctgatggcccagacagggaatggatacgctgacctgggctccaaccaccatatcgcaatctaccggctgcccgatgggaaggccgacttcgagattgtgtcactgtttgatgctagcagaaggctggcacagagaaatccaatcgtgcagaggacacgagcagacggagccagcttcgtcatgtccctggcagccggagaggccatcatgattcccgaaggctcaaagaaagggatctggattgtgcagggagtctgggcaagcggacaggtggtcctggagagggacaccgatgctgaccactctacaactacccgccctatgccaaaccccatcctgaaggacgatgccaagaaagtgagtatcgatcctattggccgagtccggccatcaaatgactaa

SEQ ID NO: 18 - DNA, 3255 bp, Corynebacterium diphtheriae
atgaagtaccatgtcggaatcgatgtcggaaccttttctgtggggctggctgctattgaagtggatgacgctggaatgcctattaagaccctgagtctggtgtcacacattcatgactcaggactggatcctgacgagatcaagagcgctgtgaccaggctggcaagctccggaatcgcccggagaacaaggcgcctgtaccgacggaagagaaggcgcctgcagcagctggataagttcatccagaggcagggctggccagtgatcgagctggaagattacagcgaccccctgtatccttggaaggtgcgcgccgaactggccgcttcttatattgctgacgagaaggaacggggggagaaactgagtgtggctctgagacacatcgcaaggcatcgcggatggaggaacccttacgccaaggtgtctagtctgtatctgccagatggcccctcagacgccttcaaggctattagggaggaaatcaaacgcgctagcggccagcctgtgccagagactgcaaccgtcgggcagatggtgaccctgtgcgaactgggcacactgaagctgcgaggagagggaggagtgctgagtgcacggctgcagcagtcagattacgcccgcgagatccaggaaatttgtcgaatgcaggagatcggccaggaactgtatcgcaagatcattgacgtggtgttcgcagccgagtccccaaagggctctgcctcaagccgggtggggaaagatcctctgcagccaggaaagaacagagcactgaaagccagcgacgcttttcagcgataccggattgctgcactgatcggcaatctgagagtcagggtggatggggagaagaggattctgagcgtggaggagaagaacctggtgttcgaccacctggtgaatctgactccaaagaaagagcccgaatgggtgaccatcgccgaaattctgggcatcgatcgcgggcagctgatcggaacagctactatgaccgacgatggagagcgagcaggagcccgaccccctacacacgatactaacagaagtattgtgaacagccggatcgcaccactggtcgactggtggaaaacagctagcgcactggagcagcacgccatggtgaaggcactgtccaacgccgaagtcgacgattttgattctcccgagggagcaaaagtgcaggcattctttgccgatctggacgatgacgtccacgccaagctggacagcctgcatctgcctgtgggacgagcagcttactccgaggacactctggtcagactgacccgacggatgctgagtgatggggtggacctgtataccgcccggctgcaggagttcggaattgaacctagctggaccccacccacaccaagaatcggagagcctgtcggcaatccagccgtcgaccgggtgctgaaaacagtgagcagatggctggaatccgcaacaaagacttggggcgccccagagagggtcatcattgagcacgtgcgcgaaggcttcgtcactgagaaacgcgctcgagaaatggatggggacatgagaaggcgcgcagcccggaacgccaagctgtttcaggagatgcaggaaaagctgaatgtgcagggcaaacccagtcgagccgatctgtggagataccagtcagtgcagagacagaactgccagtgtgcctattgcgggtccccaattaccttttctaatagtgaaatggaccacatcgtgcccagagcagggcagggatccaccaacacaagggagaatctggtcgccgtgtgccatcgctgtaaccagtctaagggcaatacacccttcgctatttgggcaaaaaacacttctatcgaaggggtcagtgtgaaggaggccgtggaacggaccagacattgggtcactgataccggcatgagaagcactgacttcaagaagttcaccaaggctgtggtcgagcggtttcagagagcaacaatggatgaggaaatcgacgccagaagcatggaatccgtcgcctggatggctaatgagctgaggagccgcgtggctcagcacttcgcatcccatggaaccacagtcagggtgtaccgaggcagcctgacagcagaggctcgacgggcatctgggatcagtggaaagctgaaattctttgatggcgtggggaagtccaggctggatagaaggcaccatgctattgacgctgcagtgatcgcattcacctctgactatgtggccgaaacactggctgtccgctcaaacctgaaacagagccaggcccaccgacaggaggctcctcagtggagagagttcaccggcaaggatgcagagcatcgagcagcttggagagtgtggtgccagaagatggaaaaactgagcgccctgctgaccgaggacctgcgagatgaccgggtggtcgtgatgtctaacgtgcgactgcggctgggaaatggcagtgcccacaaggaaaccattggcaaactgtcaaaggtgaaactgtcctctcagctgtcagtcagcgatatcgacaaagcaagttcagaggccctgtggtgtgctctgaccagagagcccggattcgatcctaaggaaggcctgcccgctaaccctgagagacacatcagggtgaatgggacacatgtctacgccggggacaatattggactgtttccagtgtcagcaggaagcatcgcactgaggggaggatacgcagagctgggcagctccttccaccatgctcgcgtgtataaaattacttccggcaagaaacccgcatttgccatgctgagggtgtacaccatcgatctgctgccttatcgcaaccaggacctgtttagcgtggaactgaagccacagacaatgtccatgaggcaggctgagaagaaactgcgcgacgctctggcaactgggaatgcagaatatctgggatggctggtcgtggatgacgagctggtcgtggatacatctaagattgccactgaccaggtcaaagcagtggaggccgaactggggactatccgccgatggcgggtggatggattcttttccccctctaaactgagactgaggcctctgcagatgtccaaggaggggatcaagaaagagtccgctcccgaactgtctaaaatcattgacagaccaggatggctgcccgccgtgaacaagctgttctctgatggaaatgtcaccgtcgtgcggagagactctctgggacgcgtgcgactggagagtacagcccacctgcctgtcacttggaaggtgcagtaa

SEQ ID NO: 19 - DNA, 3393 bp, Streptococcus pasteurianus
atgactaacggcaagattctggggctggacattggcatcgcaagcgtgggggtggggattattgaggcaaaaactggaaaggtggtgcatgccaattcccggctgttctctgccgctaacgctgagaacaatgcagaacggagagggtttaggggatctaggcgcctgaatcgacggaagaaacaccgcgtgaagcgagtccgggatctgttcgagaaatacggaatcgtcaccgactttcgcaacctgaatctgaacccttatgagctgcgagtgaagggcctgaccgaacagctgaaaaacgaggaactgttcgcagccctgagaacaatctctaagagaagggggattagttacctggacgatgccgaggacgatagtaccggatcaacagactatgctaagagcatcgatgagaatcgccgactgctgaaaaacaagacaccaggccagattcagctggagaggctggaaaagtacggccagctgcgcgggaatttcaccgtctatgacgagaacggggaagcccatcgcctgatcaatgtgtttagtacatcagattacgagaaagaagcacggaagatcctggagacacaggccgactacaacaagaaaatcacagctgagttcattgacgattatgtggaaatcctgacccagaaacgaaagtactatcacggccccgggaacgaaaagagccggactgactacggacggttccggaccgatgggaccacactggagaatattttcggaatcctgattggcaagtgcaacttttaccctgatgaatatcgagcaagcaaggccagctacaccgcacaggagtataatttcctgaacgacctgaacaatctgaaggtgagcaccgaaacagggaagctgtcaacagagcagaaagaaagcctggtggagtttgccaagaatactgctaccctgggacccgctaaactgctgaaggagatcgcaaaaattctggactgtaaggtggatgagatcaaaggatacagagaggacgataaaggcaagccagatctgcataccttcgagccctataggaaactgaagtttaatctggaaagcatcaacattgacgatctgtcccgcgaagtgatcgacaagctggctgatattctgactctgaacaccgagagagaaggaatcgaggacgcaattaagaggaatctgccaaaccagttcacagaggaacagatcagcgagatcatcaaggtgcggaagagccagtccactgctttcaataagggctggcactcttttagtgcaaaactgatgaacgagctgatccccgaactgtacgccacctccgacgagcagatgacaattctgactcggctggaaaaattcaaggtcaataagaaaagctccaaaaacacaaagactatcgacgagaaggaagtcactgatgagatctacaatcctgtggtcgccaagagcgtgagacagaccatcaaaatcattaacgctgcagtcaagaaatatggcgacttcgataagatcgtgattgaaatgccacgggataaaaatgctgacgatgagaagaagttcatcgacaagagaaataaggagaacaagaaggaaaaggacgatgccctgaaaagggccgcttacctgtataattctagtgacaagctgcccgatgaggtgttccacggcaacaagcagctggaaaccaaaatccgactgtggtatcagcagggggagcggtgcctgtatagtggaaagcccatctcaattcaggagctggtgcataactctaacaatttcgaaatcgatcacattctgcctctgtcactgagctttgacgatagtctggccaataaggtgctggtctacgcttggacaaaccaggagaaaggccagaaaaccccttatcaggtcatcgactccatggatgcagcctggtctttcagggagatgaaggactacgtgctgaaacagaagggactgggcaagaaaaagcgcgactatctgctgactaccgagaacatcgataagattgaagtgaagaagaagttcatcgagaggaatctggtggatactcgctacgcatctcgagtggtcctgaactctctgcagagtgccctgagagagctggggaaagacactaaggtgtctgtggtcaggggacagttcaccagtcagctgcggagaaaatggaagatcgataagagccgcgagacataccaccatcacgcagtggacgccctgatcattgctgcatcaagccagctgaaactgtgggagaagcaggacaatcccatgtttgtggattatggcaagaaccaggtggtcgacaaacagactggggagatcctgtccgtgtctgacgatgagtacaaggaactggtgttccagcccccttatcagggctttgtgaataccatctcctctaaagggttcgaggacgaaattctgtttagctaccaggtggattccaaatataaccggaaggtcagtgacgcaaccatctactcaacaagaaaagccaagattggcaaggataagaaagaggaaacctacgtgctgggaaaaatcaaggacatctactcccagaatggcttcgataccttcatcaagaagtacaacaaagataagactcagttcctgatgtatcagaaggactctctgacatgggagaacgtgatcgaagtcattctgagggactacccaacaactaagaaaagcgaggacggcaaaaatgatgtgaagtgcaacccctttgaggaatacaggcgcgagaatgggctgatctgtaagtattccaagaaagggaaaggaactcccatcaagagcctgaagtactatgacaagaaactggggaactgcatcgatattaccccagaggaatcacgcaataaggtcatcctgcagagcattaacccttggcgagccgacgtgtacttcaatccagagacactgaagtacgaactgatgggcctgaaatattcagatctgagctttgaaaagggcactgggaactaccatatcagccaggagaaatatgacgctatcaaagagaaggaaggaattggcaagaaatccgagttcaagtttacactgtaccgcaacgacctgatcctgatcaaggatatcgccagtggcgagcaggaaatctacagattcctgtcaagaactatgcccaatgtgaaccactacgtcgagctgaagccttacgacaaggaaaagttcgataacgtgcaggagctggtcgaagcactgggagaggcagataaagtgggacgatgtatcaaaggactgaataagccaaacatcagcatctacaaggtgagaaccgacgtcctgggaaacaaatatttcgtgaagaaaaagggcgacaaacccaagctggattttaagaacaacaagaagtaa

SEQ ID NO: 20 - DNA, 3249 bp, Neisseria cinerea
atggctgccttcaaacctaatcctatgaactacatcctgggcctggacattggaatcgcttctgtcgggtgggctatcgtggaaatcgacgaggaagagaaccctatcagactgattgatctgggagtcagagtgtttgaaagggcagaggtgccaaagaccggcgactccctggccgctgcacggagactggctcggtctgtcaggcgcctgacacgacggagagcacacaggctgctgcgagctaggcgcctgctgaagagagagggcgtgctgcaggccgctgacttcgatgaaaacggcctgatcaagagcctgcccaatactccttggcagctgagagcagccgctctggacaggaagctgaccccactggagtggtctgccgtgctgctgcacctgatcaagcatcgcggctacctgagtcagcgaaaaaatgaaggggagacagcagataaggagctgggagcactgctgaaaggagtggccgacaacactcatgctctgcagaccggcgattttaggacacccgctgagctggcactgaataagttcgaaaaagagagtggacacattcgaaaccagcggggcgactattcacataccttcaaccgcaaggatctgcaggccgagctgaatctgctgtttgaaaagcagaaagagttcgggaatccccacgtgtccgacgggctgaaagaaggaatcgagacactgctgatgactcagaggcctgcactgtctggcgatgccgtgcagaagatgctggggcattgcacctttgaaccaacagagcccaaggcagccaaaaacacctacacagccgagaggttcgtgtggctgacaaagctgaacaatctgcgcatcctggaacagggcagtgagcggcccctgactgacaccgaaagagccacactgatggatgagccttacaggaagtctaaactgacttatgcccaggctcgcaagctgctggacctggacgatactgccttctttaagggcctgaggtacgggaaagataatgcagaagccagcaccctgatggagatgaaggcctatcacgctatctcccgcgccctggaaaaagagggcctgaaggacaagaaatctcccctgaacctgagtcctgaactgcaggatgagattgggaccgcttttagcctgttcaagactgacgaggatatcaccggacgcctgaaagaccgagtgcagcccgaaattctggaggcactgctgaagcacatcagttttgataaattcgtgcagatttcactgaaggccctgcgacggatcgtccctctgatggagcagggcaatcggtacgacgaggcctgcaccgagatctacggagatcattatggcaagaaaaacacagaagagaaaatctatctgccccctattcctgccgacgagatccggaatccagtggtcctgagagctctgtcacaggcaagaaaagtgatcaacggagtggtcagaaggtacggcagccctgctaggatccacattgaaaccgcacgcgaagtgggaaagtcctttaaagaccgcaaggaaatcgagaagcgacaggaagagaatagaaaagatagggaaaagtctgctgcaaaattcagggagtactttccaaacttcgtgggcgaacccaagagtaaagacatcctgaagctgcgcctgtacgagcagcagcacgggaagtgtctgtatagcggaaaagaaattaacctgggccggctgaatgaaaagggctatgtggagatcgatcatgcactgcccttttccagaacatgggacgattctttcaacaataaggtcctggctctggggagcgagaaccagaacaagggaaatcagactccttacgaatatttcaacgggaaggacaatagccgagaatggcaggagtttaaagcccgcgtggagacaagccggttcccacgaagcaagaaacagcggattctgctgcagaagtttgacgaagatggattcaaagagagaaacctgaatgacacccggtacatcaacagatttctgtgccagttcgtggctgatcacatgctgctgaccggaaagggcaaacgccgagtctttgcaagcaacggccagatcacaaatctgctgaggggcttctgggggctgcggaaggtgagagccgagaatgaccgccaccatgcactggatgccgtggtcgtggcttgttccactattgcaatgcagcagaagatcaccaggtttgtgcgctataaagagatgaacgccttcgacggaaagacaattgataaagaaactggcgaggtgctgcaccagaaggcacattttcctcagccatgggagttcttcgcccaggaagtgatgatccgggtctttgggaagcctgacggaaaaccagagttcgaagaggccgataccccagaaaagctgcggacactgctggctgaaaaactgagctccagacccgaggcagtgcacaagtacgtcacccccctgttcattagcagggcccctaatcgcaaaatgtccgggcagggacatatggagactgtgaaatcagctaagcggctggacgaaggcatcagcgtgctgagagtcccactgacccagctgaagctgaaagatctggagaagatggtgaaccgggaaagagagcccaagctgtatgaagctctgaaagcaagactggaggcccacaaggacgatccagctaaagcatttgccgagcccttctacaaatatgacaaggccggcaatcggacacagcaggtgaaggctgtcagagtggagcaggtccagaaaactggggtctgggtgcacaaccataatggaattgccgacaacgctacaatcgtccgggtggatgtgttcgagaaaggcgggaagtactatctggtgcctatctactcctggcaggtcgccaagggaatcctgccagatagagctgtcgtgcagggcaaagacgaagaggattggactgtgatggacgattctttcgagtttaagttcgtcctgtacgcaaacgacctgatcaagctgacagccaagaaaaatgaatttctggggtatttcgtgtcactgaacagggcaactggagccatcgatattcgcacacatgacactgatagcaccaagggaaaaaacggcatctttcagtctgtgggcgtcaagaccgccctgagtttccagaaatatcagattgacgaactggggaaggagatccgaccctgtcggctgaagaaacgaccacccgtgcggtaa

SEQ ID NO: 21 - DNA, 3294 bp, Staphylococcus aureus
aagcggaactacatcctgggcctggacatcggcatcaccagcgtgggctacggcatcatcgactacgagacacgggacgtgatcgatgccggcgtgcggctgttcaaagaggccaacgtggaaaacaacgagggcaggcggagcaagagaggcgccagaaggctgaagcggcggaggcggcatagaatccagagagtgaagaagctgctgttcgactacaacctgctgaccgaccacagcgagctgagcggcatcaacccctacgaggccagagtgaagggcctgagccagaagctgagcgaggaagagttctctgccgccctgctgcacctggccaagagaagaggcgtgcacaacgtgaacgaggtggaagaggacaccggcaacgagctgtccaccaaagagcagatcagccggaacagcaaggccctggaagagaaatacgtggccgaactgcagctggaacggctgaagaaagacggcgaagtgcggggcagcatcaacagattcaagaccagcgactacgtgaaagaagccaaacagctgctgaaggtgcagaaggcctaccaccagctggaccagagcttcatcgacacctacatcgacctgctggaaacccggcggacctactatgagggacctggcgagggcagccccttcggctggaaggacatcaaagaatggtacgagatgctgatgggccactgcacctacttccccgaggaactgcggagcgtgaagtacgcctacaacgccgacctgtacaacgccctgaacgacctgaacaatctcgtgatcaccagggacgagaacgagaagctggaatattacgagaagttccagatcatcgagaacgtgttcaagcagaagaagaagcccaccctgaagcagatcgccaaagaaatcctcgtgaacgaagaggatattaagggctacagagtgaccagcaccggcaagcccgagttcaccaacctgaaggtgtaccacgacatcaaggacattaccgcccggaaagagattattgagaacgccgagctgctggatcagattgccaagatcctgaccatctaccagagcagcgaggacatccaggaagaactgaccaatctgaactccgagctgacccaggaagagatcgagcagatctctaatctgaagggctataccggcacccacaacctgagcctgaaggccatcaacctgatcctggacgagctgtggcacaccaacgacaaccagatcgctatcttcaaccggctgaagctggtgcccaagaaggtggacctgtcccagcagaaagagatccccaccaccctggtggacgacttcatcctgagccccgtcgtgaagagaagcttcatccagagcatcaaagtgatcaacgccatcatcaagaagtacggcctgcccaacgacatcattatcgagctggcccgcgagaagaactccaaggacgcccagaaaatgatcaacgagatgcagaagcggaaccggcagaccaacgagcggatcgaggaaatcatccggaccaccggcaaagagaacgccaagtacctgatcgagaagatcaagctgcacgacatgcaggaaggcaagtgcctgtacagcctggaagccatccctctggaagatctgctgaacaaccccttcaactatgaggtggaccacatcatccccagaagcgtgtccttcgacaacagcttcaacaacaaggtgctcgtgaagcaggaagaaaacagcaagaagggcaaccggaccccattccagtacctgagcagcagcgacagcaagatcagctacgaaaccttcaagaagcacatcctgaatctggccaagggcaagggcagaatcagcaagaccaagaaagagtatctgctggaagaacgggacatcaacaggttctccgtgcagaaagacttcatcaaccggaacctggtggataccagatacgccaccagaggcctgatgaacctgctgcggagctacttcagagtgaacaacctggacgtgaaagtgaagtccatcaatggcggcttcaccagctttctgcggcggaagtggaagtttaagaaagagcggaacaaggggtacaagcaccacgccgaggacgccctgatcattgccaacgccgatttcatcttcaaagagtggaagaaactggacaaggccaaaaaagtgatggaaaaccagatgttcgaggaaaagcaggccgagagcatgcccgagatcgaaaccgagcaggagtacaaagagatcttcatcaccccccaccagatcaagcacattaaggacttcaaggactacaagtacagccaccgggtggacaagaagcctaatagagagctgattaacgacaccctgtactccacccggaaggacgacaagggcaacaccctgatcgtgaacaatctgaacggcctgtacgacaaggacaatgacaagctgaaaaagctgatcaacaagagccccgaaaagctgctgatgtaccaccacgacccccagacctaccagaaactgaagctgattatggaacagtacggcgacgagaagaatcccctgtacaagtactacgaggaaaccgggaactacctgaccaagtactccaaaaaggacaacggccccgtgatcaagaagattaagtattacggcaacaaactgaacgcccatctggacatcaccgacgactaccccaacagcagaaacaaggtcgtgaagctgtccctgaagccctacagattcgacgtgtacctggacaatggcgtgtacaagttcgtgaccgtgaagaatctggatgtgatcaaaaaagaaaactactacgaagtgaatagcaagtgctatgaggaagctaagaagctgaagaagatcagcaaccaggccgagtttatcgcctccttctacaacaacgatctgatcaagatcaacggcgagctgtatagagtgatcggcgtgaacaacgacctgctgaaccggatcgaagtgaacatgatcgacatcacctaccgcgagtacctggaaaacatgaacgacaagaggccccccaggatcattaagacaatcgcctccaagacccagagcattaagaagtacagcacagacattctgggcaacctgtatgaagtgaaatctaagaagcaccctcagatcatcaaaaagggcaaaaggccggcggccacgaaaaaggccggccaggcaaaaaagaaaaagggatcctacccatacgatgttccagattacgcttacccatacgatgttccagattacgcttacccatacgatgttccagattacgcttaa

SEQ ID NO: 22 - DNA, 3012 bp, Campylobacter lari
atgaggattctggggtttgacattggcattaacagcatcgggtgggcttttgtggagaacgacgaactgaaggactgcggagtgcggatcttcacaaaggccgagaacccaaaaaataaggaaagcctggcactgccccggagaaatgcacgcagctccaggcgccgactgaaacggagaaaggcccggctgatcgctattaagagaatcctggccaaagagctgaagctgaactacaaggactatgtcgcagctgatggagagctgccaaaggcctacgaaggatccctggcatctgtgtacgagctgcggtataaggccctgacacagaacctggaaactaaagatctggccagagtgatcctgcacattgctaagcatagggggtacatgaacaagaacgagaagaaatcaaacgacgctaagaaaggaaagatcctgagcgctctgaaaaacaatgcactgaagctggagaactaccagagcgtgggcgaatacttctacaaggagttctttcagaaatacaagaaaaacacaaagaacttcatcaagatccgcaacactaaggataattacaacaattgcgtgctgtctagtgacctggaaaaagagctgaagctgatcctggaaaaacagaaggagttcggctacaactactctgaagatttcatcaacgagattctgaaggtcgccttctttcagcggcccctgaaggacttcagtcacctggtgggggcctgcactttctttgaggaagagaaaagggcctgtaagaacagctactctgcctgggagtttgtggctctgaccaagatcattaacgagatcaagagcctggagaagatcagcggcgaaattgtgccaacccagacaatcaacgaggtcctgaatctgatcctggacaaggggtctatcacctacaagaaattcagaagttgtatcaatctgcatgagagtatcagcttcaagagcctgaagtatgataaagaaaacgccgagaatgctaaactgatcgacttccgcaagctggtggagtttaagaaagccctgggagtccacagcctgtcccggcaggaactggatcagatctccactcatatcaccctgattaaggacaacgtgaagctgaaaaccgtcctggagaaatacaacctgagtaatgaacagatcaacaatctgctggaaattgagttcaacgattatatcaacctgagcttcaaggccctgggaatgattctgccactgatgcgcgagggcaaacgatacgacgaggcctgcgagatcgccaatctgaaacctaagaccgtggacgagaagaaagatttcctgccagcattttgtgattccattttcgcccacgagctgtctaaccccgtggtcaatagggctatcagcgaataccgcaaggtgctgaacgcactgctgaagaaatatggaaaggtccacaaaattcatctggagctggctcgcgacgtgggcctgtccaagaaagcacgagagaagatcgaaaaagagcagaaggaaaaccaggccgtgaatgcatgggccctgaaggaatgcgagaatattggcctgaaggccagcgcaaagaacatcctgaaactgaagctgtggaaagaacagaaggagatctgtatctactccggaaataagatctctattgagcacctgaaagatgaaaaggccctggaggtggaccatatctacccctattctaggagtttcgacgattcttttatcaacaaagtgctggtgttcaccaaggaaaatcaggagaaactgaacaagacacctttcgaggcctttggcaagaatattgaaaaatggagcaagatccagaccctggctcagaacctgccatacaagaaaaagaataagattctggacgagaacttcaaagataagcagcaggaggactttatctctcgaaatctgaacgacacccggtatatcgctacactgattgcaaaatacacaaaggagtatctgaacttcctgctgctgagcgaaaatgagaacgccaatctgaagagtggcgaaaaagggtcaaagatccacgtgcagactattagcgggatgctgacctccgtcctgaggcacacatgggggtttgacaaaaaggatcgcaacaatcatctgcaccatgcactggatgccatcattgtggcctacagtacaaattcaatcattaaggctttcagcgatttccggaaaaaccaggagctgctgaaggccagattctacgctaaagaactgacttccgataactataaacatcaggtcaagttctttgagcctttcaagagttttagagaaaaaatcctgtcaaagatcgacgagattttcgtgtccaaaccacctcgaaagcgagctaggcgcgcactgcacaaggatacctttcattctgagaacaagatcattgacaagtgcagctacaactccaaggaaggcctgcagattgccctgagctgtggaagagtgaggaaaatcggcactaagtatgtcgagaatgataccatcgtgagggtcgacattttcaaaaagcagaacaagttttacgctatcccaatctacgcaatggattttgccctggggatcctgcccaataagatcgtgattactggaaaagataagaacaataaccccaaacagtggcagaccattgacgaatcatacgagttctgctttagcctgtataagaatgacctgatcctgctgcagaaaaagaacatgcaggaacctgagttcgcctactataacgatttttcaatcagcacatcaagcatttgtgtggagaaacacgacaacaagttcgaaaatctgactagcaaccagaagctgctgttttccaatgcaaaagagggctctgtgaaggtcgaaagtctggggatccagaacctgaaagtgttcgagaagtacatcattacccccctgggagataaaattaaggctgactttcagcctcgagaaaacatcagcctgaaaaccagtaaaaagtatggcctgaggtaa

SEQ ID NO: 23 - DNA, 16386 bp, Artificial Sequence
  Vektor1_TaU6
  misc_feature (16239)..(16258): n is a, c, g, or t
ttgtacaaagtggttcgataattccgatccagcctaggcccgggcctgaggacgcgccttactagtggatcccttcaccgccattgcaaaaattgtcaataaatatttagagtgggtggcatcagaaaaacatctctagtggactctcttcctatcatagctactcgggctgtagatagaacgagggcacaagagttgggtggcgtaggtttactcgtgacctcaactcttttggctgtgtcttacgtctaagatgggtttggcatgtgagaaacataggtctaagcaattcatgttagggctgttgcattgttgttgcatcaaccaaatgtccagatagcagttcatgctacatctagttgaaaaccctcatcattaggcggaacatgtgttcttttttagcatagtcaaagtcagattgcggcactcgctcatccacggaaagaattttccctgtgcaggcatctcgatcaaaagacgcaaattaatttttgaatagcgatataacaatatctaattaacgtttcttgttttctgcgaaatgtctttcatcataaaatgagtcatctcgatgagcccaagtgacatagcccaacaccccaccccaccaataaaagtgaagaaaacatgttgggaaaactataccaagtaaaatacgagttgttctaaagaaaaagtaaagtacgagttagatcgcaccctgtcctggagtgtggcttgatgatccaactcctagcattgtatccctgtttttggatgatgtaactattatttacaatgaataaagaggtgttttactagtaaaaaaatcttgaggggaggagaaaataatggaggtcttttttcaaaccgatggactattatttttagtgaaagagaataatattattggaaaaattattctatccacttattttatattggcagaatacaaagaatggtggggtccacgcggaacttgcggcccccgaaacctatcgagggcgcggtacccaagcaaggaacggaggaaacttgcggggcccgaaacctagtgataaaaggcatatcatccacacgatgaagatctgacggaccatatctcccaccacggaaagccatcagacgaggatcagacggccaggaaggaaccctagcgcccgccggtgccaatataaagcgccactctctctcgtcttaagccccagcctctccattcccctctccctctcgattacgaggtgtgttgttcatccgtcccgaatccatccatcccctcttcagatgtgttgttcatggctctaatagctctagatctgcttgtttgtgttgtttagctctagatctactcgcgcgcgcttctctctcgatctcctgtagaacaattttggttggttttttgtgcatatccatggtaattttgtctgcaatatggaggaggctttctaagctcctacgtagcatcgatctttagaattccctcggtttctgtttatttcttcgcgagggctctctgttatctgtaggagtagctgtaagcgcggttcgttacggattaatcgtcatgcttagttgaacctatcggtcgaaggatttgtgtgggttgtcgtgtagaattgacaccatctacttactgtactgatatgccgatctgtaggatactcttcattacttttgtttactgctagttgtggtgtagatttagcattctcaaacccatgctgtagcgtttctaatattgttacatagatctaccggtgcctgttaattgtattcgatcgggcgtttctacatctgtccgcccacctagttttatatgtggtaatcaaaattgcgttgacttcgtgatgctgtctgtgtactgtttttaatcgctcttacttagatgatcaacatggtgatggttacgatttactgttttctaatccctgttacttcgatgctgcagtttgattgatgggcccagaacgacgcccggccgacatccgccgtgccaccgaggcggacatgccggcggtctgcaccatcgtcaaccactacatcgagacaagcacggtcaacttccgtaccgagccgcaggaaccgcaggagtggacggacgacctcgtccgtctgcgggagcgctatccctggctcgtcgccgaggtggacggcgaggtcgccggcatcgcctacgcgggcccctggaaggcacgcaacgcctacgactggacggccgagtcgaccgtgtacgtctccccccgccaccagcggacgggactgggctccacgctctacacccacctgctgaagtccctggaggcacagggcttcaagagcgtggtcgctgtcatcgggctgcccaacgacccgagcgtgcgcatgcacgaggcgctcggatatgccccccgcggcatgctgcgggcggccggcttcaagcacgggaactggcatgacgtgggtttctggcagctggacttcagcctgccggtaccgccccgtccggtcctgcccgtcaccgagatctgaatgccgaatttccccgatcgttcaaacatttggcaataaagtttcttaagattgaatcctgttgccggtcttgcgatgattatcatataatttctgttgaattacgttaagcatgtaataattaacatgtaatgcatgacgttatttatgagatgggtttttatgattagagtcccgcaattatacatttaatacgcgatagaaaacaaaatatagcgcgcaaactaggataaattatcgcgcgcggtgtcatctatgttactagatcgctcgaagatcccccgggctgcaggaattcaagcttggcactggccgtcgttttacaacgtcgtgactgggaaaaccctggcgttacccaacttaatcgccttgcagcacatccccctttcgccagctggcgtaatagcgaagaggcccgcaccgatcgcccttcccaacagttgcgcagcctgaatggcgaatgagcttgagcttggatcagattgtcgtttcccgccttcagtttaaactatcagtgtttgacaggatatattggcgggtaaacctaagagaaaagagcgtttattagaataacggatatttaaaagggcgtgaaaaggtttatccgttcgtccatttgtatgtgcatgccaaccacagggttcccctcgggatcaaagtactttgatccaacccctccgctgctatagtgcagtcggcttctgacgttcagtgcagccgtcttctgaaaacgacatgtcgcacaagtcctaagttacgcgacaggctgccgccctgcccttttcctggcgttttcttgtcgcgtgttttagtcgcataaagtagaatacttgcgactagaaccggagacattacgccatgaacaagagcgccgccgctggcctgctgggctatgcccgcgtcagcaccgacgaccaggacttgaccaaccaacgggccgaactgcacgcggccggctgcaccaagctgttttccgagaagatcaccggcaccaggcgcgaccgcccggagctggccaggatgcttgaccacctacgccctggcgacgttgtgacagtgaccaggctagaccgcctggcccgcagcacccgcgacctactggacattgccgagcgcatccaggaggccggcgcgggcctgcgtagcctggcagagccgtgggccgacaccaccacgccggccggccgcatggtgttgaccgtgttcgccggcattgccgagttcgagcgttccctaatcatcgaccgcacccggagcgggcgcgaggccgccaaggcccgaggcgtgaagtttggcccccgccctaccctcaccccggcacagatcgcgcacgcccgcgagctgatcgaccaggaaggccgcaccgtgaaagaggcggctgcactgcttggcgtgcatcgctcgaccctgtaccgcgcacttgagcgcagcgaggaagtgacgcccaccgaggccaggcggcgcggtgccttccgtgaggacgcattgaccgaggccgacgccctggcggccgccgagaatgaacgccaagaggaacaagcatgaaaccgcaccaggacggccaggacgaaccgtttttcattaccgaagagatcgaggcggagatgatcgcggccgggtacgtgttcgagccgcccgcgcacgtctcaaccgtgcggctgcatgaaatcctggccggtttgtctgatgccaagctggcggcctggccggccagcttggccgctgaagaaaccgagcgccgccgtctaaaaaggtgatgtgtatttgagtaaaacagcttgcgtcatgcggtcgctgcgtatatgatgcgatgagtaaataaacaaatacgcaaggggaacgcatgaaggttatcgctgtacttaaccagaaaggcgggtcaggcaagacgaccatcgcaacccatctagcccgcgccctgcaactcgccggggccgatgttctgttagtcgattccgatccccagggcagtgcccgcgattgggcggccgtgcgggaagatcaaccgctaaccgttgtcggcatcgaccgcccgacgattgaccgcgacgtgaaggccatcggccggcgcgacttcgtagtgatcgacggagcgccccaggcggcggacttggctgtgtccgcgatcaaggcagccgacttcgtgctgattccggtgcagccaagcccttacgacatatgggccaccgccgacctggtggagctggttaagcagcgcattgaggtcacggatggaaggctacaagcggcctttgtcgtgtcgcgggcgatcaaaggcacgcgcatcggcggtgaggttgccgaggcgctggccgggtacgagctgcccattcttgagtcccgtatcacgcagcgcgtgagctacccaggcactgccgccgccggcacaaccgttcttgaatcagaacccgagggcgacgctgcccgcgaggtccaggcgctggccgctgaaattaaatcaaaactcatttgagttaatgaggtaaagagaaaatgagcaaaagcacaaacacgctaagtgccggccgtccgagcgcacgcagcagcaaggctgcaacgttggccagcctggcagacacgccagccatgaagcgggtcaactttcagttgccggcggaggatcacaccaagctgaagatgtacgcggtacgccaaggcaagaccattaccgagctgctatctgaatacatcgcgcagctaccagagtaaatgagcaaatgaataaatgagtagatgaattttagcggctaaaggaggcggcatggaaaatcaagaacaaccaggcaccgacgccgtggaatgccccatgtgtggaggaacgggcggttggccaggcgtaagcggctgggttgtctgccggccctgcaatggcactggaacccccaagcccgaggaatcggcgtgacggtcgcaaaccatccggcccggtacaaatcggcgcggcgctgggtgatgacctggtggagaagttgaaggccgcgcaggccgcccagcggcaacgcatcgaggcagaagcacgccccggtgaatcgtggcaagcggccgctgatcgaatccgcaaagaatcccggcaaccgccggcagccggtgcgccgtcgattaggaagccgcccaagggcgacgagcaaccagattttttcgttccgatgctctatgacgtgggcacccgcgatagtcgcagcatcatggacgtggccgttttccgtctgtcgaagcgtgaccgacgagctggcgaggtgatccgctacgagcttccagacgggcacgtagaggtttccgcagggccggccggcatggccagtgtgtgggattacgacctggtactgatggcggtttcccatctaaccgaatccatgaaccgataccgggaagggaagggagacaagcccggccgcgtgttccgtccacacgttgcggacgtactcaagttctgccggcgagccgatggcggaaagcagaaagacgacctggtagaaacctgcattcggttaaacaccacgcacgttgccatgcagcgtacgaagaaggccaagaacggccgcctggtgacggtatccgagggtgaagccttgattagccgctacaagatcgtaaagagcgaaaccgggcggccggagtacatcgagatcgagctagctgattggatgtaccgcgagatcacagaaggcaagaacccggacgtgctgacggttcaccccgattactttttgatcgatcccggcatcggccgttttctctaccgcctggcacgccgcgccgcaggcaaggcagaagccagatggttgttcaagacgatctacgaacgcagtggcagcgccggagagttcaagaagttctgtttcaccgtgcgcaagctgatcgggtcaaatgacctgccggagtacgatttgaaggaggaggcggggcaggctggcccgatcctagtcatgcgctaccgcaacctgatcgagggcgaagcatccgccggttcctaatgtacggagcagatgctagggcaaattgccctagcaggggaaaaaggtcgaaaaggtctctttcctgtggatagcacgtacattgggaacccaaagccgtacattgggaaccggaacccgtacattgggaacccaaagccgtacattgggaaccggtcacacatgtaagtgactgatataaaagagaaaaaaggcgatttttccgcctaaaactctttaaaacttattaaaactcttaaaacccgcctggcctgtgcataactgtctggccagcgcacagccgaagagctgcaaaaagcgcctacccttcggtcgctgcgctccctacgccccgccgcttcgcgtcggcctatcgcggccgctggccgctcaaaaatggctggcctacggccaggcaatctaccagggcgcggacaagccgcgccgtcgccactcgaccgccggcgcccacatcaaggcaccctgcctcgcgcgtttcggtgatgacggtgaaaacctctgacacatgcagctcccggagacggtcacagcttgtctgtaagcggatgccgggagcagacaagcccgtcagggcgcgtcagcgggtgttggcgggtgtcggggcgcagccatgacccagtcacgtagcgatagcggagtgtatactggcttaactatgcggcatcagagcagattgtactgagagtgcaccatatgcggtgtgaaataccgcacagatgcgtaaggagaaaataccgcatcaggcgctcttccgcttcctcgctcactgactcgctgcgctcggtcgttcggctgcggcgagcggtatcagctcactcaaaggcggtaatacggttatccacagaatcaggggataacgcaggaaagaacatgtgagcaaaaggccagcaaaaggccaggaaccgtaaaaaggccgcgttgctggcgtttttccataggctccgcccccctgacgagcatcacaaaaatcgacgctcaagtcagaggtggcgaaacccgacaggactataaagataccaggcgtttccccctggaagctccctcgtgcgctctcctgttccgaccctgccgcttaccggatacctgtccgcctttctcccttcgggaagcgtggcgctttctcatagctcacgctgtaggtatctcagttcggtgtaggtcgttcgctccaagctgggctgtgtgcacgaaccccccgttcagcccgaccgctgcgccttatccggtaactatcgtcttgagtccaacccggtaagacacgacttatcgccactggcagcagccactggtaacaggattagcagagcgaggtatgtaggcggtgctacagagttcttgaagtggtggcctaactacggctacactagaaggacagtatttggtatctgcgctctgctgaagccagttaccttcggaaaaagagttggtagctcttgatccggcaaacaaaccaccgctggtagcggtggtttttttgtttgcaagcagcagattacgcgcagaaaaaaaggatctcaagaagatcctttgatcttttctacggggtctgacgctcagtggaacgaaaactcacgttaagggattttggtcatgcatgatatatctcccaatttgtgtagggcttattatgcacgcttaaaaataataaaagcagacttgacctgatagtttggctgtgagcaattatgtgcttagtgcatctaatcgcttgagttaacgccggcgaagcggcgtcggcttgaacgaatttctagctagacattatttgccgactaccttggtgatctcgcctttcacgtagtggacaaattcttccaactgatctgcgcgcgaggccaagcgatcttcttcttgtccaagataagcctgtctagcttcaagtatgacgggctgatactgggccggcaggcgctccattgcccagtcggcagcgacatccttcggcgcgattttgccggttactgcgctgtaccaaatgcgggacaacgtaagcactacatttcgctcatcgccagcccagtcgggcggcgagttccatagcgttaaggtttcatttagcgcctcaaatagatcctgttcaggaaccggatcaaagagttcctccgccgctggacctaccaaggcaacgctatgttctcttgcttttgtcagcaagatagccagatcaatgtcgatcgtggctggctcgaagatacctgcaagaatgtcattgcgctgccattctccaaattgcagttcgcgcttagctggataacgccacggaatgatgtcgtcgtgcacaacaatggtgacttctacagcgcggagaatctcgctctctccaggggaagccgaagtttccaaaaggtcgttgatcaaagctcgccgcgttgtttcatcaagccttacggtcaccgtaaccagcaaatcaatatcactgtgtggcttcaggccgccatccactgcggagccgtacaaatgtacggccagcaacgtcggttcgagatggcgctcgatgacgccaactacctctgatagttgagtcgatacttcggcgatcaccgcttcccccatgatgtttaactttgttttagggcgactgccctgctgcgtaacatcgttgctgctccataacatcaaacatcgacccacggcgtaacgcgcttgctgcttggatgcccgaggcatagactgtaccccaaaaaaacatgtcataacaagaagccatgaaaaccgccactgcgccgttaccaccgctgcgttcggtcaaggttctggaccagttgcgtgacggcagttacgctacttgcattacagcttacgaaccgaacgaggcttatgtccactgggttcgtgcccgaattgatcacaggcagcaacgctctgtcatcgttacaatcaacatgctaccctccgcgagatcatccgtgtttcaaacccggcagcttagttgccgttcttccgaatagcatcggtaacatgagcaaagtctgccgccttacaacggctctcccgctgacgccgtcccggactgatgggctgcctgtatcgagtggtgattttgtgccgagctgccggtcggggagctgttggctggctggtggcaggatatattgtggtgtaaacaaattgacgcttagacaacttaataacacattgcggacgtttttaatgtactgaattaacgccgaattgctctagccaatacgcaaaccgcctctccccgcgcgttggccgattcattaattgcagcgtgacccggtcgtgcccctctctagagataatgagcattgcatgtctaagttataaaaaattaccacatattttttttgtcacacttgtttgaagtgcagtttatctatctttatacatatatttaaactttactctacgaataatataatctatagtactacaataatatcagtgttttagagaatcatataaatgaacagttagacatggtctaaaggacaattgagtattttgacaacaggactctacagttttatctttttagtgtgcatgtgttctcctttttttttgcaaatagcttcacctatataatacttcatccattttattagtacatccatttagggtttagggttaatggtttttatagactaatttttttagtacatctattttattctattttagcctctaaattaagaaaactaaaactctattttagtttttttatttaataatttagatataaaatagaataaaataaagtgactaaaaattaaacaaataccctttaagaaattaaaaaaactaaggaaacatttttcttgtttcgagtagataatgccagcctgttaaacgccgtcgatcgacgagtctaacggacaccaaccagcgaaccagcagcgtcgcgtcgggccaagcgaagcagacggcacggcatctctgtcgctgcctctggacccctctcgagagttccgctccaccgttggacttgctccgctgtcggcatccagaaattgcgtggcggagcggcagacgtgagccggcacggcaggcggcctcctcctcctctcacggcaccggcagctacgggggattcctttcccaccgctccttcgctttcccttcctcgcccgccgtaataaatagacaccccctccacaccctctttccccaacctcgtgttgttcggagcgcacacacacacaaccagatctcccccaaatccacccgtcggcacctccgcttcaaggtacgccgctcgtcctccccccccccccctctctaccttctctagatcggcgttccggtccatggttagggcccggtagttctacttctgttcatgtttgtgttagatccgtgtttgtgttagatccgtgctgctagcgttcgtacacggatgcgacctgtacgtcagacacgttctgattgctaacttgccagtgtttctctttggggaatcctgggatggctctagccgttccgcagacgggatcgatctaggataggtatacatgttgatgtgggttttactgatgcatatacatgatggcatatgcagcatctattcatatgctctaaccttgagtacctatctattataataaacaagtatgttttataattattttgatcttgatatacttggatgatggcatatgcagcagctatatgtggatttttttagccctgccttcatacgctatttatttgcttggtactgtttcttttgtcgatgctcaccctgttgtttggtgttacttctgcaggggtaccgccatggataagaagtactctatcggactcgatatcggaactaactctgtgggatgggctgtgatcaccgatgagtacaaggtgccatctaagaagttcaaggttctcggaaacaccgataggcactctatcaagaaaaaccttatcggtgctctcctcttcgattctggtgaaactgctgaggctaccagactcaagagaaccgctagaagaaggtacaccagaagaaagaacaggatctgctacctccaagagatcttctctaacgagatggctaaagtggatgattcattcttccacaggctcgaagagtcattcctcgtggaagaagataagaagcacgagaggcaccctatcttcggaaacatcgttgatgaggtggcataccacgagaagtaccctactatctaccacctcagaaagaagctcgttgattctactgataaggctgatctcaggctcatctacctcgctctcgctcacatgatcaagttcagaggacacttcctcatcgagggtgatctcaaccctgataactctgatgtggataagttgttcatccagctcgtgcagacctacaaccagcttttcgaagagaaccctatcaacgcttcaggtgtggatgctaaggctatcctctctgctaggctctctaagtcaagaaggcttgagaacctcattgctcagctccctggtgagaagaagaacggacttttcggaaacttgatcgctctctctctcggactcacccctaacttcaagtctaacttcgatctcgctgaggatgcaaagctccagctctcaaaggatacctacgatgatgatctcgataacctcctcgctcagatcggagatcagtacgctgatttgttcctcgctgctaagaacctctctgatgctatcctcctcagtgatatcctcagagtgaacaccgagatcaccaaggctccactctcagcttctatgatcaagagatacgatgagcaccaccaggatctcacacttctcaaggctcttgttagacagcagctcccagagaagtacaaagagattttcttcgatcagtctaagaacggatacgctggttacatcgatggtggtgcatctcaagaagagttctacaagttcatcaagcctatcctcgagaagatggatggaaccgaggaactcctcgtgaagctcaatagagaggatcttctcagaaagcagaggaccttcgataacggatctatccctcatcagatccacctcggagagttgcacgctatccttagaaggcaagaggatttctacccattcctcaaggataacagggaaaagattgagaagattctcaccttcagaatcccttactacgtgggacctctcgctagaggaaactcaagattcgcttggatgaccagaaagtctgaggaaaccatcaccccttggaacttcgaagaggtggtggataagggtgctagtgctcagtctttcatcgagaggatgaccaacttcgataagaaccttccaaacgagaaggtgctccctaagcactctttgctctacgagtacttcaccgtgtacaacgagttgaccaaggttaagtacgtgaccgagggaatgaggaagcctgcttttttgtcaggtgagcaaaagaaggctatcgttgatctcttgttcaagaccaacagaaaggtgaccgtgaagcagctcaaagaggattacttcaagaaaatcgagtgcttcgattcagttgagatttctggtgttgaggataggttcaacgcatctctcggaacctaccacgatctcctcaagatcattaaggataaggatttcttggataacgaggaaaacgaggatatcttggaggatatcgttcttaccctcaccctctttgaagatagagagatgattgaagaaaggctcaagacctacgctcatctcttcgatgataaggtgatgaagcagttgaagagaagaagatacactggttggggaaggctctcaagaaagctcattaacggaatcagggataagcagtctggaaagacaatccttgatttcctcaagtctgatggattcgctaacagaaacttcatgcagctcatccacgatgattctctcacctttaaagaggatatccagaaggctcaggtttcaggacagggtgatagtctccatgagcatatcgctaacctcgctggatctcctgcaatcaagaagggaatcctccagactgtgaaggttgtggatgagttggtgaaggtgatgggaaggcataagcctgagaacatcgtgatcgaaatggctagagagaaccagaccactcagaagggacagaagaactctagggaaaggatgaagaggatcgaggaaggtatcaaagagcttggatctcagatcctcaaagagcaccctgttgagaacactcagctccagaatgagaagctctacctctactacctccagaacggaagggatatgtatgtggatcaagagttggatatcaacaggctctctgattacgatgttgatcatatcgtgccacagtcattcttgaaggatgattctatcgataacaaggtgctcaccaggtctgataagaacaggggtaagagtgataacgtgccaagtgaagaggttgtgaagaaaatgaagaactattggaggcagctcctcaacgctaagctcatcactcagagaaagttcgataacttgactaaggctgagaggggaggactctctgaattggataaggcaggattcatcaagaggcagcttgtggaaaccaggcagatcactaagcacgttgcacagatcctcgattctaggatgaacaccaagtacgatgagaacgataagttgatcagggaagtgaaggttatcaccctcaagtcaaagctcgtgtctgatttcagaaaggatttccaattctacaaggtgagggaaatcaacaactaccaccacgctcacgatgcttaccttaacgctgttgttggaaccgctctcatcaagaagtatcctaagctcgagtcagagttcgtgtacggtgattacaaggtgtacgatgtgaggaagatgatcgctaagtctgagcaagagatcggaaaggctaccgctaagtatttcttctactctaacatcatgaatttcttcaagaccgagattaccctcgctaacggtgagatcagaaagaggccactcatcgagacaaacggtgaaacaggtgagatcgtgtgggataagggaagggatttcgctaccgttagaaaggtgctctctatgccacaggtgaacatcgttaagaaaaccgaggtgcagaccggtggattctctaaagagtctatcctccctaagaggaactctgataagctcattgctaggaagaaggattgggaccctaagaaatacggtggtttcgattctcctaccgtggcttactctgttctcgttgtggctaaggttgagaagggaaagagtaagaagctcaagtctgttaaggaacttctcggaatcactatcatggaaaggtcatctttcgagaagaacccaatcgatttcctcgaggctaagggatacaaagaggttaagaaggatctcatcatcaagctcccaaagtactcactcttcgaactcgagaacggtagaaagaggatgctcgcttctgctggtgagcttcaaaagggaaacgagcttgctctcccatctaagtacgttaactttctttacctcgcttctcactacgagaagttgaagggatctccagaagataacgagcagaagcaacttttcgttgagcagcacaagcactacttggatgagatcatcgagcagatctctgagttctctaaaagggtgatcctcgctgatgcaaacctcgataaggtgttgtctgcttacaacaagcacagagataagcctatcagggaacaggcagagaacatcatccatctcttcacccttaccaacctcggtgctcctgctgctttcaagtacttcgatacaaccatcgataggaagagatacacctctaccaaagaagtgctcgatgctaccctcatccatcagtctatcactggactctacgagactaggatcgatctctcacagctcggtggtgattcaagggctgatcctaagaagaagaggaaggtttgaggcgcgccgagctccaggcctcccagctttcgtccgtatcatcggtttcgacaacgttcgtcaagttcaatgcatcagtttcattgcccacacaccagaatcctactaagtttgagtattatggcattggaaaagctgttttcttctatcatttgttctgcttgtaatttactgtgttctttcagtttttgttttcggacatcaaaatgcaaatggatggataagagttaataaatgatatggtccttttgttcattctcaaattattattatctgttgtttttactttaatgggttgaatttaagtaagaaaggaactaacagtgtgatattaaggtgcaatgttagacatataaaacagtctttcacctctctttggttatgtcttgaattggtttgtttcttcacttatctgtgtaatcaagtttactatgagtctatgatcaagtaattatgcaatcaagttaagtacagtataggcttgagctccctaggcctgttatccctaacaagtttgtacaaaaaagcaggctgagctcgaccaagcccgttattctgacagttctggtgctcaacacatttatatttatcaaggagcacattgttactcactgctaggagggaatcgaactaggaatattgatcagaggaactacgagagagctgaagataactgccctctagctctcactgatctgggcgcatagtgagatgcagcccacgtgagttcagcaacggtctagcgctgggcttttaggcccgcatgatcgggctttgtcgggtggtcgacgtgttcacgattggggagagcaacgcagcagttcctcttagtttagtcccacctcgcctgtccagcagagttctgaccggtttataaactcgcttgctgcatcagacttgnnnnnnnnnnnnnnnnnnnngttttagagctagaaatagcaagttaaaataaggctagtccgttatcaacttgaaaaagtggcaccgagtcggtgctttttttctagacccagctttcttgtacaaagttggcattaacccagctttc

SEQ ID NO: 24 - DNA, 16792 bp, Artificial Sequence
  Vektor1_ZmU3
  misc_feature (16645)..(16664): n is a, c, g, or t
ttgtacaaagtggttcgataattccgatccagcctaggcccgggcctgaggacgcgccttactagtggatcccttcaccgccattgcaaaaattgtcaataaatatttagagtgggtggcatcagaaaaacatctctagtggactctcttcctatcatagctactcgggctgtagatagaacgagggcacaagagttgggtggcgtaggtttactcgtgacctcaactcttttggctgtgtcttacgtctaagatgggtttggcatgtgagaaacataggtctaagcaattcatgttagggctgttgcattgttgttgcatcaaccaaatgtccagatagcagttcatgctacatctagttgaaaaccctcatcattaggcggaacatgtgttcttttttagcatagtcaaagtcagattgcggcactcgctcatccacggaaagaattttccctgtgcaggcatctcgatcaaaagacgcaaattaatttttgaatagcgatataacaatatctaattaacgtttcttgttttctgcgaaatgtctttcatcataaaatgagtcatctcgatgagcccaagtgacatagcccaacaccccaccccaccaataaaagtgaagaaaacatgttgggaaaactataccaagtaaaatacgagttgttctaaagaaaaagtaaagtacgagttagatcgcaccctgtcctggagtgtggcttgatgatccaactcctagcattgtatccctgtttttggatgatgtaactattatttacaatgaataaagaggtgttttactagtaaaaaaatcttgaggggaggagaaaataatggaggtcttttttcaaaccgatggactattatttttagtgaaagagaataatattattggaaaaattattctatccacttattttatattggcagaatacaaagaatggtggggtccacgcggaacttgcggcccccgaaacctatcgagggcgcggtacccaagcaaggaacggaggaaacttgcggggcccgaaacctagtgataaaaggcatatcatccacacgatgaagatctgacggaccatatctcccaccacggaaagccatcagacgaggatcagacggccaggaaggaaccctagcgcccgccggtgccaatataaagcgccactctctctcgtcttaagccccagcctctccattcccctctccctctcgattacgaggtgtgttgttcatccgtcccgaatccatccatcccctcttcagatgtgttgttcatggctctaatagctctagatctgcttgtttgtgttgtttagctctagatctactcgcgcgcgcttctctctcgatctcctgtagaacaattttggttggttttttgtgcatatccatggtaattttgtctgcaatatggaggaggctttctaagctcctacgtagcatcgatctttagaattccctcggtttctgtttatttcttcgcgagggctctctgttatctgtaggagtagctgtaagcgcggttcgttacggattaatcgtcatgcttagttgaacctatcggtcgaaggatttgtgtgggttgtcgtgtagaattgacaccatctacttactgtactgatatgccgatctgtaggatactcttcattacttttgtttactgctagttgtggtgtagatttagcattctcaaacccatgctgtagcgtttctaatattgttacatagatctaccggtgcctgttaattgtattcgatcgggcgtttctacatctgtccgcccacctagttttatatgtggtaatcaaaattgcgttgacttcgtgatgctgtctgtgtactgtttttaatcgctcttacttagatgatcaacatggtgatggttacgatttactgttttctaatccctgttacttcgatgctgcagtttgattgatgggcccagaacgacgcccggccgacatccgccgtgccaccgaggcggacatgccggcggtctgcaccatcgtcaaccactacatcgagacaagcacggtcaacttccgtaccgagccgcaggaaccgcaggagtggacggacgacctcgtccgtctgcgggagcgctatccctggctcgtcgccgaggtggacggcgaggtcgccggcatcgcctacgcgggcccctggaaggcacgcaacgcctacgactggacggccgagtcgaccgtgtacgtctccccccgccaccagcggacgggactgggctccacgctctacacccacctgctgaagtccctggaggcacagggcttcaagagcgtggtcgctgtcatcgggctgcccaacgacccgagcgtgcgcatgcacgaggcgctcggatatgccccccgcggcatgctgcgggcggccggcttcaagcacgggaactggcatgacgtgggtttctggcagctggacttcagcctgccggtaccgccccgtccggtcctgcccgtcaccgagatctgaatgccgaatttccccgatcgttcaaacatttggcaataaagtttcttaagattgaatcctgttgccggtcttgcgatgattatcatataatttctgttgaattacgttaagcatgtaataattaacatgtaatgcatgacgttatttatgagatgggtttttatgattagagtcccgcaattatacatttaatacgcgatagaaaacaaaatatagcgcgcaaactaggataaattatcgcgcgcggtgtcatctatgttactagatcgctcgaagatcccccgggctgcaggaattcaagcttggcactggccgtcgttttacaacgtcgtgactgggaaaaccctggcgttacccaacttaatcgccttgcagcacatccccctttcgccagctggcgtaatagcgaagaggcccgcaccgatcgcccttcccaacagttgcgcagcctgaatggcgaatgagcttgagcttggatcagattgtcgtttcccgccttcagtttaaactatcagtgtttgacaggatatattggcgggtaaacctaagagaaaagagcgtttattagaataacggatatttaaaagggcgtgaaaaggtttatccgttcgtccatttgtatgtgcatgccaaccacagggttcccctcgggatcaaagtactttgatccaacccctccgctgctatagtgcagtcggcttctgacgttcagtgcagccgtcttctgaaaacgacatgtcgcacaagtcctaagttacgcgacaggctgccgccctgcccttttcctggcgttttcttgtcgcgtgttttagtcgcataaagtagaatacttgcgactagaaccggagacattacgccatgaacaagagcgccgccgctggcctgctgggctatgcccgcgtcagcaccgacgaccaggacttgaccaaccaacgggccgaactgcacgcggccggctgcaccaagctgttttccgagaagatcaccggcaccaggcgcgaccgcccggagctggccaggatgcttgaccacctacgccctggcgacgttgtgacagtgaccaggctagaccgcctggcccgcagcacccgcgacctactggacattgccgagcgcatccaggaggccggcgcgggcctgcgtagcctggcagagccgtgggccgacaccaccacgccggccggccgcatggtgttgaccgtgttcgccggcattgccgagttcgagcgttccctaatcatcgaccgcacccggagcgggcgcgaggccgccaaggcccgaggcgtgaagtttggcccccgccctaccctcaccccggcacagatcgcgcacgcccgcgagctgatcgaccaggaaggccgcaccgtgaaagaggcggctgcactgcttggcgtgcatcgctcgaccctgtaccgcgcacttgagcgcagcgaggaagtgacgcccaccgaggccaggcggcgcggtgccttccgtgaggacgcattgaccgaggccgacgccctggcggccgccgagaatgaacgccaagaggaacaagcatgaaaccgcaccaggacggccaggacgaaccgtttttcattaccgaagagatcgaggcggagatgatcgcggccgggtacgtgttcgagccgcccgcgcacgtctcaaccgtgcggctgcatgaaatcctggccggtttgtctgatgccaagctggcggcctggccggccagcttggccgctgaagaaaccgagcgccgccgtctaaaaaggtgatgtgtatttgagtaaaacagcttgcgtcatgcggtcgctgcgtatatgatgcgatgagtaaataaacaaatacgcaaggggaacgcatgaaggttatcgctgtacttaaccagaaaggcgggtcaggcaagacgaccatcgcaacccatctagcccgcgccctgcaactcgccggggccgatgttctgttagtcgattccgatccccagggcagtgcccgcgattgggcggccgtgcgggaagatcaaccgctaaccgttgtcggcatcgaccgcccgacgattgaccgcgacgtgaaggccatcggccggcgcgacttcgtagtgatcgacggagcgccccaggcggcggacttggctgtgtccgcgatcaaggcagccgacttcgtgctgattccggtgcagccaagcccttacgacatatgggccaccgccgacctggtggagctggttaagcagcgcattgaggtcacggatggaaggctacaagcggcctttgtcgtgtcgcgggcgatcaaaggcacgcgcatcggcggtgaggttgccgaggcgctggccgggtacgagctgcccattcttgagtcccgtatcacgcagcgcgtgagctacccaggcactgccgccgccggcacaaccgttcttgaatcagaacccgagggcgacgctgcccgcgaggtccaggcgctggccgctgaaattaaatcaaaactcatttgagttaatgaggtaaagagaaaatgagcaaaagcacaaacacgctaagtgccggccgtccgagcgcacgcagcagcaaggctgcaacgttggccagcctggcagacacgccagccatgaagcgggtcaactttcagttgccggcggaggatcacaccaagctgaagatgtacgcggtacgccaaggcaagaccattaccgagctgctatctgaatacatcgcgcagctaccagagtaaatgagcaaatgaataaatgagtagatgaattttagcggctaaaggaggcggcatggaaaatcaagaacaaccaggcaccgacgccgtggaatgccccatgtgtggaggaacgggcggttggccaggcgtaagcggctgggttgtctgccggccctgcaatggcactggaacccccaagcccgaggaatcggcgtgacggtcgcaaaccatccggcccggtacaaatcggcgcggcgctgggtgatgacctggtggagaagttgaaggccgcgcaggccgcccagcggcaacgcatcgaggcagaagcacgccccggtgaatcgtggcaagcggccgctgatcgaatccgcaaagaatcccggcaaccgccggcagccggtgcgccgtcgattaggaagccgcccaagggcgacgagcaaccagattttttcgttccgatgctctatgacgtgggcacccgcgatagtcgcagcatcatggacgtggccgttttccgtctgtcgaagcgtgaccgacgagctggcgaggtgatccgctacgagcttccagacgggcacgtagaggtttccgcagggccggccggcatggccagtgtgtgggattacgacctggtactgatggcggtttcccatctaaccgaatccatgaaccgataccgggaagggaagggagacaagcccggccgcgtgttccgtccacacgttgcggacgtactcaagttctgccggcgagccgatggcggaaagcagaaagacgacctggtagaaacctgcattcggttaaacaccacgcacgttgccatgcagcgtacgaagaaggccaagaacggccgcctggtgacggtatccgagggtgaagccttgattagccgctacaagatcgtaaagagcgaaaccgggcggccggagtacatcgagatcgagctagctgattggatgtaccgcgagatcacagaaggcaagaacccggacgtgctgacggttcaccccgattactttttgatcgatcccggcatcggccgttttctctaccgcctggcacgccgcgccgcaggcaaggcagaagccagatggttgttcaagacgatctacgaacgcagtggcagcgccggagagttcaagaagttctgtttcaccgtgcgcaagctgatcgggtcaaatgacctgccggagtacgatttgaaggaggaggcggggcaggctggcccgatcctagtcatgcgctaccgcaacctgatcgagggcgaagcatccgccggttcctaatgtacggagcagatgctagggcaaattgccctagcaggggaaaaaggtcgaaaaggtctctttcctgtggatagcacgtacattgggaacccaaagccgtacattgggaaccggaacccgtacattgggaacccaaagccgtacattgggaaccggtcacacatgtaagtgactgatataaaagagaaaaaaggcgatttttccgcctaaaactctttaaaacttattaaaactcttaaaacccgcctggcctgtgcataactgtctggccagcgcacagccgaagagctgcaaaaagcgcctacccttcggtcgctgcgctccctacgccccgccgcttcgcgtcggcctatcgcggccgctggccgctcaaaaatggctggcctacggccaggcaatctaccagggcgcggacaagccgcgccgtcgccactcgaccgccggcgcccacatcaaggcaccctgcctcgcgcgtttcggtgatgacggtgaaaacctctgacacatgcagctcccggagacggtcacagcttgtctgtaagcggatgccgggagcagacaagcccgtcagggcgcgtcagcgggtgttggcgggtgtcggggcgcagccatgacccagtcacgtagcgatagcggagtgtatactggcttaactatgcggcatcagagcagattgtactgagagtgcaccatatgcggtgtgaaataccgcacagatgcgtaaggagaaaataccgcatcaggcgctcttccgcttcctcgctcactgactcgctgcgctcggtcgttcggctgcggcgagcggtatcagctcactcaaaggcggtaatacggttatccacagaatcaggggataacgcaggaaagaacatgtgagcaaaaggccagcaaaaggccaggaaccgtaaaaaggccgcgttgctggcgtttttccataggctccgcccccctgacgagcatcacaaaaatcgacgctcaagtcagaggtggcgaaacccgacaggactataaagataccaggcgtttccccctggaagctccctcgtgcgctctcctgttccgaccctgccgcttaccggatacctgtccgcctttctcccttcgggaagcgtggcgctttctcatagctcacgctgtaggtatctcagttcggtgtaggtcgttcgctccaagctgggctgtgtgcacgaaccccccgttcagcccgaccgctgcgccttatccggtaactatcgtcttgagtccaacccggtaagacacgacttatcgccactggcagcagccactggtaacaggattagcagagcgaggtatgtaggcggtgctacagagttcttgaagtggtggcctaactacggctacactagaaggacagtatttggtatctgcgctctgctgaagccagttaccttcggaaaaagagttggtagctcttgatccggcaaacaaaccaccgctggtagcggtggtttttttgtttgcaagcagcagattacgcgcagaaaaaaaggatctcaagaagatcctttgatcttttctacggggtctgacgctcagtggaacgaaaactcacgttaagggattttggtcatgcatgatatatctcccaatttgtgtagggcttattatgcacgcttaaaaataataaaagcagacttgacctgatagtttggctgtgagcaattatgtgcttagtgcatctaatcgcttgagttaacgccggcgaagcggcgtcggcttgaacgaatttctagctagacattatttgccgactaccttggtgatctcgcctttcacgtagtggacaaattcttccaactgatctgcgcgcgaggccaagcgatcttcttcttgtccaagataagcctgtctagcttcaagtatgacgggctgatactgggccggcaggcgctccattgcccagtcggcagcgacatccttcggcgcgattttgccggttactgcgctgtaccaaatgcgggacaacgtaagcactacatttcgctcatcgccagcccagtcgggcggcgagttccatagcgttaaggtttcatttagcgcctcaaatagatcctgttcaggaaccggatcaaagagttcctccgccgctggacctaccaaggcaacgctatgttctcttgcttttgtcagcaagatagccagatcaatgtcgatcgtggctggctcgaagatacctgcaagaatgtcattgcgctgccattctccaaattgcagttcgcgcttagctggataacgccacggaatgatgtcgtcgtgcacaacaatggtgacttctacagcgcggagaatctcgctctctccaggggaagccgaagtttccaaaaggtcgttgatcaaagctcgccgcgttgtttcatcaagccttacggtcaccgtaaccagcaaatcaatatcactgtgtggcttcaggccgccatccactgcggagccgtacaaatgtacggccagcaacgtcggttcgagatggcgctcgatgacgccaactacctctgatagttgagtcgatacttcggcgatcaccgcttcccccatgatgtttaactttgttttagggcgactgccctgctgcgtaacatcgttgctgctccataacatcaaacatcgacccacggcgtaacgcgcttgctgcttggatgcccgaggcatagactgtaccccaaaaaaacatgtcataacaagaagccatgaaaaccgccactgcgccgttaccaccgctgcgttcggtcaaggttctggaccagttgcgtgacggcagttacgctacttgcattacagcttacgaaccgaacgaggcttatgtccactgggttcgtgcccgaattgatcacaggcagcaacgctctgtcatcgttacaatcaacatgctaccctccgcgagatcatccgtgtttcaaacccggcagcttagttgccgttcttccgaatagcatcggtaacatgagcaaagtctgccgccttacaacggctctcccgctgacgccgtcccggactgatgggctgcctgtatcgagtggtgattttgtgccgagctgccggtcggggagctgttggctggctggtggcaggatatattgtggtgtaaacaaattgacgcttagacaacttaataacacattgcggacgtttttaatgtactgaattaacgccgaattgctctagccaatacgcaaaccgcctctccccgcgcgttggccgattcattaattgcagcgtgacccggtcgtgcccctctctagagataatgagcattgcatgtctaagttataaaaaattaccacatattttttttgtcacacttgtttgaagtgcagtttatctatctttatacatatatttaaactttactctacgaataatataatctatagtactacaataatatcagtgttttagagaatcatataaatgaacagttagacatggtctaaaggacaattgagtattttgacaacaggactctacagttttatctttttagtgtgcatgtgttctcctttttttttgcaaatagcttcacctatataatacttcatccattttattagtacatccatttagggtttagggttaatggtttttatagactaatttttttagtacatctattttattctattttagcctctaaattaagaaaactaaaactctattttagtttttttatttaataatttagatataaaatagaataaaataaagtgactaaaaattaaacaaataccctttaagaaattaaaaaaactaaggaaacatttttcttgtttcgagtagataatgccagcctgttaaacgccgtcgatcgacgagtctaacggacaccaaccagcgaaccagcagcgtcgcgtcgggccaagcgaagcagacggcacggcatctctgtcgctgcctctggacccctctcgagagttccgctccaccgttggacttgctccgctgtcggcatccagaaattgcgtggcggagcggcagacgtgagccggcacggcaggcggcctcctcctcctctcacggcaccggcagctacgggggattcctttcccaccgctccttcgctttcccttcctcgcccgccgtaataaatagacaccccctccacaccctctttccccaacctcgtgttgttcggagcgcacacacacacaaccagatctcccccaaatccacccgtcggcacctccgcttcaaggtacgccgctcgtcctccccccccccccctctctaccttctctagatcggcgttccggtccatggttagggcccggtagttctacttctgttcatgtttgtgttagatccgtgtttgtgttagatccgtgctgctagcgttcgtacacggatgcgacctgtacgtcagacacgttctgattgctaacttgccagtgtttctctttggggaatcctgggatggctctagccgttccgcagacgggatcgatctaggataggtatacatgttgatgtgggttttactgatgcatatacatgatggcatatgcagcatctattcatatgctctaaccttgagtacctatctattataataaacaagtatgttttataattattttgatcttgatatacttggatgatggcatatgcagcagctatatgtggatttttttagccctgccttcatacgctatttatttgcttggtactgtttcttttgtcgatgctcaccctgttgtttggtgttacttctgcaggggtaccgccatggataagaagtactctatcggactcgatatcggaactaactctgtgggatgggctgtgatcaccgatgagtacaaggtgccatctaagaagttcaaggttctcggaaacaccgataggcactctatcaagaaaaaccttatcggtgctctcctcttcgattctggtgaaactgctgaggctaccagactcaagagaaccgctagaagaaggtacaccagaagaaagaacaggatctgctacctccaagagatcttctctaacgagatggctaaagtggatgattcattcttccacaggctcgaagagtcattcctcgtggaagaagataagaagcacgagaggcaccctatcttcggaaacatcgttgatgaggtggcataccacgagaagtaccctactatctaccacctcagaaagaagctcgttgattctactgataaggctgatctcaggctcatctacctcgctctcgctcacatgatcaagttcagaggacacttcctcatcgagggtgatctcaaccctgataactctgatgtggataagttgttcatccagctcgtgcagacctacaaccagcttttcgaagagaaccctatcaacgcttcaggtgtggatgctaaggctatcctctctgctaggctctctaagtcaagaaggcttgagaacctcattgctcagctccctggtgagaagaagaacggacttttcggaaacttgatcgctctctctctcggactcacccctaacttcaagtctaacttcgatctcgctgaggatgcaaagctccagctctcaaaggatacctacgatgatgatctcgataacctcctcgctcagatcggagatcagtacgctgatttgttcctcgctgctaagaacctctctgatgctatcctcctcagtgatatcctcagagtgaacaccgagatcaccaaggctccactctcagcttctatgatcaagagatacgatgagcaccaccaggatctcacacttctcaaggctcttgttagacagcagctcccagagaagtacaaagagattttcttcgatcagtctaagaacggatacgctggttacatcgatggtggtgcatctcaagaagagttctacaagttcatcaagcctatcctcgagaagatggatggaaccgaggaactcctcgtgaagctcaatagagaggatcttctcagaaagcagaggaccttcgataacggatctatccctcatcagatccacctcggagagttgcacgctatccttagaaggcaagaggatttctacccattcctcaaggataacagggaaaagattgagaagattctcaccttcagaatcccttactacgtgggacctctcgctagaggaaactcaagattcgcttggatgaccagaaagtctgaggaaaccatcaccccttggaacttcgaagaggtggtggataagggtgctagtgctcagtctttcatcgagaggatgaccaacttcgataagaaccttccaaacgagaaggtgctccctaagcactctttgctctacgagtacttcaccgtgtacaacgagttgaccaaggttaagtacgtgaccgagggaatgaggaagcctgcttttttgtcaggtgagcaaaagaaggctatcgttgatctcttgttcaagaccaacagaaaggtgaccgtgaagcagctcaaagaggattacttcaagaaaatcgagtgcttcgattcagttgagatttctggtgttgaggataggttcaacgcatctctcggaacctaccacgatctcctcaagatcattaaggataaggatttcttggataacgaggaaaacgaggatatcttggaggatatcgttcttaccctcaccctctttgaagatagagagatgattgaagaaaggctcaagacctacgctcatctcttcgatgataaggtgatgaagcagttgaagagaagaagatacactggttggggaaggctctcaagaaagctcattaacggaatcagggataagcagtctggaaagacaatccttgatttcctcaagtctgatggattcgctaacagaaacttcatgcagctcatccacgatgattctctcacctttaaagaggatatccagaaggctcaggtttcaggacagggtgatagtctccatgagcatatcgctaacctcgctggatctcctgcaatcaagaagggaatcctccagactgtgaaggttgtggatgagttggtgaaggtgatgggaaggcataagcctgagaacatcgtgatcgaaatggctagagagaaccagaccactcagaagggacagaagaactctagggaaaggatgaagaggatcgaggaaggtatcaaagagcttggatctcagatcctcaaagagcaccctgttgagaacactcagctccagaatgagaagctctacctctactacctccagaacggaagggatatgtatgtggatcaagagttggatatcaacaggctctctgattacgatgttgatcatatcgtgccacagtcattcttgaaggatgattctatcgataacaaggtgctcaccaggtctgataagaacaggggtaagagtgataacgtgccaagtgaagaggttgtgaagaaaatgaagaactattggaggcagctcctcaacgctaagctcatcactcagagaaagttcgataacttgactaaggctgagaggggaggactctctgaattggataaggcaggattcatcaagaggcagcttgtggaaaccaggcagatcactaagcacgttgcacagatcctcgattctaggatgaacaccaagtacgatgagaacgataagttgatcagggaagtgaaggttatcaccctcaagtcaaagctcgtgtctgatttcagaaaggatttccaattctacaaggtgagggaaatcaacaactaccaccacgctcacgatgcttaccttaacgctgttgttggaaccgctctcatcaagaagtatcctaagctcgagtcagagttcgtgtacggtgattacaaggtgtacgatgtgaggaagatgatcgctaagtctgagcaagagatcggaaaggctaccgctaagtatttcttctactctaacatcatgaatttcttcaagaccgagattaccctcgctaacggtgagatcagaaagaggccactcatcgagacaaacggtgaaacaggtgagatcgtgtgggataagggaagggatttcgctaccgttagaaaggtgctctctatgccacaggtgaacatcgttaagaaaaccgaggtgcagaccggtggattctctaaagagtctatcctccctaagaggaactctgataagctcattgctaggaagaaggattgggaccctaagaaatacggtggtttcgattctcctaccgtggcttactctgttctcgttgtggctaaggttgagaagggaaagagtaagaagctcaagtctgttaaggaacttctcggaatcactatcatggaaaggtcatctttcgagaagaacccaatcgatttcctcgaggctaagggatacaaagaggttaagaaggatctcatcatcaagctcccaaagtactcactcttcgaactcgagaacggtagaaagaggatgctcgcttctgctggtgagcttcaaaagggaaacgagcttgctctcccatctaagtacgttaactttctttacctcgcttctcactacgagaagttgaagggatctccagaagataacgagcagaagcaacttttcgttgagcagcacaagcactacttggatgagatcatcgagcagatctctgagttctctaaaagggtgatcctcgctgatgcaaacctcgataaggtgttgtctgcttacaacaagcacagagataagcctatcagggaacaggcagagaacatcatccatctcttcacccttaccaacctcggtgctcctgctgctttcaagtacttcgatacaaccatcgataggaagagatacacctctaccaaagaagtgctcgatgctaccctcatccatcagtctatcactggactctacgagactaggatcgatctctcacagctcggtggtgattcaagggctgatcctaagaagaagaggaaggtttgaggcgcgccgagctccaggcctcccagctttcgtccgtatcatcggtttcgacaacgttcgtcaagttcaatgcatcagtttcattgcccacacaccagaatcctactaagtttgagtattatggcattggaaaagctgttttcttctatcatttgttctgcttgtaatttactgtgttctttcagtttttgttttcggacatcaaaatgcaaatggatggataagagttaataaatgatatggtccttttgttcattctcaaattattattatctgttgtttttactttaatgggttgaatttaagtaagaaaggaactaacagtgtgatattaaggtgcaatgttagacatataaaacagtctttcacctctctttggttatgtcttgaattggtttgtttcttcacttatctgtgtaatcaagtttactatgagtctatgatcaagtaattatgcaatcaagttaagtacagtataggcttgagctccctaggcctgttatccctaacaagtttgtacaaaaaagcaggctgagctcgaattccatctaagtatcttggtaaagcatggattaatttggatgcccacttcaggtctatgcagctccggtgccttgtgattgtgagttgtgaccgatgctcatgctattctgcatttctgcgatgtatgtagctagtagatcttcaaaactaacaccgcatgccatcatcatccactgcttgattttagtctcaccgctggccaaaaatgtgatgatgccagaaacctcaactaccttgaatcaacacgggcccaacagtgtgatgacgacagaaacaaaaaaaaatgagccaatagttcagaaggaggcactatgcagaaactacatttctgaaggtgactaaaaggtgagcgtagagtgtaattactagtagtttagccaccattacccaaatgctttcgagcttgtattaagatttcctaagctgagcatcatcactgatctgcaggccaccctcgcttcgctgccaagatcaacagcaaccatgtggcggcaacatccagcattgcacatgggctaaagattgagctttgtgcctcgtctagggatcagctgaggttatcagtctttcctttttttcatccaggtgaggcatcaagctactactgcctcgattggctggacccgaagcccacatgtaggataccagaatgggccgacccaggacgcagtatgttggccagtcccaccggttagtgccatctcggttgctcacatgcgtagaagccagcttaaaaatttagctttggtgactcacagcattgnnnnnnnnnnnnnnnnnnnngttttagagctagaaatagcaagttaaaataaggctagtccgttatcaacttgaaaaagtggcaccgagtcggtgctttttttctagacccagctttcttgtacaaagttggcattaacccagctttc

SEQ ID NO: 25 - DNA, 3256 bp, Brome mosaic virus strain Fescue segment RNA1, complete sequence cDNA DQ530423
gagcgttaacgtagaccacggaacgaggttcaatcccttgtcgaccacggttctactacttgttctttgtttttcaccaacaaaatgtcaagttctatcgatttgctgaagttgattgctgagaagggtgctgccagccagagtgcccaagacatcgtagacaatcaggtcgcgcaacagttatctgcgcagattgaatacgcgaaaaggtctaagaaaatcaacgttcgcaataagctctctattgaggaggctgacgccttccgtgaccgttatggtggtgcctttgatttaaatttgactcagcagtatcatgcaccccatagcctggctggtgctctgcgtgtagcggagcattacgactgtctcgacagttttccccctgaagaccccgttatagatttcggagggtcttggtggcatcacttttcaagaagggataaaagggtgcacagttgttgtcctgtgttgggtgttagagacgctgcccgacatgaggagaggatgtgccgcatgcggaaaattttgcaagaaagcgatgatttcgatgaagtcccgaacttttgtcttaaccgagctcaagattgtgatgtccaagctgattgggctatctgtatccatggcggttatgatatgggcttccaaggtctgtgtgacgccatgcattcgcatggagtacgcgtactacgtggtaccgttatgttcgacggcgccatgttgtttgaccgcgagggttttcttcccttgcttaaatgtcactggcaacgtgacgggtcaggcgcggatgaggtgatcaaattcgactttgaaaatgaaagcacattatcttacatccatggatggcaagatttgggctcctttttcaccgagtcggtgcattgcatcgatggaaccacctatctgttggagcgcgaaatgctgaaatgtaacatcatgacctataagatcatcgctacaaatttacgctgcccccgggagacactacgtcactgtgtatggtttgaagacatatctaagtacgtgggagtctcaatacctgaagactggagtctcaatcgctggaaatgtgtgcgcgtcgccaaaaccacagtgagagaggtagaggagatagctttcagatgtttcaaggaaaataaagaatggaccgagaacatgaaagctgtcgcatctatcttatccgccaagtcgtcgactgttattattaacggtcaggctatcatggctggtgagcgcttagacattgaagattatcatctagtggcctttgctttgactttgaatctgtatcaaaagtacgaaaagcttacggccctccgcgatgggatggaatggaaaggttggtgccatcacttcaaaactaggttttggtggggtggagattcatccagggcgaaagtaggatggctgagaacattggctagcagatttcccctactacgtctggattcttatgcggacagttttaagtttctgactcgtctctcaaacgttgaagaatttgagcaagattctgtaccaatatcacgtttgagaacgttttggactgaagaggacttattcgaccggctggagcatgaagtgcagacagccaagaccaagcgctcgaagaagaaggcgatagtcccgccagctgctgagatacctcaggaggagtttcatgatgcccctgagagttcgagccctgagtccgtcagtgatgacgttaaaccggtgactgatgtggtcccggatgccgaggtgtctgttgaggtaccaacggaccctcgtggcatatctagacacggagccatgaaggaatttgtgcgttattgtaagagattacataacaactccgagtctaatcttcgtcacctatgggacatttccggcggtcgcggaagtgagatcgcaaataagagcatcttcgagacctaccatcgcatagacgatatggtgaatgtccatttggccaacggtaactggttgtatcctaaaaaatacgattacaccgttggatataatgagcatggtttaggtccgaagcacgcagatgaaacgtacattgttgataaaacatgtgcatgctctaacttgagggacattgcagaagctagcgccaaagtttctgtccctacatgcgatatttccatggttgatggagttgcgggatgcggtaaaaccactgccataaaagatgcattccgtatgggagaggacctaattgtgacggcgaatcgtaaatcggccgaggacgtcaggatggctttattccctgacacttttaattccaaggtagctttggatgttgtgcgcaccgcggattctgcgatcatgcacggtgtaccgtcctgtcataggctgcttgttgatgaggctggtttactacattacggtcaactcctggtggtggctgctctgtctaaatgttcacaagttcttgcctttggggacacagagcagatttcgttcaagtctcgtgacgcgggttttaaattgctccacggtaatctgaaatatgatcgccgtgacgttgttcacaagacttaccggtgtccgcaagatgttatcgctgctgttaatctgctgaagcgtaaatgcggtaatagggacacgaagtatcaatcctggacatctgagtccaaagtttctagaagtctcacgaagcgtcgtattacttctgttttgcaggtcactattgatccgaacagaacgtatcttacgatgactcaagctgataaagcggcccttcaaacgagggctaaggactttcccgtgagcaaggactggattgatggacatataaaaacagtacacgaagcgcaagggatctctgttgacaatgtcgctttggttcggcttaagtcgaccaaatgtgatttgtttaaacatgaggagtactgtttggttgccttaacacgacacaagaagtcctttgagtattgctttaacggcgagctcgctggtgatttgatctttaattgtgttaagtgatgcgcttgtctctgtgtgagacctctgctcgaggagagccctgttccaggtaggaacgttgtggtctaacttaagactagctgaatcggtgctataaccgatagtcgtggttgacacgcagacctcttacaagagtgtctaggcgcctttgagagttactctttgctctcttcggaagaacccctaggggttcgtgcatgggcttgcatagcaagtcttagaatgcgggtgccttacagtgttgaaaaacactgtaaatctctaaaagagaccattaattaagctc

SEQ ID NO: 26 - DNA, 2895 bp, Brome mosaic virus strain Fescue segment RNA2, complete sequence cDNA DQ530424
gagcgttaacacgcgtgtaaaccacggaacgaggttcaatcccttgtcgacccacggtttgcgcaacacacatctaaccttgttgttgttgtgttttgtttctttctactatcaccaagatgtcttcgaaaacctgggatgatgatttcgttcgccaggtcccgtctttccaatggatcatagatcaatccttagaagacgaggtggaggctgctagccttcaggtgcaggagccggcagacggagttgccattgacggatctctcgcgagttttaaattagctatagcgcccttggagataggaggggtgttcgatcccccttttgaccgagtgcgctggggctctatttgcgataccgtccagcaaatggttcaacagttcaccgatagaccactgattcctcaggctgaaatggcacggatgttatatcttgacattccgggctcttttgtgctcgaagatgaaatcgatgactggtatcctgaggatactagtgacggttacggtgtatcgtttgccgccgatgaagatcatgcgagcgatctaaaactcgccagtgattcctcgaactgtgaaattgaggaagttcgtgttactggagatacccccaaggagctgacccttggagataggtacatgggcattgacgaagagtttcagactaccaatactgattacgacatcactcttcagatcatgaatcctattgaacatagggtttcgcgcgttattgatacgcactgccatccagataaccctgacatctccactgggccaatttatatggagagagtcagccttgctagaacagaagcaaccagtcattccatactgccaacccatgcttatttcgatgattcgtaccatcaagcccttgttgagaatggtgattattccatggactttgataggatcagacttaagcaaagtgatgtagactggtacagggaccccgataaatattttcaaccaaaaatgaatatcgggagtgctcagcgaagagttggtactcagaaagaagtcttaaccgcacttaaaaagcgaaacgcggatgttccagaaatgggagacgcgattaacatgaaggaaactgcgaaggctatagcaaagcgctttcgtagcacattccttaatgttgacggtgaagactgtctgagagcttctatggatgtcatgactaagtgtcttgagtaccataagaagtggggtaagcacatggacttacaaggtgtgaatgtggcagcagagactgatttacgtcggtaccagcatatgctgaagtctgatgtaaaacctgttgtaactgacacccttcacttggaacgagcagtagcagctactataacatttcatagtaaaggtgtgactagtaatttttcaccctttttcactgcttgtttcgagaagttatcattggccctgaaatccaggttcattgtgcctatcggaaagatatcctctctggagcttaagaatgtccgcttgaataacagatactttcttgaagcggacctaagcaaatttgataaatctcagggtgagctgcacctagagtttcagagagagatacttcttgcgctgggctttccagcgccgctgacgaattggtggtctgattttcatcgcgattcttatttatcagaccctcatgccaaggtgggaatgtccgtttccttccaacgcagaactggtgatgcgtttacatatttcgggaatactcttgtcactatggctatgattgcatatgcctctgatctaagtgactgtgactgtgcaatattctcaggagatgattctttaatcatttctaaagttaaaccagtcttggataccgatatgttcacgtctctctttaatatggagataaaagttatggaccctagtgtgccctacgtttgtagtaagtttcttgttgaaactgaaatgggcaattgggtgtctataccagaccctatgagagagatccagcgcttagctaagcgaaagattctgcgtgaagaacagatgctcagagcacatttcgtttccttctgcgatcgaatgaagtttattaatcaacttgatgagaagatgattacgatgctctgtcattttgtttatctgaaatatgggaaagaaaaaccttggattttcgaggaggttagagctgctcttgcggctttttctttatactccgagaatttcctgaggttctctgattgctactgtaccgaaggcatcagagtttatcagatgagcgatcctgtatgtaagttcaaacgcactatggaagagcgtaaaactgatggtgactggtttcacaactggaagaatccaaagtttcctggtgtgttagacaaagtctacagaacccttggaatttattcctcggactgtagtactaaggagctccctgtcaaacggatcggacgtttacatgaggcccttgagcgtgagtcactcagattagcgaatgatcgtaggaccacacaacgcttgaaaaagaaggtcgacgattacgctaccggtagaggaggcctaacgtcagttgatgctttgctcttgaagtcccattgtgagacttttaagccctctgatctgagatgatcggttctatatgatatatgaacctaagctgtgagcagccctttggttaaggttaaaaactcctggtcaggtagaccactttggctaagtttaaaagcttgttgaatcagtacaataactgatagtcgtggttgacacgcagacctcttacaagagtgtctaggtgcctttgagagttactctttgctctcttcggaagaacccttaggggttcgtgcatgggcttgcatagcaagtcttagaatgcgggtaccgtacagtgttgaaaaacactgtaaatctctaaaagagaccattaattaagctc

SEQ ID NO: 27 - DNA, 2148 bp, Brome mosaic virus strain Fescue segment RNA3 T1025C cDNA
gagcccatgggttaacgtaaaataccaactaattctcgttcgattccggcgaacattctattttaccaacatcggttttttcagtagtgatactgtttttgttcccgatgtctaacatagtttctcccttcagtggttcctcacgaactacgtctgacgttggcaagcaagcgggaggtactagcgacgagaagctcattgagtcgctgttctctgaaaaggctgtgaaagagatagctgccgagtgtaaactcggatgttataactatctgaagtctaatgaaccccgcaactatatagacctggtgccaaagtcacacgtatctgcttggctctcatgggctacacccaagtatgataaaggagagttaccttccaggggattcatgaacgttccacgcatcgtttgttttctcgttcgtaccacagatagcgcagagtccggttctataaccgtgagcctgtgcgattctggtaaggctgctcgtgctggagtactcgaagccattgataatcaggaggccacaattcagttgtcggctttacctgctttgatagctttgacgcctagctatgattgtccgatggaagtcatcggcggtgatagcggtaggaatcgatgttttgggatagcaacccaacttagcggtgtggtggggacaacaggttccgttgcagttactcatgcttattggcaagctaatttcaaagcgaagcccaacaactataagttgcatggtcccgctacaattatggtaatgccatttgacagactgagacaactcgataagaaaagcctcaaaaattacatcagaggtatttctaaccagtctgtggatcatgggtatcttctcggaagaccgttacaatctgttgatcaggttgcccaggaagatttgttagttgaggaatccgagtctccttccgctctcggcagaggtgtgaaggatagtaagtctgtatccgcgtcatctgtcgctggacttcctgtgtccagtccttcgcttagaattaaataggtaaatccggtctaacaagctcggtccatttcgtggagttaagcaagctggggagacccccgacagccgtttggatcagcgctcgcgtctcgtttgggttcaattcccttaccttacaacggcgtgttgagataggtcctcgggggaggttatccatgtttgtggatattctatgttgtgtgtctgagttattaaaaaaaaaaaaaaaaaaaaaagatctatgtcctaattcagcgtattaataatgtcgacttcaggaactggtaagatgactcgcgcgcagcgtcgagctgccgctcgtagaaatcgtcggaccgctacggtccaaccggtaattgtcgaaccattcgctgctggccaaggcaaggccattaaagcgattgcaggatacagcatatcaaagtgggaggcgtcttcggacgcgattacagcgaaagccaccaatgccatgagtatcactctgccccatgagctctcttctgaaaagaataaggagcttaaggtcggcagggtgctgctttggttgggacttcttcctagcgttgctgggaggattaaggcttgtgttgctgagaaacaggcacaggccgaggccgcttttcaagtagccttggcggttgctgactcctcgaaagaggtggtcgcggccatgtatacggacgcctttcgaggggcgactctgggggatttgcttaatctccagatttatctgtatgcatctgaagcagtgcctgctaaggcggtcgttgtacatctagaagttgagcacgtaaggcctacgttcgatgacttcttcaccccggtttataggtagtgcccctgctcggagagcccctgactgggttaaagtcacaggccccttgtctcaggtagagaccctgtccaggtaggacactttggctaaggttaaaagcttgttgaatcagtacaataactgatagtcgtggttgacacgcagacctcttacaagagtgtctaggtgcctttgagagttactctttgctctcttcggaagaacccttaggggttcgtgcatgggcttgcatagcaagtcttagaatgcgggtaccgtacagtgttgaaaaacactgtaaatctctaaaagagaccattaattaactgcaggctc

SEQ ID NO: 28 - DNA, 2114 bp, Brome mosaic virus strain Fescue segment RNA3 cDNA DQ530425
gtaaaataccaactaattctcgttcgattccggcgaacattctattttaccaacatcggttttttcagtagtgatactgtttttgttcccgatgtctaacatagtttctcccttcagtggttcctcacgaactacgtctgacgttggcaagcaagcgggaggtactagcgacgagaagctcattgagtcgctgttctctgaaaaggctgtgaaagagatagctgccgagtgtaaactcggatgttataactatctgaagtctaatgaaccccgcaactatatagacctggtgccaaagtcacacgtatctgcttggctctcatgggctacacccaagtatgataaaggagagttaccttccaggggattcatgaacgttccacgcatcgtttgttttctcgttcgtaccacagatagcgcagagtccggttctataaccgtgagcctgtgcgattctggtaaggctgctcgtgctggagtactcgaagccattgataatcaggaggccacaattcagttgtcggctttacctgctttgatagctttgacgcctagctatgattgtccgatggaagtcatcggcggtgatagcggtaggaatcgatgttttgggatagcaacccaacttagcggtgtggtggggacaacaggttccgttgcagttactcatgcttattggcaagctaatttcaaagcgaagcccaacaactataagttgcatggtcccgctacaattatggtaatgccatttgacagactgagacaactcgataagaaaagcctcaaaaattacatcagaggtatttctaaccagtctgtggatcatgggtatcttctcggaagaccgttacaatctgttgatcaggttgcccaggaagatttgttagttgaggaatccgagtctccttccgctctcggcagaggtgtgaaggatagtaagtctgtatccgcgtcatctgtcgctggacttcctgtgtccagtccttcgcttagaattaaataggtaaatccggtctaacaagcttggtccatttcgtggagttaagcaagctggggagacccccgacagccgtttggatcagcgctcgcgtctcgtttgggttcaattcccttaccttacaacggcgtgttgagataggtcctcgggggaggttatccatgtttgtggatattctatgttgtgtgtctgagttattaaaaaaaaaaaaaaaaaaaaaagatctatgtcctaattcagcgtattaataatgtcgacttcaggaactggtaagatgactcgcgcgcagcgtcgagctgccgctcgtagaaatcgtcggaccgctacggtccaaccggtaattgtcgaaccattcgctgctggccaaggcaaggccattaaagcgattgcaggatacagcatatcaaagtgggaggcgtcttcggacgcgattacagcgaaagccaccaatgccatgagtatcactctgccccatgagctctcttctgaaaagaataaggagcttaaggtcggcagggtgctgctttggttgggacttcttcctagcgttgctgggaggattaaggcttgtgttgctgagaaacaggcacaggccgaggccgcttttcaagtagccttggcggttgctgactcctcgaaagaggtggtcgcggccatgtatacggacgcctttcgaggggcgactctgggggatttgcttaatctccagatttatctgtatgcatctgaagcagtgcctgctaaggcggtcgttgtacatctagaagttgagcacgtaaggcctacgttcgatgacttcttcaccccggtttataggtagtgcccctgctcggagagcccctgactgggttaaagtcacaggccccttgtctcaggtagagaccctgtccaggtaggacactttggctaaggttaaaagcttgttgaatcagtacaataactgatagtcgtggttgacacgcagacctcttacaagagtgtctaggtgcctttgagagttactctttgctctcttcggaagaacccttaggggttcgtgcatgggcttgcatagcaagtcttagaatgcgggtaccgtacagtgttgaaaaacactgtaaatctctaaaagagacca

SEQ ID NO: 29 - DNA, 2145 bp, Brome mosaic virus strain RNA3 R-BMV cDNA
gagcccatgggttaacgtaaaataccaactaattctcgttcgattccggcgaacattctattttaccaacatcggttttttcagtagtgatactgtttttgttcccgatgtctaacatagtttctcccttcagtggttcctcacgaactacgtctgacgttggcaagcaagcgggaggtactagcgatgagaagctcattgagtcgctgttctctgaaaaggctgtgaaagagatagctgccgagtgtaaactcggatgttataactatctgaagtctaatgaaccccgcaactatatagacctggtgccaaagtcacacgtatctgcttggctctcatgggctacatccaagtatgataaaggagagttaccttccaggggattcatgaacgttccacgcatcgtttgttttctcgttcgtaccacagatagcgcagagtccggttctataaccgtgagcctgtgcgattctggtaaggctgctcgtgctggagtactcgaagccattgataatcaggaggccacaattcagttgtcggctttacctgctttgatagctttgacgcctagctatgattgtccgatggaagtcatcggcggtgatagcggtaggaatcgatgttttgggatagcaacccaacttagcggtgtggtggggacaacaggttccgttgcagttactcatgcgtattggcaagctaatttcaaagcgaagcccaacaactataagttgcatggtcccgctacaattatggtaatgccatttgacagactgagacaactcgataagaaaagcctcaaaaattatattagaggtatttctaaccagtctgtggatcatgggtatcttctcggaagaccgttacaatctgttgatcaggttgcccaggaagatttgttagttgaggaatccgagtctccttccgctctcggcagaggtgtgaaggatagtaagtctgtatccgcgtcatctgtcgctggacttcctgtgtccagtcctacgcttagaattaaataggtaaatccggtctaacaagctcggtccatttcgtagagttaagcaagctggggagacccccgacagccgtttggatcagcgctcgcgtctcgtttgggttcaattcccttaccttacaacggcgtgttgagataggtcctcgggggaggttatccatgtttgtggatattctatgttgtgtgtctgagttattattaaaaaaaaaaaaaaaagatctatgtcctaattcagcgtattaataatgtcgacttcaggaactggtaagatgactcgcgcgcagcgtcgtgctgccgctcgcagaaatcgttggaccgctagggtccaaccagtaattgtcgaaccactcgctgctggccaaggcaaggccattaaagcgattgcaggatacagcatatcaaagtgggaggcgtcttcggacgcgattacagcgaaagccaccaatgccatgagtatcactctgccccatgagctctcttctgaaaagaataaggagcttaaggtcggcagggtgctgctttggttgggacttcttcctagcgttgctgggaggattaaggcttgtgttgctgagaaacaggcacaggccgaggctgcttttcaagtagccttggcggttgcagactcctcgaaagaggtggtcgcggccatgtatacggacgcctttcgaggggcgactctgggggatttgcttaatctccagatttatctgtatgcatctgaagcagtgcctgctaaggcggtcgttgtacatctagaagttgagcacgtaaggcctacgttcgatgacttcttcaccccggtttataggtagtgcccctgctcggagagcccctgactgggttaaagtcacaggccccttgtctcaggtagagaccctgtccaggtaggacactttggctaaggttaaaagcttgttgaatcagtacaataactgatagtcgtggttgacacgcagacctcttacaagagtgtctaggtgcctttgagagttactctttgctctcttcggaagaacccttaggggttcgtgcatgggcttgcatagcaagtcttagaatgcgggtaccgtacagtgttgaaaaacactgtaaatctctaaaagagaccattaattaactgcaggctc

SEQ ID NO: 30 - DNA, 2111 bp, Brome mosaic virus strain RNA3 gi|331498|gb|J02042.1|MBRCG3Z Brome mosaic virus 3a and coat protein genes, complete cds
gtaaaataccaactaattctcgttcgattccggcgaacattctattttaccaacatcggttttttcagtagtgatactgtttttgttcccgatgtctaacatagtttctcccttcagtggttcctcacgaactacgtctgacgttggcaagcaagcgggaggtactagcgatgagaagctcattgagtcgctgttctctgaaaaggctgtgaaagagatagctgccgagtgtaaactcggatgttataactatctgaagtctaatgaaccccgcaactatatagacctggtgccaaagtcacacgtatctgcttggctctcatgggctacatccaagtatgataaaggagagttaccttccaggggattcatgaacgttccacgcatcgtttgttttctcgttcgtaccacagatagcgcagagtccggttctataaccgtgagcctgtgcgattctggtaaggctgctcgtgctggagtactcgaagccattgataatcaggaggccacaattcagttgtcggctttacctgctttgatagctttgacgcctagctatgattgtccgatggaagtcatcggcggtgatagcggtaggaatcgatgttttgggatagcaacccaacttagcggtgtggtggggacaacaggttccgttgcagttactcatgcgtattggcaagctaatttcaaagcgaagcccaacaactataagttgcatggtcccgctacaattatggtaatgccatttgacagactgagacaactcgataagaaaagcctcaaaaattatattagaggtatttctaaccagtctgtggatcatgggtatcttctcggaagaccgttacaatctgttgatcaggttgcccaggaagatttgttagttgaggaatccgagtctccttccgctctcggcagaggtgtgaaggatagtaagtctgtatccgcgtcatctgtcgctggacttcctgtgtccagtcctacgcttagaattaaataggtaaatccggtctaacaagctcggtccatttcgtagagttaagcaagctggggagacccccgacagccgtttggatcagcgctcgcgtctcgtttgggttcaattcccttaccttacaacggcgtgttgagataggtcctcgggggaggttatccatgtttgtggatattctatgttgtgtgtctgagttattattaaaaaaaaaaaaaaaagatctatgtcctaattcagcgtattaataatgtcgacttcaggaactggtaagatgactcgcgcgcagcgtcgtgctgccgctcgcagaaatcgttggaccgctagggtccaaccagtaattgtcgaaccactcgctgctggccaaggcaaggccattaaagcgattgcaggatacagcatatcaaagtgggaggcgtcttcggacgcgattacagcgaaagccaccaatgccatgagtatcactctgccccatgagctctcttctgaaaagaataaggagcttaaggtcggcagggtgctgctttggttgggacttcttcctagcgttgctgggaggattaaggcttgtgttgctgagaaacaggcacaggccgaggctgcttttcaagtagccttggcggttgcagactcctcgaaagaggtggtcgcggccatgtatacggacgcctttcgaggggcgactctgggggatttgcttaatctccagatttatctgtatgcatctgaagcagtgcctgctaaggcggtcgttgtacatctagaagttgagcacgtaaggcctacgttcgatgacttcttcaccccggtttataggtagtgcccctgctcggagagcccctgactgggttaaagtcacaggccccttgtctcaggtagagaccctgtccaggtaggacactttggctaaggttaaaagcttgttgaatcagtacaataactgatagtcgtggttgacacgcagacctcttacaagagtgtctaggtgcctttgagagttactctttgctctcttcggaagaacccttaggggttcgtgcatgggcttgcatagcaagtcttagaatgcgggtaccgtacagtgttgaaaaacactgtaaatctctaaaagagacca

SEQ ID NO: 31 - DNA, 2150 bp, Brome mosaic virus C-BMVA/G
gagcccatgggttaacgtaaaataccaactaattctcgttcgattccggcgaacattctattttaccaacatcggttttttcagtagtgatactgtttttgttcccgatgtctaacatagtttctcccttcagtggttcctcacgaactacgtctgacgttggcaagcaagcgggaggtactagcgacgagaagctcattgagtcgctgttctctgaaaaggctgtgaaagagatagctgccgagtgtaaactcggatgttataactatctgaagtctaatgaaccccgcaactatatagacctggtgccaaagtcacacgtatctgcttggctctcatgggctacacccaagtatgataaaggagagttaccttccaggggattcatgaacgttccacgcatcgtttgttttctcgttcgtaccacagatagcgcagagtccggttctataaccgtgagcctgtgcgattctggtaaggctgctcgtgctggagtactcgaagccattgataatcaggaggccacaattcagttgtcggctttacctgctttgatagctttgacgcctagctatgattgtccgatggaagtcatcggcggtgatagcggtaggaatcgatgttttgggatagcaacccaacttagcggtgtggtggggacaacaggttccgttgcagttactcatgcttattggcaagctaatttcaaagcgaagcccaacaactataagttgcatggtcccgctacaattatggtaatgccatttgacagactgagacaactcgataagaaaagcctcaaaaattacatcagaggtatttctaaccagtctgtggatcatgggtatcttctcggaagaccgttacaatctgttgatcaggttgcccaggaagatttgttagttgaggaatccgagtctccttccgctctcggcagaggtgtgaaggatagtaagtctgtatccgcgtcatctgtcgctggacttcctgtgtccagtcctacgcttagaattaaataggtaaatccggtctaacaagctcggtccatttcgtagagttaagcaagctggggagacccccgacagccgtttggatcagcgctcgcgtctcgtttgggttcaattcccttaccttacaacggcgtgttgagataggtcctcgggggaggttatccatgtttgtggatattctatgttgtgtgtctgagttattattaaaaaaaaaaaaaaaagatctatgtcctaattcagcgtattaatttaacaatgtcgacttcaggaactggtaagatgactcgcgcgcagcgtcgagctgccgctcgtagaaatcgtcggaccgctacggtccaaccggtaattgtcgaaccattcgctgctggccaaggcaaggccattaaagcgattgcaggatacagcatatcaaagtgggaggcgtcttcggacgcgattacagcgaaagccaccaatgccatgagtatcactctgccccatgagctctcttctgaaaagaataaggagcttaaggtcggcagggtgctgctttggttgggacttcttcctagcgttgctgggaggattaaggcttgtgttgctgagaaacaggcacaggccgaggccgcttttcaagtagccttggcggttgctgactcctcgaaagaggtggtcgcggccatgtatacggacgcctttcgaggggcgactctgggggatttgcttaatctccagatttatctgtatgcatctgaagcagtgcctgctaaggcggtcgttgtacatctagaagttgagcacgtaaggcctacgttcgatgacttcttcaccccggtttataggtagtgcccctgctcggagagcccctgactgggttaaagtcacaggccccttgtctcaggtagagaccctgtccaggtaggacactttggctaaggttaaaagcttgttgaatcagtacaataactgatagtcgtggttgacacgcagacctcttacaagagtgtctaggtgcctttgagagttactctttgctctcttcggaagaacccttaggggttcgtgcatgggcttgcatagcaagtcttagaatgcgggtaccgtacagtgttgaaaaacactgtaaatctctaaaagagaccattaattaactgcaggctc

SEQ ID NO: 32 - DNA, 3787 bp, Barley stripe mosaic virus BSMV ND18 RNA1 U35767
gtatgtaagttgcctttgggtgtaaaatttcttgcatgcacataatcgtaatcgattcttcttgatctctaaacaacactttcccgttagcatggctagcgatgagattgtccgcaatctgatctcccgtgaggaggtgatgggtaatttgattagcacagcttctagctcagtaaggtcacccttacatgacgtactgtgctcgcacgtaaggaccatcgtcgattccgtggataagaaagcggtcagtcgcaagcatgttgatgtacggcgcaacatctcctctgaagagttacagatgttgataaatgcatatcctgaatatgccgtttcatcctcagcttgtgaatctggtactcatagcatggcggcttgttttcgatttctggagacagaatacctcttagatatggttccaatgaaagagacttttgtttatgacattggtggtaactggttttctcatatgaagtttcgtgctgatagagaaattcattgttgctgtccgatcttatctatgagagattctgaaagactggaaacacgcatgatggcaatgcaaaaatatatgcgtggatcgaaagacaaaccgttacgcttgttaagccgttatcaaaatatcctgcgtgaacaagcggcgagaacaactgcctttatggcaggtgaggtgaatgcgggtgttctcgatggagatgtgttttgtgagaacacttttcaagactgtgtgagacaggtgcccgaaggttttttgaagacagctatagcagttcatagcatctacgatatcaaagtggaagaatttgcgtctgcattgaaaagaaaaggtataacacaggcttatgggtgcttcctgtttcctcctgctgtattgataggtcagaaggaaggtattttaccttccgtggacggtcattacttggtggagaatggcaggattaagttcttctttgcgaatgatccgaatgccggttactctcatgaccttaaggattatctgaagtatgtggaaaaaacctacgtggatataaaggatggagtgtttgctattgagctgatgcaaatgcgaggtgataccatgttctttaagatcacggatgtcaccgcagcaatgtatcatatgaaatacagaggtatgaaacgtgatgaaacattcaaatgcattccgttgctaaaaaattcatccgttgtcgtacctctattttcgtgggacaaccgttctttaaagatcacaagtggtttattaccacgaactttggtcgagcaaggtgcggcgtttattatgaaaaacaaggagaaggacttgaacgttgctgtgttgaagaactatctttccgctgtgaacaactcatacattttcaacggatcccaggttagagatggtgtgaaaattgccccggatttaatctccaaattggcagtgactctgtacctgagagaaaaggtctatcgacaaagagaaaattcaatcataagttatttcgagcaagaaatgcttcacgatcccaacttgaaagccatgtttggagactttctgtggtttgttccaaatactctctcgagtgtctggaagaacatgcgaaaatcactgatggaatggtttggctacgcagaatttgacttgactacttttgatatttgcgatcccgttctctacgtagagatagtggatcggtataagatcattcaaaaagggcgaattccacttggtgagttttttgattgtcatgaagaatgcgagaattacgaactgcgtgagaaggagaaaaatgacctagcggtgaaaatggcccagaaggtaacagggacggtgaccgaatgcgagaaggacctgggacctcttgttcaaccgataaaacagatattggttcaacttgtgatgcccaatttggtcagagcgctgtgtagacctcgtagcccaacgtctcctttggacttaaatatcccagggtcaactccatcacactcaagttcagattctgaacaatctatgactgaagaagcgagctgcgccattgcgggtagcgtaccaacatgggaaattgcgactaagaaagatctaacctttcagcgaattgatgaagatatgtctcgacgaactggtatgcctccaagaccaaaagtaacttctagttacaacatgaatgccagagctgagtttctctactatcaactgtgtagcgtgatttgtgaaagggctcagattttgagtgtcatcgaagactttcgtcagaatttgatattctcagataaagtggccgttccattgaacgctagattctacagttttcagtcattgcaacccggatgggtgttcaagactccatcgcatagtgaagtaggccacagttatgcagtacattttgacttcaagacagttggaaccgatttggaagagagcctagctttttgccgaatggtaccgatttcatgggataaaagcggcaaatacatcgcgacaactcctcattttcccgagagacatggttactacgtgatttgtgacaacactaaattgtgtaacaattggcttatttacaataagttagttgatgtctacgcacgagtggctgatagacctctgagatttgagttgattgacggagttcctggctgcggaaagtcaaccatgattttaaacagctgtgatattcgacgcgaagttgttgttggtgaaggaaggaatgcaactgatgacttaagggagaggttcaagcgtaagaaaaatttgaatagtaagactgctaatcatagagttcgaacgcttgacagcttattacttgctgaaggaccttgtgtaccgcaagctgataggtttcattttgatgaagctctaaaagttcattacggcgccataatgttctgtgctgataagcttggtgcctcagaaattctcgctcagggagatagggctcaactgccgatgatctgtcgtgtagaaggtattgaacttcaatttcaatctcctgattacacgaagacgatcataaatcctaagctacgatcataccgtatccctggagatgttgccttctatttgagtgctaaggaattttacaaagttaaaggaatacctcaaaaggttacaacttctaacagtgtgaaacgttccctgtacgctagaggcgaaacaactccggaaagattcgtgagtttgcttgatgttccggtgagaaaaaacacccattatctaaccttcttacaagctgagaaggaaagtttgatgagtcatttgattccaaagggtgtgaagaaagagtctatttcaacgattcatgaggcgcagggtggtacctatgaaaatgtgattctggtccgtttgcaacggacgcccaatgaaatttatccgggtggacctaggtccgccccttacattgtggttgggacttcaaggcatacaaaaactttcacttattgtagtgttacggacgataagttgcttttagatatcgccgacgtcggtggtattgcacatacacctattcgtacttttgaatctcatatagtttaaaaaaaaaaaaaaaaaaaaaaaaaaaaaaaaaaaaaaaaaaatgtttgatcagatcattcaaatctgatggtgcccatcaaccatatgatgggagtgtttgcaagtccactataatcgaacttgaaaacgatgcctgaattggaaaccatgaatcttaacggattctggagagaaaatttaggaattggtatgtaagctacaacttccggtagctgcgtcacactttaagagtgtgcatactgagccgaagctcagcttcggtcccccaagggaagacca

SEQ ID NO: 33 - DNA, 3239 bp, Barley stripe mosaic virus BSMV ND18 RNA2 U35770
gtaaaagaaaaggaacaaccctgttgttgttcgacgctatactaaatatatattatcttattagtgcatttcttttaccacttcacagtatgccgaacgtttctttgactgctaagggtggaggacactacaacgaggatcaatgggatacacaagttgtggaagccggagtatttgacgattggtgggtccacgtagaagcctggaataaatttctagacaatttacgtggtatcaactttagcgttgcttcctctcggtcgcaagtcgctgaatgcttagctgcgttagatcgtgatctacctgctgatgtagacagacggtttgcaggtgctagaggacaaattggtttacccaattatcttcctgcgccaaaattctttcgtctcgataagcgaactatcgctgaactgactagactctctcgtcttacggatcagccgcacaacaatcgtgatatagagcttaaccgagcgaaaagagccacaactaacccatctcccccggcgcaggcaccgtcggagaatcttactcttcgtgatgttcaaccgttaaaggatagtgcgttgcattatcaatacgtgttgattgacctacagagtgcgagactcccagtgtataccaggaagactttcgaacgtgaactcgctttggaatggatcattccagatgccgaggaagcgtgacctgctgttgaagcggtaaaaggatgtacatatgtatcttatttattttgtttatctattttcttttacttttagtttttgctttttacgcgttaactagatgtattgactttagccatggacatgacgaaaactgttgaggaaaagaaaacaaatggaactgattcagtgaaaggtgtttttgaaaactcgacgattcccaaagttccgactggacaggaaatgggtggtgacgattcttctacttctaaattaaaggaaactctaaaagttgccgatcagactccattgtccgttgacaacggtgccaaatccaaattggattcttctgatagacaagttcctggtcctaagttggcaacaactgtggaaaaggaacctgagttgaaacccaacgttaagaagtccaagaagaaaagaatccaaaaacctgctcaaccgagtaggcccaatgaccttaaaggcgggactaagggatcatctcaagtgggtgaaaatgtgagtgagaactatactgggatttctaaggaagcagctaagcaaaagcagaagacacccaagtctgtgaaaatgcaaagcaatctggccgataagttcaaagcgaatgatactcgtagatcggaattaattaacaagtttcagcaatttgtgcatgaaacctgtcttaaatctgattttgagtacactggtcgacagtatttcagagctagatcaaatttctttgaaatgattaagctcgcatccttgtatgacaaacatctaaaggaatgtatggcgcgagcctgcaccctagaacgagaacgattgaagcgtaagttactcctagtacgagctttgaaaccagcagttgacttccttacgggaatcatctctggagttcctggctcaggaaaatcaaccattgtgcgtactttgctcaaaggtgaatttccggctgtttgtgctttggccaatcctgccttaatgaacgactattctggtattgaaggcgtttacgggttagatgacctgttgctttctgcagttccgataacgtctgatttattgatcatagatgaatatacacttgctgagagcgcggaaatcctgttgttacaacgaagactcagagcctctatggtgttgttagtcggggatgtagctcaaggaaaagccaccactgcttccagtattgagtatttaactctgccggtgatctacagatcagagacgacttatcgtttgggacaagagactgcttcgctttgcagcaagcagggtaacagaatggtttcaaagggtggaagggacacagtgatcattactgattacgatggcgaaacagatggaacggagaaaaatatcgcttttactgtcgatacagttcgagatgtgaaagattgcgggtacgattgtgccctggcaattgatgtgcaagggaaagaattcgattcagtgactttattcctaaggaacgaagaccggaaagctttagcagataagcatttgcgtttagtcgctttgagcagacataagtcgaagttaatcatcagggccgacgcggaaattcgtcaagcattcctgacaggtgatattgacttgagctctaaggcgagtaactctcatcgttattctgcaaaaccggatgaagaccacagttggttcaaggccaaataagtattggccaattgtcgccggaatcggtgtcgttggattgtttgcgtatttgatcttttcaaatcaaaaacattctacggaatccggcgataatattcacaaattcgccaacggaggtagttacagggacgggtcaaagagtataagttataatcgtaatcatccttttgcctatggcaatgcctcatcccctggaatgttgttgcccgcaatgcttaccatcatcggaatcatttcctatttatggcgaacaagagattccgtgctcggagactcaggcggaaacaattcctgcggagaagactgtcagggcgaatgtcttaacggacattctcgacgatcattactatgcgatattggctagtctttttatcattgctctatggttattgtatatatatctaagcagtatacctacggagactggtccctacttctatcaagatctgaactctgtgaagatctatggaataggggctacgaatccagaagttattgcggccatccaccattggcagaagtacccttttggggaatctccgatgtggggaggtttagtcagtgttttgagcgttcttcttaaaccgctgacgttagtttttgcgttaagcttttttctcttactttcttcaaaaaggtaaaaaaaaaaaaaaaaaaaatgtttgatcagatcattcaaatctgatggtgcccatcaaccatatgatgggagtgtttgcaagtccactataatcgaacttgaaaacgatgcctgaattggaaaccatgaatcttaacggattctggagagaaaatttaggaattggtatgtaagctacaacttccggtagctgcgtcacactttaagagtgtgcatactgagccgaagctcagcttcggtcccccaagggaagacca

SEQ ID NO: 34 - DNA, 2790 bp, Barley stripe mosaic virus BSMV ND18 RNA3 U13917
gtatagcttgagcattaccgtcgtgtaattgcaacacttggcttgccaaataacgctaaagcgttcacgaaacaaacaacacttcggcatggatgttgtgaagaaattcgccgtcatgtcagtgactgtagtagcaggtcccgtccttacgctttcatcacctgtggtggtgacgtttggaacaggcttaattgccgtatctttggtgaaacggttgctacaggaacaaccccgtgtaattgctcacgatcacgaacattacccaggtggttctgagagcagttctagctcttgtgctaccgcgcctattttacgtaatctttcgcgagatcagtgcgattcagagaatattggatgcagttctagcgcctgttctccgtctgaaattgtgaaagttacaaggcaggtagtgggagttgaacgtggtctttaccgggacatttttcaggacaacgaaatcccatcagtcatggaagagaaactgcagaaactcctttactctgagggtgagaagattcgaagacgttgccaatttgaagcatcaacgatgcactcacgcaaagtaaaggttccggaggtaggtactatcccagatatccaaacttggttcgatgctacgtttcctggtaactccgttaggttttctgatttcgacggttatactgttgctacggaggacattaacatggatgttcaggattgtagacttaagttcgggaagacttttcgaccttatgaatttaaggaatcactgaaaccagtactgaggacagcaatgccagaaaaacgacagggtagtttgattgaaagtgtgctggcctttcgtaaaagaaatttggctgcgcccagattacaaggagctttgaatgaatggcacacaattgagaatgtgctaacgaaggcgttaaaggtattcttctttgaagatttaattgatcgaacggatcactgcacttacgagtcagcgctcagatggtgggataaacaatcagtgacagctcgagcgcagctcgtggcggatcagcggaggttatgtgatgttgacttcacgacttataacttcatgataaaaaatgatgtaaagccgaagttagatctaacacctcaagttgaatatgcagctttgcagactgttgtatatcctgataagatagtcaatgctttctttggtccgatcataaaggagattaatgaacggatcatcagagcgcttagacctcatgtggtctttaattctcgtatgactgctgatgaactgaatgaaacagctgcctttttgacacctcataagtacagagccttagagattgatttttcaaaatttgataaatcaaagactgggcttcatatcaaagctgtcattggactctataagctctttggcctagatggcctgttaaaagtgctctgggaaaaatcgcaatatcagacttacgtgaaagatagaaacttcggtctcgaggcatatctattgtatcagcaaaagtcaggaaattgtgacacttacggttcgaacacctggtctgccgccttggcgttgttagattgtcttcctttggaagatgcacatttctgtgtatttggtggtgatgattcattgatattgtttgatcagggatacataatttccgacccatgccggcaacttgccggtacttggaatcttgaatgtaaagtgttcgacttcaagtaccccgcattttgtggtaaatttctgctgtgcatagatggaaaatatcaatttgttccagatgcggcaaaatttatcacaaaattaggtagaactgatgtgagagatgtagaagttttgagtgagatttatatctctatcaatgacaattacaaatcttacaaagactttaaggtgcttgatgctttggataaggctttagtggatagatatcgatccccttatagtgctatttctgctttggtttctttatgttatcatatctttgactttaataagtttaagttgctgtttaattgtgaagggaaatttgtggataagaagctgagaaaagacttcgagtggtgaactctaggtcctgatgtttaaatctactgtatttaccttcgcatgatggctactttctcttgtgtgtgttgtggtaccttaactacaagtacttactgtggtaagagatgtgagcgaaagcatgtatattctgaaacaagaaataagagattggaactttacaagaagtatctattggaaccgcaaaaatgcgccctgaatggaatcgttggacacagttgtggaatgccatgctccattgcggaagaggcttgtgatcaactgccaatcgtgagtaggttctgtggccaaaagcatgcggatctgtatgattcacttctgaaacgttctgaacaggagttacttcttgaatttctccagaagaagatgcaggagctgaaactttctcatatcgtaaaaatggctaagcttgaaagtgaggttaacgcaatacgtaagtccgtagcttcttcttttgaagattctgttggatgtgatgattcttcttccgtttctaagtaaaaaaaaaaaaaaatgtttgatcagatcattcaaatctgatggtgcccatcaaccatatgatgggagtgtttgcaagtccactataatcgaacttgaaaacgatgcctgaattggaaaccatgaatcttaacggactctggagagaaaatttaggaattggtatgtaagctacaacttccggtagctgcgtcacactttaagagtgtgcatactgagccgaagctcagcttcggtcccccaagggaagacca

SEQ ID NO: 35 - DNA, 3768 bp, Barley stripe mosaic virus BSMV_RNA1_gi|19744917|ref|NC_003469.1|
gtatgtaagttgcctttgggtgtaaaatttcttgcatgcacataatcgtaatcgattcttcttgatctctaaacaacactttcccgttagcatggctagcgatgagattgtccgcaatctgatctcccgtgaggaggtgatgggtaatttgattagcacagcttctagctcagtaaggtcacccttacatgacgtactgtgctcgcacgtaaggaccatcgtcgattccgtggataagaaagcggtcagtcgcaagcatgaagatgtacggcgcaacatctcctctgaggaattgcagatgttgataaatgcatatcctgaatatgccgtttcatcctcagcttgtgaatctggtactcatagcatggcggcttgttttcgatttctggagacagaatatctcttagatatggttccaatgaaagagacttttgtttatgacattggtggcaactggttttctcatatgaagtttcgtgctgatagagaaattcattgttgctgtccgatcttatctatgagagattctgaaagactggaaacacgcatgatggcaatgcaaaaatatatgcgtggatcgaaagacaaaccgttacgcttgttaagccgttatcaaaatatcctgcgtgaacaagcggcgagaacaactgcctttatggcaggtgaggtgaatgcgggtgttctcgatggagatgtgttttgtgagaacacttttcaagactgtgtgagacgagtgcccgaaggttttttgaagacagctatagcagttcatagcatctacgatatcaaagtggaggaatttgcgtctgcattgaaaagaaaaggtataacacaggcttatgggtgtttcctgtttcctcctgctgtattgataggtcagaaggaaggcattttaccttccgtggacggtcattacttggtggagaatggcaggattaagttcttctttgcgaatgatccgaatgccggttactctcatgaccttaaggattatctgaagtatgtggaaaagacctatgtggatatagaggatggagtgtttgctattgagctgatgcaaatgcgaggtgataccatgttctttaagatcacggatgtcaccgcagcaatgtatcatatgaaatacagaggtatgaaacgcgatgaaacattcaaatgcattccgttgctaaagaattcatctgttgtcgtacctctattttcgtgggacaaccgttctttaaagatcacaagtggtttactaccacgaactttggtcgagcagggtgcggcttttattatgaaaaacaaggagaaggacttgaacgttgctgtgttgaagaactatctttccgctgtgaacaactcatacattttcaacggatcccaggttagagatggcgtgaaaattgccccggatttaatctccaagttggcagtgactctgtacctgagagaaaaagtctatcgacaaagagaaaattcaatcataagttatttcgagcaagaaatgcttcacgatcccaacttgaaagccatgtttggagactttctgtggtttgttccaaatactctctcgagtgtctggaagaacatgcgaaaatcactgatggaatggtttggctacgcagaatttgacttgactacttttgatatttgcgatcccgttctctatgtagagatagtggatcggtataagatcattcaaaaagggcgaattccacttggtgagttctttgattgtcatgaagaatgcgagaattacgaactgcgtgagaaggagaaaaacgacctagcggtgaaaatggcccagaaggtaacagggacggtgaccgaatgcgagaaggacctgggacctcttgttcaaccgataaaagagatattggttcaacttgtgatgcccaatttggtcagagcgctgtgtagacctcgtagcccaacgtctcctttggacttaaaaagtatcccagggtcaactccatcacactcaagttcagattctgaacactctatgactgaagaagcgagctgcaccattgcgggtagcgtaccaacatgggaaattgcgactaggaaagatctaacctttcagcgaattgatgaagatatgtctcgacgaactggtatgcctccaagaccaaaagtaacttctagttacaacatgaatgccagagctgagtttctctactatcaactgtgtagcgtgatttgtgaaagggctcagattttgagtgtcatcgaagactttcgtcagaatttgatattctcagataaagtggccgttccattgaacgctagattctacagttttcagtcattgagacccggatgggtgttcaaaactccatcgcatagtgaagtaggccacagttatgcagtacattttgacttcaagacaattggaaccgatttggaagagagcctagctttttgccgaatggtaccgatttcatgggataaaagcggcaaatacatcgcgacaactcctcattttcccgagagacatggttactacgtgatttgtgacaacactaaattgtgtaacaattggcttatttacaataagttagttgacgtctacgcactagtggctgatagacctctgagattcgagttgattgacggagttcctggctgcggaaagtcaaccatgattttaaacagctgtgatattcgacgcgaagttgttgttggtgaaggacggaatgcaactgatgacttaagggagaggttcaagcgtaagaaaaatttgaatagtaagactgctaatcacagagttcgaacgcttgacagcttattacttgctgaaggaccttgtgtaccgcaagctgataggtttcattttgatgaagctctaaaagttcattacggcgccataatgttctgtgctgataagcttggtgcctcagaaattctcgctcagggagatagggctcaattgccaatgatctgtcgtgtagaaggtattgaacttcaatttcaatctcctgattacacgaagacgatcataaatcctaagctacggtcataccgtatccctggagatgttgccttctatttgagtgctaaggaattttacaaagttaaaggaatacctcaaaaggttataacttctaacagtgtgaaacgttccttgtacgctagaggcgaaacgactccggaaagattcgtgagtttgcttgatgttccggtgagaaaagacacccactatctaaccttcttacaagctgagaaggaaagtttgatgagtcatttgattccaaagggtgtgaagaaagagtctatttcaacgattcatgaggcgcagggtggtacctatgaaaatgtgattctggtccgtttgcaacggacgcccaatgaaatttatccgggtggacctaggtccgccccttacattgtggttgggacttcaaggcatacaaaaactttcacttattgtagtgttacggacgataagttgcttttagatatcgccgacgtcggtggtattgcacatacacctattcgtacttttgaatctcatatagtttaaaaaaaaaaaaaaaaaaaaatgtttgatcagatcattcaaatctgatggtgcccatcaaccatatgatgggagtgtttgcaagtccactataatcgaacttgaaaacgatgcctgaattggaaaccatgaatcttaacggattctggagagaaaatttaggaattggtatgtaagctacaacttccggtagctgcgtcacactttaagagtgtgcatactgagccgaagctcagcttcggtcccccaagggaagacca

SEQ ID NO: 36 - DNA, 3289 bp, Barley stripe mosaic virus BSMV_RNA2_gi|19744922|ref|NC_003481.1|
gtaaaagaaaaggaacaaccctgttgttgttcgacgctatactaaatatatattatcttattagtgcatttcttttaccgcttcacagtatgccgaacgtttctttgactgctaagggtggaggacactacatcgaggatcaatgggatacacaagttgtggaagccggagtatttgacgattggtgggtccacgtagaagcctggaataaatttctagacaatttacgtggtatcaactttagcgttgcttcctctcggtcgcaagtcgctgaatacttagctgcgttagatcgtgatctacctgctgatgtagacagacggtttgcaggtgctaggggacaaattggttcacccaattatcttcctgcgccaaaattctttcgtctcgataagcgaactatcgctgaactgactagactctctcgtcttacggatcagccgcacaacaatcgcgatatagaacttaaccgagcgaaaagagccacaactaacccatctcccccggcgcaggcaccgtcggagaatctcactcttcgtgatgttcaaccgttaaaggatagtgcgttgcattatcaatacgtgttgattgacctacagagtgcgagactcccggtgtataccaggaagactttcgaacgtgaactcgctttggaatggatcattccagatgccgaggaagcgtgacctgctgtcgaagcggtaaaaggatgtacatatgtatcttatttattttgtttatctattttcttttgcttttagtttttgctttttacgcattaactagatgtattgactttagccatggacatgacgaaaactgttgaggaaaagaaaacaaatggaactgattcagtgaaaggtgtttttgaaaactcgacgattcccaaagttccgactggacaggaaatgggtggtgacggttcttctacttctaaattaaaggaaactctgaaagttgccgatcagactccattgtccgttgacaatggtgccaaatccaaattggattcctctgatagacaagttcctggagttgccgatcagactccattgtccgttgacaatggtgccaaatccaaattggattcctctgatagacaagttcctggacctgagttgaaacccaacgttaagaagtccaagaagaaaagaatccaaaaacctgctcaaccgagtgggcccaatgaccttaaaggcgggactaagggatcatctcaagtgggtgaaaatgtgagtgagaactatactgggatttctaaggaagcagctaagcaaaagcagaagacgcccaagtctgtgaaaatgcaaagcaatctggccgataagttcaaagcgaatgatactcgtagatcggaattaattaacaagtttcagcaatttgtgcatgaaacctgtcttaaatctgattttgagtacactggtcgacagtatttcagagctagatcaaatttctttgaaatgattaagctcgcatccttgtatgacaaacatctaaaggaatgtatggcgcgagcctgcaccctagaacgtgaacgattgaagcgtaagttactcctagtacgagctttgaaaccagcagttgacttccttacgggaatcatctctggagttcctggctcaggaaaatcaaccattgtgcgtactttgctcaaaggtgaatttccggctgtttgtgctttggccaatcctgccttaatgaacgactattctggtattgaaggcgtttacgggttagatgacctgttgctttctgcagttccgataacgtctgatttattgatcatagatgaatatacacttgctgagagcgcggaaatcctgttgttacaacgaagactcagagcctctatggtgttgttagtcggggatgtagctcaaggaaaagccaccactgcttccagtattgagtatttaactctgccggtgatctacagatcagagacgacttatcgtttgggacaagagactgcttcgctttgcagcaagcagggtaacagaatggtttcaaagggtggaagggacacagtgatcattactgattacgatggcgaaacagatgaaacggagaaaaatatcgcttttactgtcgatacagttcgagatgtgaaagattgcgggtacgattgtgccctggcaattgatgtgcaagggaaagaattcgattcagtgactttattcctaaggaacgaagaccggaaagctttagcagataagcatttgcgtttagtcgctttgagcagacataagtcgaagttaatcatcagggccgacgcggaaattcgtcaagcattcctgacaggtgatattgacttgagctctaaggcgagtaactctcatcgttattctgcaaaaccggatgaagaccacagttggttcaaggccaaataagtattggccaattgtcgccggaatcggtgtcgttggattgtttgcgtatttgatcttttcaaatcaaaaacattctacggaatccggtgataatattcacaaattcgccaacggaggtagttacagagacgggtcaaagagtataagttataatcgtaatcatccttttgcctatggcaatgcctcatcccctggaatgttgttgcccgcaatgcttaccatcatcggaatcatttcctatttatggcgaacaagagattccgtgctcggagactcaggcggaaacaactcctgtggagaagactgtcagggcgaatgtcttaacggacattctcgacgatcattactatgcgatattggctagtctttttatcattgctctatggctattgtatatatatctaagcagtatacctacggagactggtccctacttctatcaagatctgaactctgtgaagatctatggaataggggctacgaacccagaagttattgcggccatccaccattggcagaagtacccttttggggaatctccgatgtggggaggtttaatcagtgttttgagtattcttcttaaaccgctgacattagtttttgcgttaagcttttttctcttactttcttcaaaaaggtaaaaaaaaaaaaaaaaaaaaaatgtttgatcagatcattcaaatctgatggtgcccatcaaccatatgatgggagtgtttgcaagtccactataatcgaacttgaaaacaatgcctgaattggaaaccatgaatcttaacggattctggagagaaaatttaggaattggtatgtaagctacaacttccggtagctgcgtcacactttaagagtgtgcatactgagccgaagctcagcttcggtcccccaagggaagacca

SEQ ID NO: 37 - DNA, 3164 bp, Barley stripe mosaic virus BSMV_RNA3_gi|19744919|ref|NC_003478.1|
gtatagcttgagcattaccgtcgtgtaattgcaacacttggcttgccaaataacgctaaagcgttcacgaaacaaacaacaattcggcatggatgttgtgaagaaattcgccgtcatgtcagtgactgtagtagcaggtcccgtccttacgctttcatcacctgtggtggtgacgtttggaacaagcttaattgccgtatctttggtgaaacggttgctacaggaacaaccccgtgtaattgctcacgatcacgaacattacccaggtggttctgagagcagttctagctcttgtgctaccgcgcctattttacgtaatctttcgcgagatcagtgcgattcagagaatattggatgcagttctagcgcctgttctccgtctgaaattgtgaaagttacaaggcaggtagtggaagttgaacgtggtctttaccgggacaaacaacaattcggcatggatgttgtgaagaaattcgccgtcatgtcagtgactgtagtagcaggtcccgtccttacgctttcatcacctgtggtggtgacgtttggaacaagcttaattgccgtatctttggtgaaacggttgctacaggaacaaccccgtgtaattgctcacgatcacgaacattacccaggtggttctgagagcagttctagctcttgtgctaccgcgcctattttacgtaatctttcgcgagatcagtgcgattcagagaatattggatgcagttctagcgcctgttctccgtctgaaattgtgaaagttacaaggcaggtagtggaagttgaacgtggtctttaccgggacatttttcaggacaacgaaatcccatcagtcatggaagagaaactgcagaaactcctttactctgagggtgagaagattcgaagacgttgccaatttgaagcatcaacgatgcactcacgcaaagtaaaggttccggaggtaggtactatcccagatatccaaacttggttcgatgctacgtttcctggtaactccgttaggttttctgatttcgacggttatactgttgctacggaggacattaacatggatgttcaggattgtagacttaagttcgggaagacttttcgaccttatgaatttaaggaatcactgaaaccagtactgaggacagcaatgccagaaaagcgacagggtagtttgattgaaagtgtgctggcctttcgtaaaagaaatttggctgcgcccagattacaaggggctttgaatgaatggcacacaattgagaatgtgctgaagaaggcgttaaaggtattcttctttgaagatttaattgatcgaacggatcattgcacttacgagtcagcgctcagatggtgggataaacaatcagtgacggctcgagcgcagctcgtggcggaccaacggaggttatgtgatgttgacttcacgacttataacttcatgataaaaaatgatgtaaaaccgaagttagatctaacacctcaagttgaatatgcagctttgcagactgttgtgtatcctgataagatagtcaatgctttctttggtccgatcataaaggagattaatgaacggatcatcagagcgcttagacctcatgtggtctttaattctcgtatgactgctgatgaactgaatgaaacagttgcctttttgacacctcacaagtacagagccttagagattgacttttcaaaatttgataaatcaaagactgggcttcatatcaaagctgtcattggactctataagctctttggtctagatggcctgttaaaagtactctgggaaaaatcgcaatatcagacttacgtgaaagatagaaacttcggtctcgaggcatatctattatatcagcaaaagtcaggaaattgtgacacttacggttcgaacacctggtctgccgccttggcgttgttagattgtcttcctttggaagatgcacatttctgtgtatttggtggtgatgattcattgatattgtttgatcagggatacataatttccgacccatgccggcaacttgccggtacttggaatcttgaatgtaaagtgttcgacttcaagtaccccgcattttgtggtaaatttctgctgtgcatagatggaaaatatcagtttgttccagatgcggcaaaatttatcacaaaattaggtagaactgatgtgagagatgtagaagttttgagtgagatttatatctctatcaatgacaattacaaatcttacaaagactttaaggtgcttgatgctttggataaggctttagtggacagatatcgatccccttatagtgctatttctgctttggtttctttatgttatcatatctttgactttaataagtttaagttgctgtttaattgtgaagggaaatttgtggataagaagctgagaaaggacttcgagtggtgaactctgggtcctgatgtttaaatctactgtatttaccttcgcatgatggctactttctcttgtgtgtgttgtggtacctcaactacaagtacttactgtggtaagagatgtgagcgaaagcatgtatattctgaaacaagaaataagagattggaactttacaagaagtatctattggaaccgcaaaaatgcgccctgaatggaatcgttggacacagttgtggaatgccatgctccattgcggaagaggcttgtgatcaactgccaatcgtgagtaggttctgtggccaaaagcatgcggatctgtatgattcacttctgaaacgttctgaacaggagttacttcttgaatttctccagaagaagatgcaggagctgaaactttctcatatcgtaaaaatggctaagcttgaaagtgaggttaacgcaatacgtaagtccgtagcttcttcttttgaagattctgttggatgtgatgattcttcttccgtttctaagttgtaaaaaaaaaaaaaaaaaaaatgtttgatcagatcattcaaatctgatggtgcccatcaaccatatgatgggagtgtttgcaagtccactataatcgaacttgaaaacgatgcctgaattggaaaccatgaatcttaacggattctggagagaaaatttaggaattggtatgtaagctacaacttccggtagctgcgtcacactttaagagtgtgcatactgagccgaagctcagcttcggtcccccaagggaagacca

SEQ ID NO: 38 - DNA, 2360 bp, Maize stripe virus segment 3, complete sequence GenBank: AJ969410.1
acacaaagtcctgggtaaaaaatattattttttatcaatatatatattacttctgtccatcgaagcatgaacttttacacatcatctgttggagtgcgacaatacgaccactctttattggtcttgaatgatctcaccaacattcatatcacttgtgaggatgtccactgctctgcaaagctcctctgctacatatatgatatctacaagtctaggtacccatcaatggatgagcattctttcttgcgcttgctaaaaggtccagatgatgctgagatacttagcacctttttgagaacaatcatttggatactgtctcatgacagagacttcccagatgagttcaggattccagctacagcacttgcttcagtttatataaaatattactctgaattgaaaccaagagctcctaccaccaattgttggacatgcagaatgtccaaaaacaatctacctttccaagtcccctcaataaagggattccctgctgaagcagagctatatatagttccaatctctgatcatgatggaaagacaatagagttttcaggaatgaaaacactgtacaagtctccaagcaagaagaaacacaattatgtcatttcatcagatatgcccccacttagtgctagatacactgtctgggatggcaaatagagtagtatctgtagaatcccctttctaggagtgtacggataatgtaactaagttacattttaagaataaaaaagtgtgctaagcacactatccgaatagcaatcggatgaaggccttaacctaattttttgtttttttgcttttttgttttttatttgtttttttgttttttcatttttttggtttttttaatatattataagattttgagcactctaaaagctcaatttattatacacactatatgtacatatcaataatagtgaactaaaaagcacaagcactaaaatataatagaagcaaaagcaaagcataataaacatcataaactataataagataatattgttaaaccataataataatgacacacaaacactcaatactaatattatcatactctcattcatacttgtttttgattttccattttcccatttttttgtttttttgtataatctaatttttatggttttcttgatttttttgatttttttgtttttttgtttaaaacacacaatacaataatataacacaaacaacacacttaaatagaatatcatgacacaatgtgagcacttcccctgctcagtgccagaccgtcttatccaacgcattcttccactttatgatgatatcatcatagtatgaggaactcactcctcctcgaagaactcaatgatcaatgccttcatctcatcctgagtctttgagctgttgtctacaatggttttcatcaagctgcactgttctgccaaaaattgcttgacctgagtaccataggagcagacaacattctttccgaatgatgcaagcaaggccaagaatgactccttgaatttctcattaacatagtatggctcacatactttggtcctcccagatttcttcttcgcttcgttgaggtttttggattgacaggtgatgaccagcaaaccagtggtatactttatcatgtctatgtctttgagcaatcctctctccttcttttttgtctctggcattgttttcttagtgaccaagaaagcatgaatcacatgaatgctgaaaagaatgtggttgacactcttagttgtgcagtatggtgcagatgagctgtcaagtgtaatatattggggaacaaagtcccacagcagggaatcagtcccagacatgctaagatcagatgaatcaatagccattttcagaccagtgaactgtttggtcacctcataggatacatttggaaagagttgagctacccttcccagtgtaatagcatttgcgttgctacccacagatgaaactaatccatagcgggcaaccaatgccgctgcttcctcactgccagcagttgccttggttttcttagtgacatccttaacaaagccagtccctcggacatacctcatcacaatcatcttgacaacatcttgagcaagagttgccccacccttgtctttgagaataccaatcaaagtagccgcatcatagcctgcataccctatctgatcatgaaaggtggtcacagacgccttgttatcagtgagatacttcaaagcatctttggagatatcattgatagctttctggagatcattaagatttgcaggcttattagtggccattttcttcaagggtattggtgcaatggttatgatttagacctttctttagttgatcaatacgaaatcgattaaacgattacccagactttgtgt

SEQ ID NO: 39 - protein, 1368 aa, Streptococcus pyogenes [sequence omitted]

SEQ ID NO: 40 - DNA, 1880 bp, Brachypodium distachyon; identical to SEQ ID NO: 11

SEQ ID NO: 41 - DNA, 17 bp, Artificial Sequence
  Protospacer Region guide RNA 14
tggttctgcctctggtc

SEQ ID NO: 42 - DNA, 20 bp, Artificial Sequence
  Protospacer Region guide RNA 16
taacggatagcgctcctcgt

SEQ ID NO: 43 - DNA, 20 bp, Artificial Sequence
  Protospacer Region guide RNA 37
tggagcttaccgactcgctc

SEQ ID NO: 44 - DNA, 20 bp, Artificial Sequence
  Protospacer Region guide RNA 38
ggagcttaccgactcgctca

SEQ ID NO: 45 - DNA, 20 bp, Artificial Sequence
  Protospacer Region guide RNA 39
ggaaagctgctggcgacagg

SEQ ID NO: 46 - DNA, 20 bp, Artificial Sequence
  Protospacer Region guide RNA 43
tcctggtcgaacttttcagg

SEQ ID NO: 47 - DNA, 20 bp, Artificial Sequence
  Protospacer Region guide RNA 18
taattctagtacatggatat

SEQ ID NO: 48 - DNA, 20 bp, Artificial Sequence
  Protospacer Region guide RNA 52
cggtcataaagcagctctca

SEQ ID NO: 49 - protein, 9 aa, Simian virus 40
MAPKKKRKV

SEQ ID NO: 50 - protein, 18 aa, Agrobacterium tumefaciens
KRPRDRHDGELGGRKRAR

SEQ ID NO: 51 - protein, 18 aa, Agrobacterium tumefaciens
KRPREDDDGEPSERKRER

SEQ ID NO: 52 - protein, 17 aa, Agrobacterium tumefaciens
KLRPEDRYVQTERYGRR

SEQ ID NO: 53 - protein, 17 aa, Agrobacterium tumefaciens
KLRPEDRYIQTEKYGRR

SEQ ID NO: 54 - protein, 15 aa, Agrobacterium tumefaciens
KRRYGGETEIKLKSK

SEQ ID NO: 55 - protein, 15 aa, Agrobacterium tumefaciens
KTKYGSDTEIKLKSK

SEQ ID NO: 56 - protein, 20 aa, Agrobacterium rhizogenes
KRKRAAAKEEIDSRKKMARH

SEQ ID NO: 57 - protein, 20 aa, Agrobacterium rhizogenes
KRKRVATKEEIEPHKKMARR

SEQ ID NO: 58 - protein, 18 aa, Agrobacterium rhizogenes
KRPRVEDDGEPSERKRAR

SEQ ID NO: 59 - DNA, 3738 bp, Artificial Sequence
  pEn Chimera Vector
gggcgaattgggcccgacgtcgcatgctcccggccgccatggcggccgcgggaattcgatcaaataatgattttattttgactgatagtgacctgttcgttgcaacaaattgatgagcaatgcttttttataatgccaactttgtacaaaaaagcaggctctttttttcttcttcttcgttcatacagtttttttttgtttatcagcttacattttcttgaaccgtagctttcgttttcttctttttaactttccattcggagtttttgtatcttgtttcatagtttgtcccaggattagaatgattaggcatcgaaccttcaagaatttgattgaataaaacatcttcattcttaagatatgaagataatcttcaaaaggcccctgggaatctgaaagaagagaagcaggcccatttatatgggaaagaacaatagtatttcttatataggcccatttaagttgaaaacaatcttcaaaagtcccacatcgcttagataagaaaacgaagctgagtttatatacagctagagtcgaagtagtgattggggtcttcgagaagacctgttttagagctagaaatagcaagttaaaataaggctagtccgttatcaacttgaaaaagtggcaccgagtcggtgctttttttctagacccagctttcttgtacaaagttggcattaacccagctttcttgtacaaagttggcattataaaaaataattgctcatcaatttgttgcaacgaacaggtcactatcagtcaaaataaaatcattatttgatcactagtgaattcgcggccgcctgcaggtcgaccatatgggagagctcccaacgcgttggatgcatagcttgagtattctatagtgtcacctaaatagcttggcgtaatcatggtcatagctgtttcctgtgtgaaattgttatccgctcacaattccacacaacatacgagccggaagcataaagtgtaaagcctggggtgcctaatgagtgagctaactcacattaattgcgttgcgctcactgcccgctttccagtcgggaaacctgtcgtgccagctgcattaatgaatcggccaacgcgcggggagaggcggtttgcgtattgggcgctcttccgcttcctcgctcactgactcgctgcgctcggtcgttcggctgcggcgagcggtatcagctcactcaaaggcggtaatacggttatccacagaatcaggggataacgcaggaaagaacatgtgagcaaaaggccagcaaaaggccaggaaccgtaaaaaggccgcgttgctggcgtttttccataggctccgcccccctgacgagcatcacaaaaatcgacgctcaagtcagaggtggcgaaacccgacaggactataaagataccaggcgtttccccctggaagctccctcgtgcgctctcctgttccgaccctgccgcttaccggatacctgtccgcctttctcccttcgggaagcgtggcgctttctcatagctcacgctgtaggtatctcagttcggtgtaggtcgttcgctccaagctgggctgtgtgcacgaaccccccgttcagcccgaccgctgcgccttatccggtaactatcgtcttgagtccaacccggtaagacacgacttatcgccactggcagcagccactggtaacaggattagcagagcgaggtatgtaggcggtgctacagagttcttgaagtggtggcctaactacggctacactagaagaacagtatttggtatctgcgctctgctgaagccagttaccttcggaaaaagagttggtagctcttgatccggcaaacaaaccaccgctggtagcggtggtttttttgtttgcaagcagcagattacgcgcagaaaaaaaggatctcaagaagatcctttgatcttttctacggggtctgacgctcagtggaacgaaaactcacgttaagggattttggtcatgagattatcaaaaaggatcttcacctagatccttttaaattaaaaatgaagttttaaatcaatctaaagtatatatgagtaaacttggtctgacagttaccaatgcttaatcagtgaggcacctatctcagcgatctgtctatttcgttcatccatagttgcctgactccccgtcgtgtagataactacgatacgggagggcttaccatctggccccagtgctgcaatgataccgcgagacccacgctcaccggctccagatttatcagcaataaaccagccagccggaagggccgagcgcagaagtggtcctgcaactttatccgcctccatccagtctattaattgttgccgggaagctagagtaagtagttcgccagttaatagtttgcgcaacgttgttgccattgctacaggcatcgtggtgtcacgctcgtcgtttggtatggcttcattcagctccggttcccaacgatcaaggcgagttacatgatcccccatgttgtgcaaaaaagcggttagctccttcggtcctccgatcgttgtcagaagtaagttggccgcagtgttatcactcatggttatggcagcactgcataattctcttactgtcatgccatccgtaagatgcttttctgtgactggtgagtactcaaccaagtcattctgagaatagtgtatgcggcgaccgagttgctcttgcccggcgtcaatacgggataataccgcgccacatagcagaactttaaaagtgctcatcattggaaaacgttcttcggggcgaaaactctcaaggatcttaccgctgttgagatccagttcgatgtaacccactcgtgcacccaactgatcttcagcatcttttactttcaccagcgtttctgggtgagcaaaaacaggaaggcaaaatgccgcaaaaaagggaataagggcgacacggaaatgttgaatactcatactcttcctttttcaatattattgaagcatttatcagggttattgtctcatgagcggatacatatttgaatgtatttagaaaaataaacaaataggggttccgcgcacatttccccgaaaagtgccacctgatgcggtgtgaaataccgcacagatgcgtaaggagaaaataccgcatcaggaaattgtaagcgttaatattttgttaaaattcgcgttaaatttttgttaaatcagctcattttttaaccaataggccgaaatcggcaaaatcccttataaatcaaaagaatagaccgagatagggttgagtgttgttccagtttggaacaagagtccactattaaagaacgtggactccaacgtcaaagggcgaaaaaccgtctatcagggcgatggcccactacgtgaaccatcaccctaatcaagttttttggggtcgaggtgccgtaaagcactaaatcggaaccctaaagggagcccccgatttagagcttgacggggaaagccggcgaacgtggcgagaaaggaagggaagaaagcgaaaggagcgggcgctagggcgctggcaagtgtagcggtcacgctgcgcgtaaccaccacacccgccgcgcttaatgcgccgctacagggcgcgtccattcgccattcaggctgcgcaactgttgggaagggcgatcggtgcgggcctcttcgctattacgccagctggcgaaagggggatgtgctgcaaggcgattaagttgggtaacgccagggttttcccagtcacgacgttgtaaaacgacggccagtgaattgtaatacgactcactata

SEQ ID NO: 60 - DNA, 1023 bp, Zea mays
ctttgacttttcccttaatgacgacttattatttaatttactcgtcacgattcccctctcctggtcgaacttttcaggtggggaaagctgctggcgacaggtggaaatccctgagcgagtcggtaagctccatcttctgtactaaagtagtagttgattggactagaaatctcgtgctgattaattgttttacgcgtgcgtttgtgtggattgtaggacaaggctccctatgtagccaaggctaacaagctcaagctcgagtacaacaaggccatcgctgcctacaacaagggcgaggtagggaaactgatgcttcaattgcgttgttacttaatgtgtatatagactgctcctgctggtcatttattcaaatacgtatgcttactgaaccatgtgttgtttgttcagagcactgcagctaagaaggctcctgccaaggaggaagaggaggaagatgaagaggagtctgacaagtccaagtcggaggtcaatgacgaggatgatgaagagggtagtgaggaggtatacaaaatctattcctgtcttctccatattttttccttagacaaaataccaattaatccaggatacatagcatgttcatgcattaagcaagttgctaaatttatcttcgaccacaatgtagacctagtagtattgtattggattccatcaatgcaaaacatatgcagatttgcatatgcaaccctcttttgcaagtcctcaatatgagcatttgtttggaacacggtgcattggccttaggaagtctttaaaaatatgtcttccctctgcttgcaggatgaagatgatgacgagtgatggagctcctcgagacaatggaccgtgcttcatccaacaatggagcggctacacaaggccccgtggcgatcacaaaaaaggagcctatatccatgtactagaattattcagtttcactccacatcgtgatgttttatttttacttttgtcgtgctataacggatagcgctcctcgttggcgccactggcgggtggttctgc

SEQ ID NO: 61 - DNA, 210 bp, Artificial Sequence
  genome edited hmg13 gene
ctttgacttttcccttaatgacgacttattatttaatttactcgtcacgattcccctctcctggtcgaacttttcaggtggggaaagctgctggcgactccatgtactagaattattcagtttcactccacatcgtgatgttttatttttacttttgtcgtgctataacggatagcgctcctcgttggcgccactggcgggtggttctgc